European Patent Specification EP 3 668 988 B1, published July 23, 2025. Title: RECOMBINANT VIRAL VECTOR SYSTEMS EXPRESSING EXOGENOUS FELINE PARAMYXOVIRUS GENES AND VACCINES MADE THEREFROM. Applicant: Boehringer Ingelheim Vetmedica GmbH Boehringer Ingelheim Animal Health USA Inc. The sequence listing filed with the application follows.

SEQUENCE LISTING (95 sequences)

SEQ ID NO: 1 - DNA, 16047 bp, Feline paramyxovirus type 2
  misc_feature: FPaV-2 "Gordon strain" full genome sequence; given as a DNA sequence that correspond to the positive RNA-strand into which the negative RNA strand viral genome is transcribed, i.e. it comprises the ORFs in 5' to 3' direction like an mRNA
accagacaaagatgtctgtgacctattctaacggttagattattacttgatatttaggaataacgattccattagtcaggtaagggagaggaatcagttattctataatggctagtttactcaggtcacttgcggcattcaagaaacacagagaacaaccaactgttccttctgggtcaggagggacgatcaaaggattaaaaaatacaattattgtgcctgttcctggagatacagtcatcactaccagatcgaacttactgttcagattagtctacataattggtaatccagatacacctttaagcacttcaacaggggcaataatatcattgttgacattatttgttgaatctccaggtcaattaattcaaagaatcgctgatgatcctgatgctgtttttaaattagtagaggtggttcctgaggttggtaatcctggagaattaacttttgcatctagaggaattaacttggataaacaagctcaacaatactttagattggctgagaaaaatgatcaaggatattatgtaagtttggggtttgaaaatccaccaaatgatgatgatataacgtcaagtcctgaaatctttaattatattttagcatctgtacttgcacagatctggattctcctagctaaggctgtaactgctccagacacagctgctgaggctgaaaaccgtaggtggattaaattgatgcaacaacgcagagtggatggtgagcttagattaagtaaaggatggttggacttagtgaggaataaaatcgcatcggatatcacaattagaaggtttatggtagcattagttcttgacattaaacgttctcctggaacaagaccaagaattgctgaaatgatttgtgatatagacaattatattgtggaggccggactggcaagttttctgttaactatcaaatttggtatagaaacacgttacccggcattagcgttacatgagttttcgggggaattagccactattgaaggactcatgaaattgtaccagtctatgggagaaatggcaccatacatggtcattctagagaattcgatccagactaggtttagtgctgggtcttatccgttactctggagctatgctatgggtgttggtgtagaacttgaaagatcaatgagtggattaaacttcacaagaagtttctttgatcctacgtacttcaggttgggtcaggagatggtaagaaggtcttcaggaatggttaatagctcatttgccaaagaacttggactatctgaacatgaaacacaacttgttagccagatcattaactcaggtggtgagtcaggtataccgaaatttgatggatttagagcaaacccaacaacatttctaggggctaaggacaacatcactgataggagtgaagatccattgattgcaattccagggtcatcaggacaaccattgccaggttatgaccccaatatctcaggtgactcatatagaattgatagtagcactaaagacacaaacaatatatcagatggaggaacaaatccaagtcatgatgtttccaattctgctatggaagagctgagaagattggtagagtctaccaacaagattgatacaaagaaatctgaaagcccaggcatcgttaatcattacaacgatactgaccttctgagataataaggatatattcaggtagatctttacagaatttaaattaagaaaaacttaggacctcaaggttcacactcctctggcctttatcagaattcggccaattcctcactcactccatgtcagcagaacaaatccaacaagttagacatggccttgaatccttgcaagagatcaaaaacaaccctccaccctctcaagatgtcaatcttgccagggaaatttacgaatccattaaacaaacaggaacaccttcaacacaaggagggaccattacaggaaataatactgcgtcagggtgtgacaattactcaatgcatagccagggatcaggtccttctgtttcaggtgctgacaagaatatcgagagacttactggacccgattattcagaattatgggatccagaaggtaacctctgcatgctattcgaaagcgatgatgatgacaacaattattcagagattaatggccggtctaccgctatcgaaggattggatgaacagaataataaggacccaggtattaaacaatcaggagatcagtgttctgaaggagtgtctaagattaattcatcttctagtccccaagaagctacattatcttctgggagatctgatatatctgggacaggagtatctccctgtgcctctttggatataactgttaatgaattagaagatgcaactgttaagaatagtaataatatgaaaggaaattggccaatcccaaagttgcttgtcaaaccaccaccaagaatgaaatcactttctgactctgttacaccattaaaaggggccaccgacgggaaatcagtcttacctgggatggagattacattgtccgggaagaatggtgcaaccctacctgtacacccatttacacaacctataaaagactcaaatgcagatgtaagcaatgtccgtcaacatgtcccaagtgtgactgatggtcatagtgatgataatgaggaagtacccggtttgcataaagaaactatagacaaagctgatctatctatgcaggacatatacaatttaattcttggatttaaggatgattacaggaaactatcaaataaattggatatgatactagagatgaaacaagatattgataatcttaaaaagagtagtgcaaaaatacaacttgcattatcaacaattgaaggacatctgtccagtgttatgattgctattccaggttcaggtattgatataaatcaagatgagaagaaggatcaattaaactctgacttaaagccattactagggagggaccattgccgtgcatttcgtgaagtcactaatcctttagatgaaacgtcattgaccaacgctccgaccaaacatgttgctaagatcaacaaaaattgcactcttcagaaaatcaataacaatgagacatctgcaattaagtttgtacctaatgatagccatgcaagtatctcgactatcaagtctattgtcaaatcctcaaaccttaatcaagagcttaaagtcaagttactgacaattctatctcaaattaaaggggtagacaatattaaggagttttatgagaaagttatgatattgatcaagaataataactgatcttgactaatcaatagatactacttatcaaatctcgctctgacatcaagtgaattcatctttattaacaagtattaatcttaaataattataaaaaacttaggagttcaggattagtgggtcatatacaatatgactgagatattcaatctggatgaaagttcatggtcagtcaagggaacactggacccattgacgcctgatacttatcctgatgggcgcctagtacccaagattcgggttattgatcccggtctaggtgatcgtaaaagtggaggatatatgtacttactccttcacggtgtcatcgaggacagtgagaccgtcataaatccgaaagggagagcatttggagctttccctttaggcgtagggcaatcaaccgagaacccagaagacttatttaaggaaatattaaccctcaacattgttactcgcaggactgctggcttcaatgaaaaattggtgtattataatactacacctctaaatctactaaccccttggaaaaaagtactagcatatggaagtatctttactgctaatcaggtctgcaataatacaagttctatccctatagacattcctcagaaatttcgacctgtctatttaactgttaccaagttatcggatgatggatattatcagatacctaaaatgatacaggatttcaaatcatcaaactctgttgcatttaacatccttgtgcatctatcaatgggaacaattttacttgactcatctaaaggctctcgagtaggaaaccctgcagaaaatttgatcacattcatgattcatattgggaatttcaaacggaagaataataaagcttattctcccgaatattgtaagaggaaaataatgaggcttggattaattttctcactaggagccattggtggaacaagtttgcatattcgatgcacaggcaaaatgagtaagagattacaagcctacttagggtttaaaagaactttatgttatcctctgatgtatgtcaatgagggtctaaataaaaccttatggagaaatgaatgcaaaattgagaaggttcaagcagtattacagccatcagttccgaatgaatttaagatttatgatgatataatcattgataacacgaatggcctctttaaggttaagtaagctgtgactagtatcaggagttactagtcaaaatcatgtgttgatatccgaattaatagctttaagttgaatatattaaacctgtgataatttaaatttgaaacataattagtatgtagtattgtattaatcagtttataatcttgtttgaggatccaaattataaccctattaggtattgccactccagtcttacaggtaaatctaagcgaatatacaaataattgatattcgggattaaacaatacttgtatattaatccataggtatattagattttactatattcaattattataatgtttattgagttaagctctcatgattataaaaaactaaggattccacataatcacagtttgattgccaattgatgtgtttagtattagttgtgtgaaatattgatattaataaggttaatcaacttttgtacagaagtgaaagtgtaattagatagaaatagattaatccttagtagccgttttgataattgaattgattcttgttttaattctgaattgagattattaatcaccagctcggcataatgtataagattaaggttgtaatcatgggttttttactgttatcagatattacatttgcacaggtaggttgggataatttaacctcaattggagttataagtactaaacaatataactataagataactactttgaatactaatcaactcatggtgatcaaaatggtacccaatatatcatcaattattaactgtactaaacttgaattagcaaaatatagggaactgattacaggaatactgagaccaattaatgaatcattagaattgatgaattcatatatcaacatgagaacaggttcagagagattcataggggctgttatagcaggagtagctctaggggttgcaactgcggcgcagataacatcgggaattgccttacataattcgattatgaataaaaaacagatacaggaattaaggaaagcccttagtactacaaataaggcaattgatgagataaggattgcaggtgaaagaactctgatagctgtccaaggtgtgcaagattacattaacaatgttattatccctatgcaagagaaactccagtgcgatattttagcctcacagctatctattgccctactcagatactatactaatatactgactgtttttggaccaagtataagagatcctattactagtacaatttctatacaagctctcagtcaagcattcaatggtaatctacaggcattgcttgatggattagggtatactggacaagacttacatgatctcatagaaagtagatctatcactggtcaaattattcacgctgatatgactgatttattccttgtattgagaatcaattatccatctattacggatatgcaaggagtggtaatatatgagctgaattctatcacatatcatattggacctgaagagtggtacactattatgcctaatttcatagctgttcagggatttctggtatctaatttcgatgaacgtaaatgttcaattactaaaacaagtatactgtgtcaacagaattcaatttatcctatgtcaaccgaaatgcaaagatgtataaaaggtgagattaaattctgtccaaggtccaaagcaattgggacattagttaatcgatttatattaattaatgggaatctaatggccaattgtttgggtattatctgtagatgttatacctcaggtcaaattataacgcaagacccaaataaattaatcacaattatatcacaagaagaatgtagagaggttggtgttgatgggattcgtataatggtggggcctaaaaaattaccggatgttatctttaatgccagactagaaataggtgtacctatctcattaagcaagctggatgttgggaccgacttggcaattgcttcagctaaactcaataactctaaggcacttttggagcagtctgataaaatcttaaattctatgtctaagttggattctttaaattcacgtatcttaggatctgtctttataattatgataatcttcgtgactgtaattgtgattatttggattatttgtaaaaagtgtagaaataagaggaacaaattaagtgcttctattgaacccctctacatacctccctcttataattcaccccatagcatagttaaatctatttgaaatataagtgtataatctgatataacagatgcagtagaattattaatcaatgataatattattatgataatgattcagttagatgttcattgtatctcataacttaatattgacaaatttcaattagttaaatttattctcttcataatatgtatttgtttaattatcctagattcatgtactgttattaaattggtcatctttaataactaactcagcaatactatcctatacacatgtattagctaataacgatgtaatattgccatttaataataagtacctagtagaatgggaagcattagctgtagtcaatgaaccattacctgctcaattagaaaaaacttaggaatccatgttaatgggagctggccatcatggaatctaataacaacaagtactataaagattcaaaccggtattttagcaagatactagatgagaacaagacggtaaataatcatctgtatagtcttagtataaggataattaccgttatagctattgttgtgagtctaattgcaacaacaataaccatcattaatgctataagcggaaggactactcttaataataatatggacatgctactcaaccaacaagacaagattaataatatcaaggaaatgatatttgatcgtatctatcccctgataaatgccatgagtacagagcttggtcttcacattccaactttattggatgagctgactaaatcaattgatcaaaaaatcaagataatgactccaccacttgaaactacaacatctaatctcaattggtgtatcaaccccccaaatggcattattgtagatcctaaaggttattgtgaaggcttggaactgtcaaaaacttataagttattacttgatcaattagatatgttaagaaagaaatcacttattattaataagaaaagtattaatcagtgtagacttgttgatagttcgaatatcgtctttgcaacagttaatatacaatctacaccgagattcttaaatcttggtcacacagttagtaaccaacgtataacattcggtcaaggaacatatagtagcacttatattataactatacaagaggatggattaactgatgttcagtaccgagtatttgaaataggatatatctcagatcaatttggaaccttcccttctctaatcgtttccagagtactacctgtgcgaatggtacttggaatggaatcttgtacactgaccagtgacaagtttgggggttattttttatgcatgaacattccgacacgctctatatatgattatgtcaacataagagacttaaagtcactatacgtcacaatccctcattatggcaaaattaattacacttactttaattttgggaaagtcagaagcccacatgaaattgataagatttggcttacatcagaaaggggacagatgatttcaggttactttgcagcatttgttacgattacaattagaaattataacaattatccctataaatgcttacataacccgtgtcttgaaagatctgagagttattgcaaaggatggtacaaaaatattacaggtactgatgatgttccaatattagcatatctattagttgaaatgaatgatgaggaaggacccttaattacattggttgagataccaccttacaattatacggctccttctcataattccctttactatgatgataaaattaacaaattaataatgacaacatctcatataggatacattcaaatcaatgaagtgcatgaagtcattgtcggggataatcttaaggctattctcttaaacagattatctgatgaacaccctactcttactgcttgtagatttaatcaggaaattaaagagcgacatatatctgatggattaataatatctaactctgctcttattgatatacaagaacgtatgtatgttacagttaaggctgttccacccataggaaattataacttcacggtagagttgcattcacggtcaaatacatcttacgtagggttgccaaggcagttcaatgctaggtatgacaaactgcatctcgaatgctttgcctgggataggtcttggtggtgcgctttgatacctcaattttcattaagttggaatgaatctctttcagtagatactgccattttcaacttaataaactgtaattaagtttgtggcttgttctagattgatcatttgaataacagttgattaagccaaagttagtaaatacatacattaacctgttcttgaccaagtatatatcccaatccaattataaaaaacttaggactcaaggtgttgatggcaatggagcaatcagattatcaagatattttatatccagaggtacatctcaacagtcctatagttatctctaaattagtgggtattttggagtattctaaggttgttcacaatcagcagttatctgatcacacaatagtcaagaatatacaatttagattgagaaatggattcaatagtccaagaatacaaacactgttagttatgggtgaaattatcaataaaatcaaaaataaatacccaaattatttgcacataccttatcctgaatgtaatcaaaagttatttaggatagctgacccggagttaacatctaaactagaagccctcttggacaaaggtgacacattatatcttaagattaagacagagatcatagcttgtttcgataagttaaaaactaaaatgagcataaccaatgatctgattagtgacaataggcagctaatttcagatctacctataattgtcaagggatctcaatggtttttcccttttttgctctggttctctgttaaaactgagactaggaactgtattcgacaaaatcaaaaaactcgtgttaggtcacaataccgacctcatttgtcagaaactaaaagaattacgctggtcgttactcatgacttgatcacaatatttgaccacgtcaacaaatgtatatatcatctgacttttgagatgttgttgatgtattgtgatgtagtagaagggaggttaatgaccgaagcatctatgagtctagatcacagatttattaacctattgtcgagggtccagtatatgtgggatctattagatgggatgtttgagagtctaggaaatcagctatattcaatcattgcactcttagaacctctctctcttgcctatctacagttgatggatgcagacccacagatacggggtacatttttacaccattgcctttcagagttggaagaactcttatttagtaaattcccttttgatcctgtaatttatgaaaatctaattagtggacttgattacatctatttaacagacgatattcatttaactgctgagatattttctttctttagaagttttggtcatccttatttagaagcacaaaatgcagctagcaatgttaggaaatatatgaatcaacctaaagttatctcataccagactctaatgcaaggacatgcaattttttgtggcattataataaatgggttcagagatcgtcacggagggacatggccacccgtagagctaccacatcatgcatccgctgtaattagaaatgctcagttatctggagaaggattaacacctgagcagtgtgctcaatactggaggtcattttgtggatttaaatttaaatgttttatgccattaagtttagatagcgacctcaccatgtaccttagagacaaggcattatcacctattaagaatgagtgggactctgtgtatgctaaagagtatttaagatacaaccctggcttaccgactagctctcgaagattagtcaatgtatttcttgaagatgataaatttgatccgtacgaaatgattatgtacgtaataaacggtgattatttaagggataatgagttcaatctctcatatagtcttaaagaaaaggagatcaaggaggtaggccgattgttcgctaaaatgacttataaaatgagagcttgtcaggtaatagcagaaaatttaattgcaaatggagttgggaaattttttaaagacaatgggatggcgaaggatgaacataaattaaccaaaacattacataagctggccatttctggtgtacctaaagataattttcaactctatttaagtgaatgttgggaacaagtggtagaacaatgcgtaaccagtacgcaaacaaaaaatcaaattatcagttcacactcaagaaaatcagttgcatcaaagtttccaagatcaaatcccaatgataggggtattctaaatagtggcagacatttgaataaacatccaaaacatccttcaaacaccgaatactatgaaactgtcagtagttttataactactgatctcaagaaatattgcctcaactggcgctatgaatcaagtagtgtgtttgcagaaagactcaatgagatttatgggttaccaggattttttcattggcttcatagaattttggagaaatctgtattatatgttagtgatccatccagtccacctgattttgatcaacatgttgatattgattcagttccaaatgatcatatttttatcaaatacccaatgggtgggatagaaggattttgtcaaaaattatggacaatcagcacaatcccatttttatatttagcagcttttgatacaggggttagaatatcttcgttggttcaaggtgataatcaagcaattgcagtgaccaaaagagttccatcgtcctggagttattcgagaaaaaaagaggagtcaactaaagttacaacacaatattttttaaacttaagacaacgcttacatgatataggtcatgagttaaaggcaaatgagactattatatcttcacacttttttgtttactctaagggtatttattatgatggtatacttctttcacaatcccttaaaagtattgcaagatgtgttttttggtccgagacaattgtcgatgagactaggtcagcttgcagcaatatatccactacccttgctaaagctattgaacggggttatgataaattcgtggcatacgctattaatatatataagactatacaccaggtcttaattgcattatcttttactattaatcccactatgactccggacataacagaacctttttataaaagtttagatttacttaaaaacctcattctgataccagcaccattgggtgggatgaattacatgaatatgagcagattatttgttagaaacataggtgatcccattacagcttcatttgctgacatcaagcgtatgatcgaatgcgggttattagggcacaatgttctctcacaaataatgtatcagaaatgtggtacctcgaaatacttagattgggctagtgacccttattccataaatcttccttatagtcaaagcatgaccaaagtattaaaaaatataaccgcgagatatgttctcatgcacagtcctaaccctatgctaaaagatttattccatgagaagtcacaagaagaagatgagattcttgctgaatttttgctggatcgtcagttaataatccctagagctgcacatgaaattttatcgaattcagtaacaggagctagagagtcgattgcagggatgcttgatactactaaaggacttattcgagccagtatgtcaagaggtggtctgacatcttcacttgtgttgaaattgtcaacatatgattatcaacaatttagaacatgccttgaatggctttatgcccctaccacaggaatagcagtaagtgctgattcttgttcagtttttttagccagagctattcgaaaaaggatgtgggttcacctgactaaaggaagagaaatttatggcctagaagtgcctgatatattagaatgtatgcagagcaatgtaattgttgatcatgaagattgttattcatgtattcaaggatcaagatactacacatggttttttgtaccttctaattgtcagcttgatcagattaacaagtctacaaattctctacgggttccttacattggctctactacagaggaaagaagtgacatgaaattatcatacgtcagatcccctagtaggccacttaaggcagcagtccgaattgcagcagtctacacatgggcatacggtgatgacgatctgtcttggcgtgaggcttggtacttggcaaggactagggcaaatgttactttcgatgagcttaaattagtaacacccatagctacctctacgaacttggcacatagattaagggacaggagtactcaagttaagtattcaggaacttcattagtaagagtggcacgctatacaacaatatccaatgataatatgtcatttgtcattaatgacaaaaaggtagatactaattttgtctatcaacagggcatgttattgggtttgagtatcctagaatatatatttagatactgtaaaagtactggtcaatcaaatactgtagttcacttgcatgcagatgttaattgttgcataatccaaatgacagatcaaccttatactccaagcttaacgaaaaaattacctgagattaaacctattaataataagttgatttatgatccagctcctataattgatactgatgcagctaggttatattctcagaagtacttatcacacctgatagattttccaaattggtcaatgaatcagctaaatgtagttttagcaaaagtagttgcaatatctattgtggacttgataactaaagcgagtaaagatcatctcaatgaaattatggcagttgttggagatgatgacattaatagctttataacagaatttttgctagttgatccgaggctatttacattgtacttaggtcaatacacgtcacttcaatgggcatatgaaattcattatcaccgacccgtaggcaaataccagatggcagaagtgttacacactttactgtcaagagcaagtaaaggtatatttaatatattaactaatgcttttagtcatcctagagtttacaaaagattttgggaatgtggattactggagcctatttatggaccatacatagggagccaaaatttatatagtacagtaattgattacctttacaatgcttatataacttatttagatgcttatctatctgatcatatcgaagatgcagacatagtaatatgtgagacagaagaaacttgtctagctaataggattgataactatcaaggtaggcatctagccgtacttattgatctttattgtgattctactaggtgtcctaatataaaagggtcagacacaatcatgcgaaactcaattctcaaatcttttattgataatgagagaaggacaagtccattaggtctaacatggaatcttgatccattactcatagatcatttcagttgttcaattacttatctgaggagaggtattattaaacagattaggctaaggtttgatccaaacatatctattgagttggttaaattggcaaaacctgaagtgattcatcaaggaccaaaaataccgtcttcttgggcccttatagatattaatcctgaggtcaatgatcttaatacagttttcggagaattaaatagtaaatggaaagatattcctattggacaaattagaattcaaaattatgagatccatgcttaccgaagaattggagttaattcaactgcatgttataaagcattggaaatgctatctgtactaacccggtttatgtctaacccagcaggagctttgtttttaggagagggtgcagggtcaatgttagttacctatcgtgcgtttatcccgttcaagagaatttattataatagtggaatttctatacaaaatattcaaagccaaagagaactaagtctatacccatctgaagtagccttggttgataataaaaatcgtttgaccagtgatcctgatatcaaagtcttatttaatggcaagccagaatccacgtgggttgggaatatagactgctttgcttatattctgagtcatattgaaacttctagtttaacattaatccacagtgatattgaatctagcttgagtaaaacaaagaataagattcttgaggagctttgccatattctatcaatggcactgattttaggaaagattggatctgtattagttattaagctgttaccacgggttggtgactacacatattcattttgcaagtatgcgtcagaattctaccaacagaatttttttattttacctagatttagcaacatgtcatcatctgaaatttactacgttggagttcatttaaataccaatagactggttgatccagataggattgtgcaatatataatcaggaatctccaatctactccagttactttcttatcttacattttggaaactaaatatagaaataatatggttacaaattatgggctctgcttgtctgatggacataaaagcgattacttgtcatcaatcaccaagatagaaaatgttcttttatcatgtggattggaattgaatggacctaagattatacagcaattatctggacatgactacgccaatggagagattagcttagaatcaagtataatggtactggttagagaatatctaaatgcaactatccaaggtcgggaaacactaggtcttttttcaccttaccctgtgttacatgagagtcagttaagagaaattaacaggtgcattgcattgaagtatgttgtatatttacttttttactcaacctctgtaggatctagtagacaaatcatgagcaatctcagaaaaggagtattaatgtatgacttaagagatgagtttttcatggaaaggttatcaacaaatttcaagaaaaaaataatgtcacaagaggttaaaactacatggatctttaatattgatgtaccaacaagaaaagctctgtataaattagttggttattcacttatcattaatcacgtataacaagtgtattgagttggtaatattctagatgaacaagtataggtttatgtacagtaagtgattaaatattagattcaggtagataaacttcctaatagtgtatcctatagataacctaaggctatttaatgttagattaattagaaaaaacttcttgaattatgatagacttcaacccctggctaagacttatcatttaaaattataaccaagttgtcctgataatatcagatctcattaattacttgatagcgtaatataacaggtgcatgatgatcctttattactcatatacctgttattaagctcctgttcaaattatcccctatttaagttgccttttaaattacctaatatgttttgtaatgagaaacattgatacatacaaagctaaagaagcctgattttatctaaggttgtatctaattgttgtcaatttataattcggaatatctgggccctaaacctcctccaaatatactaaaaggttttaaaaaaacaaaaaaggtttcttacttattgtacggacctatagctttcttttgtctggt

SEQ ID NO: 2 - DNA, 16045 bp, Feline paramyxovirus type 2
  misc_feature: FPaV-2 "TV25 strain" full genome sequence; given as a DNA sequence that correspond to the positive RNA-strand into which the negative RNA strand viral genome is transcribed, i.e. it comprises the ORFs in 5' to 3' direction like an mRNA
accagacaaagatgtctgtgacctattctaacggttagattattacttgatatttaggaataacgattccattagtcaggtaagggagaggaatcagttattctataatggctagtttactcaggtcacttgcggcattcaagaaacacagagaacaaccaactgttccttctgggtcaggagggacgatcaaaggattaaaaaatacaattattgtgcctgttcctggagatacagtcatcactaccagatcgaacttactgttcagattagtctacataattggtaatccagatacacctttaagcacttcaacaggggcaataatatcattgttgacattatttgttgaatctccaggtcaattaattcaaagaatcgctgatgatcctgatgctgtttttaaattagtagaggtggttcctgaggttggtaatcctggagaattaacttttgcatctagaggaattaacttggataaacaagctcaacaatactttagattggctgagaaaaatgatcaaggatattatgtaagtttggggtttgaaaatccaccaaatgatgatgatataacgtcaagtcctgaaatcttaaattatattttagcatctgtacttgcacagatctggattctcctagctaaggctgtaactgctccagacacaggtggtgaggctgaaaatcgtaggtggattaaattgatgcaacaacgcagagtggatggtgagcttagattaagtaaaggatggttggacttagtgaggaataaaatcgcatcggatatcacaattagaaggtttatggtagcattagttcttgacattaaacgttctcctggaacaagaccaagaattgctgaaatgatttgtgatatagacaattatattgtggaggccggactggcaagttttctgttaactatcaaatttggtatagaaacacgttacccagcattggcgttacatgagttttcgggggaattagccactattgaaggactcatgaaattgtaccagtctatgggagaaatggcaccatacatggtcattctagagaattcgatccagactaggtttagtgctgggtcttatccgttactctggagctatgctatgggtgttggtgtagaacttgagagatcaatgagtggattaaacttcacaagaagtttctttgatcctacgtacttcaggttgggtcaggagatggtaagaaggtcttcaggaatggttaatagctcatttgctaaagaacttggactatctgaacatgaaacacaacttgttagccagatcattaactctggtggtgaatcaggtataccgaaatttgatggatttagagcaaacccaacaacatttctaggggctaaggacaacatcactgataggagtgaagatccattgattgcaattccagggtcatcaggacaaccattgccaggtcatgaccccaatatctcaggtgactcatatagaattgatagtagcactaaagacacgaacaatatatcagatggaggaacaaatccaagtcatgatgtttccaattctgctatggaagagctgagaagattggtagagtctaccaacaagattgatacaaagaaatctgaaagcccaggcattgttaatcattacaacgatactgaccttctgagataataaggatatattcaggtagatctttacagaatttaaattaagaaaaacttaggacctcaaggttcacactcctctggccttcatcagaactcggccaattcctcactcactccatgtcagcagaacaaatccaacaagttagacatggccttgaatccttgcaagagatcaaaaacaaccctccaccctctcaagatgtcaatcttgccagggaaatttacgaatccattaaacaaacaggaacaccttcaacacaaggagggaccattacaggaaataatactacgtcagggtgtgacaattactcaatgcatagccagggatcaggtccttctgtttcaggtgctgacaagaatatcgagagacttactggacccgattattcagaattatgggatccagaaggtaacctctgcatgctattcgaaagcgatgatgatgacaacaattattcagagattaatggccggtctaccgctatcgaaggattggatgaacagaataataaggacccaggtattaaacaatcaggagatcagtgttctgaaggagtgtctaagattaattcatcttctagtccccaagaagctacattatcttctgggagatctgatatatctgggacaggagtatctccctgtgcctctttggatataactgttaatgaattagaagatgcaactgttaagaatagtaataatatgaaaggaaattggccaatcccaaagttgcttgtcaaaccaccaccaagaatgaaatcactttctgactctgttacaccattaaaaggggccaccgacgggaaatcagtcttacctgggatggagattacattgtccgggaagaatggtgcaaccctacctgtacacccatttacacaacctgtaaaagactcaaatgcagatgtaagcaatgtccgtcaacatgtcccaagtgtgactgatggttatagtgatgataatgaggaagtacccggtttgcataaagaaactatagacaaagctgatctatctatgcaggacatatacaatttaattcttggatttaaggatgattacaggaaactatcaaataaattggatatgatactagagatgaaacaagatattgataatcttaaaaagagtagtgcaaaaatacaacttgcattatcaacaattgaaggacatctgtccagtgttatgattgctattccaggttcaggtattgatatgaatcaagatgagaagaaggatcaattaaactctgacttaaagccattactagggagggaccattgccgtgcatttcgtgaagtcactaatcctttagatgaaacgtcattgaccaacgctccgaccaaacatgttgctaagatcaacaaaaattgcactcttcagaaaatcaataagaatgagacatctgcaattaagtttgtacctaatgatagctatgcaagtatctcgactatcaagtctattgtcaaatcctcaaaccttaatcaagagcttaaagtcaagttactgacaattctatctcaaattaaaggggtagacaatattaaggagttttatgagaaagttatgatattgatcaagaataataactgatcttgactaatcaatagatactacttatcaaatctagctctgacatcaagtgaattcatctttattaacaagtattaatcttaaataattataaaaaacttaggagttcaggatcagtgggtcatatacaatatgactgagatattcaatctggatgaaagttcatggtcagtcaagggaacactggacccattgacgcctgatacttatcctgatgggcgcctagtacccaagattcgggttattgatcccggtctaggtgatcgtaaaagtggaggatatatgtacttactccttcacggtgtcatcgaggacagtgagaccgtcataaatccgaaagggagagcatttggagctttccctttaggtgtagggcaatcaaccgagaacccagaagacttatttaaggaaatattaaccctcaacattgttactcgcaggactgctggcttcaatgaaaaattggtgtattataatactacacctctaaatctactaaccccttggaaaaaagtactagcatatggaagtatctttactgctaatcaggtctgcaataatacaagttctatccctatagacattcctcagaaatttcgacctgtctatttaactgttaccaagttatcggatgatggatattatcagatacctaaaatgatacaggatttcaaatcatcaaactctgttgcatttaacatccttgtgcatctatcaatgggaacaattttacttgactcatctaaaggctctcgagtaggaaatcctgcagaaaatttgatcacattcatgattcatattgggaatttcaaacggaagaataataaagcttattctcccgaatattgtaagaggaaaataatgaggcttggattaatcttctcactaggagccattggtggaacaagtttgcatattcgatgcacaggcaaaatgagtaagcgattacaagcctacttagggtttaaaagaactttatgttatcctctgatgtatgtcaatgagggtctaaacaaaaccttatggagaaatgaatgcagaattgagaaggttcaagcagtattacagccatcagttccgaatgaatttaagatttatgatgatataatcattgataacacgaatggcctctttaaggttaagtaagctgtgactagtatcaggagttactagtcaaaatcatgtgttgatatccgaattaatagctttaagttgaatatattaaacctgtgataattcaaatttgaaacataattagtatgtagtattgtattaatcagtttgtaatcttgtttgaggatccaaattataacctattaggtattgccactccagcttacaggtaaatctaagcgaatatacaaataattgatattcgggattaaacaatacttgcatattaatccataggtatattagattttactatattcaattattataatgtttattgagttaagctctcatgattataaaaaacttaggattccacataatcacagtttgattgccaattgatgtgtttagtattagttgtgtgaaatattgatattaataaggttaatcaacttttgtacagaagtgaaggtgtaattagatagaaatagattaatccttagtagccgttttgataattgaattgattcttgttttaattctgaattgagattattaatcaccagctcggcataatgtataagattaaggttgtaatcatgggttttttactgttatcagatattacatttgcacaggtaggttgggataatttaacctcaattggagttataagtactaaacaatataactataagataactactttgaatactaatcaactcatggtgattaaaatggtacccaatatatcatcaattattaactgtactaaacttgaattagcaaaatatagggaactgattacaggaatactgagaccaattaatgaatcattagaattgatgaattcatatatcaacatgagaacaggttcagagagattcataggggctgttatagcaggagtagctctaggggttgcaactgcggcgcagataacatcgggaattgccttacataattcgattatgaataaaaaacagatacaggaattaaggaaagcccttagtactacaaataaggcaattgatgagataaggattgcaggtgaaagaactctgatagctgtccaaggtgtgcaagattacattaacaatgttattatccctatgcaagagaaactccagtgcgatattttagcctcacagctatctattgccctactcagatactatactaatatactgactgtttttggaccaagtataagagatcctattactagtacaatttctatacaagctctcagtcaagcattcaatggtaatctacaggcattgcttgatggattagggtatactggacaagacttacatgatctcatagaaagtagatctatcactggtcaaataattcacgctgatatgactgatttattccttatattgagaatcaattatccatctattacggatatgcaaggagtggtaatatatgagctgaattctatcacatatcatattggacctgaagagtggtacactattatgcctaatttcatagctgttcagggatttctggtatctaatttcgatgaacgtaaatgttcaattactaaaacaagtatactgtgtcaacagaattcaatttatcctatgtcaaccgaaatgcaaagatgtataaaaggtgagattaaattctgtccaaggtccaaagcaattgggacattagttaatcgatttatattaattaatgggaatctaatggccaattgtttgggtattatttgtagatgttatacctcaggtcaaattataacgcaagacccaaataaattaatcacaattatatcacaagaagaatgtagagaggttggtgttgatgggattcgtataatggtgggacctaaaaaattaccggatgttatctttaatgccagactagaaataggtgtacctatctcattaagcaagctggatgttgggaccgatttggcaattgcttcagctaaactcaataactctaaggcacttttggagcagtctgataaaatcttaaattctatgtctaagttggattctttaaattcacgtatcttaggatctgtctttataatgatgataatctttgtgattgtaattgtgattatttggattatttgtaagaagtgtagaaataagaggaacaaattaagtgcttctattgaacccctctacatacctccctcttataattcaccccatagcatagttaaatctatttgaaatataagtgtataatctgatataacagatgcagtagaattattaatcaatgataatattattatgataatgattcagttagatgttcattatatctcataacttaatattgacaaatttcaattagttaaatttattctcttcataatatgtatttgtttaattatcctagattaatgtattgttattaaactggtcatctttaatacctaactcagcaatactatcctatacacatgtattagctaataacgatgtaatattgccatttaataataagtacctagtagaatgggaagcattagctgtagtcaatgaatcattatctgctcaattagaaaaaayttaggaatccatgttaatgggagttggccatcatggagtctaataacaacaagtactataaagattcaaaccggtattttagcaagatactagatgagaacaagacggtaaataatcatctgtatagtcttagtataaggataattaccgttatagctattgttgtgagtctaattgcaacaacaataaccatcattaatgctataagcggaaggactactcttaataataatatggacatgctactcaaccaacaagacaagattaataatatcaaggaaatgatatttgatcgtatctatcccctgataaatgccatgagtacagagcttggtcttcacattccaactttattggatgagctgactaaatcaattgatcaaaaaatcaagataatgactccaccacttgaaactacgacatctaatctcaattggtgtatcaaccccccaaatggcattattgtagatcctaaaggttactgtgaaggcttggaactgtcaaaaacttataagttattacttgatcaattagatatgttaagaaagaaatcacttattattaataagaaaagtattaatcagtgtagacttgttgatagctcgaatatcatctttgcaacagttaatatacaatctacaccgagattcttaaatcttggtcacacagttagtaaccaacgtataacattcggtcaaggaacatatagtagcacttatattataactatacaagaggatggattaactgatgttcagtaccgagtatttgaaataggatatatctcagatcaatttggaaccttcccttctctaatcgtttctagagtactacctgtgcgaatggtacttggaatggaatcttgtacactgaccagtgacaagttcgggggttattttttatgcatgaacattccgacacgctctatatatgattatgtcaacataagagacttaaagtcactatacgtcacaatccctcattatggcaaaattaattacacttactttaattttggaaaagtcagaagcccacatgaaattgataagatttggcttacatcagaaaggggacagatgatttcaggttactttgcagcatttgttacgattacaattagaaattataacaattatccctataaatgcttacataacccgtgtcttgaaagatctgagagttattgcaaaggatggtacaaaaatattacaggtactgatgatgttccaatattagcatatctattagttgaaatgaaggatgaggaaggacctttaattacactggttgaaataccaccttacaattatacggctccttctcataattccctttactatgatgataaaattaacaaattaataatgacaacatctcatataggatacattcaaatcaatgaagtgcatgaagtcattgtcggggataatcttaaggctattctcttaaacagattatctgatgaacaccctactcttactgcttgtagatttaatcaggaaattaaagagcgacatatatctgatgggttaataatatctaactctgctcttattgatatacaagaacgtatgtatattacagttaaggctgttccacccataggaaattataacttcacggtagagttgcattcacggtcaaatacatcttacgtagggttgccaaggcagttcaatgctaggtatgacaaactgcatctcgaatgctttgcctgggataggtcttggtggtgcgctttgatacctcaattttcattaagttggaatgaatctctttcagtagatactgccattttcaacttaataaactgtaattaagtttgtggcttgttctagattgatcatttgaataacagttgattaagccgaagttagtaaatacatacattaacctgttcttgaccaagtatgtatcctaatccaattataaaaaacttaggactcaaggtgttgatggcaatggagcaatcagattatcaagatattttatatccagaggtacatctcaacagtcctatagttatctctaaattagtgggtattttggagtattctaaggttgttcacaatcagcagttatctgatcacacaatagtcaagaatatacaatttagattgagaaatggattcaatagtccaagagtacaaacactgttagttatgggtgaaattatcaataaaatcaaaaataaatacccaaattatttgcacataccttatcctgaatgtaatcaaaagttatttaggatggctgacccggagttaacatctaaactagaagccctcttggacaaaggtgacacattatatcttaagattaagacagagatcatagcttgtttcgataagttaaaaactaaaatgagcataaccaatgatctgattagtgacaataggcagctaatttcagatctacctctaattgtcaagggatctcaatggtttttcccttttttgctctggttttctgttaaaactgagactaggaactgtattcgacaaaatcaaaaaactcgtgttaggtcacaataccgacctcatttgtcagaaactaaaagaattacgctggtcgttacccctgacttgatcacaatatttgaccacgtcaacaaatgtatatatcatctgacttttgagatgttgttgatgtattgtgatgtagtagaagggaggttaatgaccgaagcatctatgagtctagatcacagatttattaacctattgtcgagggtccagtatatgtgggatctattagatgggatgtttgagagtctaggaaatcagctatattcaatcattgcactcttagaacctctctctcttgcctatctacagttgatggatgcagacccacagatacggggtacatttttacaccattgcctttcagagttggaagaactcttatttagtaaatccccttttgatcctgtgatttatgaaaatctaattagtggacttgattacatctatttaacagacgatattcatttaactgctgagatattttctttctttagaagttttggtcatccttatttagaagcacaaaatgcagctagcaatgttaggaaatatatgaatcaacctaaagttatctcataccagactctaatgcaaggacatgcaattttttgtggcattataataaatgggttcagagatcgtcacggagggacatggccacctgtagagctaccacatcatgcatccgctgtaattagaaatgctcagttatctggagaaggattaacacctgagcagtgtgctcaatactggaggtcattttgtggatttaaatttaaatgttttatgccattaagtctagatagcgacctcaccatgtaccttagagataaggcattatcacctattaagaatgagtgggattctgtgtatgctaaagagtatttaagatacaaccctggcttaccgactagctctcgaagattagtcaatgtatttctagaagatgataaatttgatccgtacgaaatgattatgtacgtaataaacggtgattatttaagggataatgagttcaatctctcatatagtcttaaagaaaaggagatcaaggaggtaggccgattgttcgctaaaatgacttataagatgagagcttgtcaggtaatagcagaaaatttaattgcaaatggagttgggaaattttttaaagacaatgggatggcgaaggatgaacataaattaaccaaaacattacataagctggctatttctggtgtacctaaagataattctcaactctatttaagtgaatgttgggaacaagtggtagaacaatgcgtaaccagtacgcaaacaaaaaatcaaattatcagttcacactcaggaaaatcagttgcatcaaagttttcaagatcaaatcccaatgataggggtattctaaatagtggtagacatttgaataaacatccaaaacatccatcaaacaccgaatactatgaaactgtcagtagttttataactactgatctcaagaaatattgcctcaactggcgctatgaatcaagtagtgtgtttgcagaaagactcaatgagatttatgggttaccaggatttttccattggcttcatagaattttggagaaatctgtattatatgttagtgatccatccagtccacctgattttgatcaacatgtcgatattgattcagttccaaatgatcatatttttatcaaatacccaatgggtgggataaaaggattttgtcaaaaattatggacaatcagcacaatcccatttttatatttagcagcctttgatacaggggttagaatatcttcgttggttcaaggtgataatcaagcaattgcagtgaccaaaagagttccatcatcctggagttattcgagaaaaaaagaggagtcaactaaagttacaacacaatattttttaaacttgagacaacgcttacatgatataggtcatgagttaaaggcaaatgagactattatatcttcacacttttttgtttactctaagggtatttattatgatggtatacttctttcacaatcccttaaaagtattgcaagatgtgttttttggtccgagacaattgtcgatgagactaggtcagcttgcagcaatatatccactacccttgctaaagctattgaacggggttatgataaatttgtagcatacgctattaatatatataagactatacaccaggtcttaattgcattatcttttactattaatcccactatgactccggacataacagaacctttttataaaagtttagatttacttaaaaacctcattctgataccagcaccattgggtgggatgaattacatgaatatgagcagattatttgttaggaacataggtgatcccattacagcttcatttgctgacatcaagcgtatgatcgaatgcgggttattagggcacaatgttctctcacaaataatgtatcagaaatgtggtacctcgaaatacttagattgggctagtgacccttattccataaatcttccttatagtcaaagcatgaccaaagtattaaaaaatataaccgcgagatatgttctcatgcatagtcctaaccctatgctaaaagatttattccatgagaagtcacaagaagaggatgagattcttgctgaatttttgctggatcgtcagttaataatccctagagctgcacatgaaattttatcgaattcagtaacaggagctagagagtcgattgcagggatgcttgatactactaaaggacttattcgagccagtatgtcaagaggtggtctgacatcttcacttgttttgaaattgtcaacatatgattatcaacaatttagaacatgccttgaatggctttatgcccctaccacaggaatagcagtaagtgctgattcttgttcagtttttttagccagagctattcgaaaaaggatgtgggttcacctgactaaaggaagagaaatttatggcctagaagtgcctgatatattagaatgtatgcagagcaatgtaattgttgatcatgaagattgttattcatgtattcaaggatcaagatactacacatggttttttgtaccttctaattgtcagcttgatcagattaacaagtctacaaattctctacgggttccttacattggctctactacagaggaaagaagtgacatgaaattatcatacgtcagatcccctagtaggccacttaaggcagcagtccgaattgcagcagtctacacatgggcatacggtgatgacgatctgtcttggcgtgaggcttggtacttggcaaggactagggcaaatgttactttcgatgagcttaaattagtaacacccatagctacctctactaacttggcacatagattaagggacaggagtactcaagttaagtattcaggaacttcattggtaagagtggcacgctatacaacaatatccaatgataatatgtcatttgttattaatgacaaaaaggtagatactaattttgtctatcaacagggcatgttattgggtttgagtatcctagaatatatatttagatactgtaaaagtactggtcaatcaaatactgtagttcacttgcatgcagatgttaattgttgcataatccaaatgacagatcaaccttatactccaagcttaacgaaaaaattacctgagattaaacctattaataataaattgatttatgatccagctcctataattgatactgatgcagctaggttatattctcagaagtacttatcacacctgatagattttccaaattggtcaatgaatcagctaaatgtagttttagcaaaagtagttgcaatatctattgtggacttgataactaaagcgagtaaagatcatctcaatgaaattatggcagttgttggagatgatgacattaatagctttataacagaatttttgctagttgatccgaggctatttacattgtacttaggtcaatacacgtcacttcaatgggcatatgaaattcattatcaccgacccgtaggcaaataccagatggcagaagtgttacacactttactgtcaagagcaagtaaaggtatatttaatatattgactaatgcctttagtcatcctagagtttacaaaagattttgggaatgtggattactggagcctatttatggaccatacatagggagccaaaatttatatagtacagtaattgattacctttacaatgcttatataacttatttagatgcttatctatctgatcatatcgaagatgcagacatagtaatatgtgagacagaagaaacttgtctagctaataggattgataactatcaaggtaggcatctcgccgtacttattgatctttattgtgattctactaggtgtcctaatataaaagggtcagacacaatcatgcgaaactcaattctcaaatcttttattgataatgagagaaggacaagtccattaggtctaacatggaatcttgatccattactcatagatcatttcagttgttcaattacttatctgaggagaggtattattaaacagattaggctaaggtttgatccaaacatatctattgagttggttaaattggcaaaacctgaagtgattcatcaaggaccaaaaataccgtcttcttgggcccttatagatattaatcctgaggtcaatgatcttaatacagttttcggagaattaaatagtaaatggaaagatattcctattggacaaattagaattcaaaattttgagatccatgcttaccgaagaattggagttaattcaactgcatgttataaagcattggaaatgctatctgtactaactcggtttatgtctaacccagcaggagctttgtttttaggagagggtgcagggtcaatgttagttacctatcgtgcgtttatcccgttcaagagaatttattataatagtggagtttctatacaaaatattcaaagccaaagggaactaagtctatacccatctgaagtagccttggtcgataataaaaatcgtttgaccagtgatcctgatatcaaagtcttatttaatggcaagccagaatccacgtgggttgggaatatagactgctttgcttatattctgagtcatattgaaacttctagtttaacattaatccacagtgatattgaatctagcttgagtaaaacaaagaataagattcttgaggagctttgccatattctatcaatggcactgattctaggaaagattggatctgtattagttattaagctattaccacgggttggtgactacacatattcattttgcaagtatgcgtcagaattctaccaacagaatttcttcattttacctagatttagtaacatgtcatcatctgaaatttactacgttggagttcatttaaataccaatagactggttgatccagataggattgtgcaatatataatcaggaatctccaatctactccagtcactttcttatcttacattttggaaactaaatatagaaataatatggttacaaattatgggctctgtttgtctgatggacataaaagcgattacttgtcatcaatcaccaagatagaaaatgttcttttatcatgtggattggaattgaatggacctaagattattcagcaattatctggacatgactacgccaatggagagattagcttagaatcaagtataatggtactggtcagagaatatctaaatgcaactatccaaggtcgagaaacactaggtcttttttcaccttaccctgtgttacatgagagtcagttaagagaaattaacaggtgcattgcattgaagtatgttgtatatttacttttttactcaacctctgtaggatctagtagacagatcatgagcaatctcagaaaaggagtattaatgtatgacttaagagatgagtttttcatggaaaggttatcaacaaatttcaagaaaaaaataatgtcacaagaggttaaaactacatggatctttaatattgatgtaccaacaagaaaagctctgtataaattagttggttattcacttatcattaatcacgtataacaagtgtattgagttggtaatattctagatgaacaagtataggtttatgtacagtaagtgattaaatattagattcaggtagataaacttcctaatagtgtatcctatagataacctaaggctatttgatgttagattaattagaaaaaacttcttgaattatgatagacttcaacccctggctaagacttatcatttaaaattataaccaagttgtcctgataatatcagatctcattaattacttgatagcgtaatataacaggtgcatgatgatcctttattactcatatacctgttattaagctcctgttcacattatcccctatttaagttgccttttaaattacctaatatgtttagtaatgagaaacattgatacatacaaagctaaagaagcctgattttatctaaggttgtatctaattgttgtcaatttataattcggaatatctgggccctaaacctcctccaaatatactaaaaggttttaaaaaaacaaaaaaggtttcttacttattgtacggacctatagctttcttttgtctggt

SEQ ID NO: 3 - DNA, 16050 bp, Feline Morbillivirus
  misc_feature: FeMoV "Lapön strain" full genome sequence; given as a DNA sequence that correspond to the positive RNA-strand into which the negative RNA strand viral genome is transcribed, i.e. it comprises the ORFs in 5' to 3' direction like an mRNA
accagacaaagatgtctgtgacctattctaacgacaagactattactaaatatttaggaataacgattccattggtgaggcgaggaggaggaatcagacattccacaatgtcgagtctactaaggtcacttgctgcatttaaaagacatagggagcaaccaactgcaccgtcaggctcaggtggtacaattaaaggattgaagaatacaattattgttccagttccaggggatacagtaattactacgaggtctaacttgttatttagattagtttatataataggcaatccagatacacctttaagtacctcaacgggagcaataatatcattgctgaccctatttgttgaatcccccggtcaattaattcaaaggattgctgatgatcctgacgcagtttttaaattagtagaagtcattcctgaagtcggtaatcctggagagctgacttttgcatctcgaggaattaatttggataagcaagctcaacaatatttcaaactggctgaaaaaaatgatcaggggtattacgttagcttaggatttgagaacccaccaaatgatgacgatataacatctagtcctgagatatttaattatattctggcatctgtacttgcacaggtttggattcttctggcaaaagctgttactgccccagataccgctgctgaggctgaaaaccgtagatggattaagttgatgcagcaacgtagagtggatggtgaactaagattgagcaaaggatggctggatctggtgaggaacaagattgcatcagatattacaataagacgattcatggtagcattagtccttgatatcaaacgttcccccggaacaagaccaagaatagctgagatgatttgtgatattgataattatattgtagaagcagggcttgcaagctttttgttgactatcaaatttggcatagaaacacgttacccagcattggcattacatgaattttctggagaactagctaccattgaggggcttatgaaattgtaccaatctatgggggaaatggcaccttacatggtaattctggaaaattcaatccaaaccaggttcagtgcagggtcttatcctctgttatggagttatgctatgggtgttggcgtagagcttgaaagatcaatgggtggacttaattttactaggagtttctttgatcctacatatttcagacttggtcaggagatggtgcgaagatcttcagggatggttaatagttcatttgcaagagaacttgggttgtctgaacatgagacacaacttgtcagccaaattgtcaattctggaggtgaatctggtatacctaagtttgatggattcagagcaaatcctacaacttttctaggagccaaggacaacataaatgatggaggtgaggaccagtcaaattcagtatcaggattgcctggaccaatattgccaagtcatgacttgaatctgtcaggtgattcatatgggaatgatagtggtatgaaaaatgtcaacgacagactaaatgaaggagtaagtccagaccatgatgtttctagctctgccatggaagaattaaggagattggttgagtctactaacagaattgacactaaaaagccagaggctccaggtgttactaaccattacaatgatactgaccttctgaaataacatgggtatcatctatttgattattatacaacttaaattaagaaaaacttaggacctcaaggttcacaactgttgacagctcaccaggaaacaatcaactccttacccaccacatgtcctctcaccaaatccaacaggttaaacatggcctcgaatctttacaagagatcaaaaacaaccctccatcttcccaagatgtcaatcttgccagggagatttacgaatccattaaacaaacaggaacaccttcagtgcaaggaggagccattacgggagataatactacgccagggggtaacaattacacaatgtatagccaaggaccaagtccttctattccaagtgttaacaagaatatcgaaggacttactggatccgatcattcaggactatgggatccagaggataacctctgcatgttattcgaaagcgatgatgatgaaaaccattattcagagattaatggccggccttccactatcgaaagattggatgaacaggataatgagaacccaagtattaaacaaccaggaaatcaatgtactgaaggagtgtttaagactgattcatcttctaattcccaagaaactacactacctgttgggagatctgatatacctgggacaggaatatcaacctgtgcctctttggatataaccgtaaatgaactcgaggatgcaactgtaagaaatagcgacaatatgaagggaaactggccaataccaaagttacttgttaagccaccacccagggcaaaatcaagcgttgatcatagcaatccattaaaaggggccacaggagggaaattagtcttacctgggatggagactacattgtccgggaagagtggtgtaaccccatctgtgcacctatctactcaacctgtaaacgacttcaatgtaaatgtaagcaatgcccgtcaacctgccccaaatgtgaataatgatcacagtgacagtggggtaatagtgcccaacttacataaagacattgaagataagtctgaaatatccattcaagatatatacaacttaatacttgggtttaaggatgattatagaaaattgtctaataaactggatatggtattagagatgaaacaagatattgacaatcttaaaaagagtagtgctaaattacaattggcattatcaactattgagggacatctatctagtgttatgatcgctattccagggtcaggtattgattccaccggggatgagaaaaaggatcagatgaacactgacttaaagccgttattggggagggatcattgcagagcatttcgagaagttaccagtcctttagatgagatgtcattagccaattctcccacaaaacatgttgctaaaataaacaaaaactgcacccttcagaaaatcaataagaatgaaacatctgcaatcaaatttgtccccaatgatagtcatgcaagcacatcaaccatcagatcaatcatcagatcatccaatcttgatcaggatttgaaaacgaaactactcacaattctatctcagattcgggggatagataatattaaggaattttatgaaaaagtcatgatactaataaagaataggaactaaacatcaccattctacatgcactactggttgtgattatcctcaatagaatctggtacaattcatttatatgcttattgttttaaaacaattataaaaaacttaggagctaaaggttattcagtcggatacaacatgactgagatattcaatcttgatgaaagctcatggtcagtcaaaggaacacttgatccactaacccctgatacctatcctgatgggcgacttgtacctaaagtccgggtaatcgatccaggtttaggagatcgcaagagtggagggtatatgtatctacttcttcatggtgtcatagaagatagtgaaaccatggttagcccgaaaggaagagcatttggggcgttcccattaggagtaggtcagtcaactgaaaacccagaagatttgtttaaagaagtattaaccctcaacattgtaactcgtaggactgctggctttaatgaaaaattagtttattataataccacgcctctacacttattgactccctggaagaaagtgttggcgtatgggagcattttcaatgctaatcaggtctgcagtgatacaagttctatcccgatagatattccacaaaaatttagacctgtatacttgactattacaaaattatctgacgatggctattatcagataccgaagatgatccaagatttcaaatcatcaaattctgttgcatttaatatccttgtgcatttatcaatgggcacaactttaattgaccaatccaaagaccctcgattaagaagtgctccagaaactatgatcacattcatgattcatattggaaatttcaaacggaagagtaacaaatcttattctcctgaatactgcaagagaaaaataataagacttggtttgatattctcattaggtgcaattggcggcacaagcttacatattagatgtacaggtaagatgagcaaacggctacaggcttatctaggattcaaaaggactctatgttaccccctgatgtatgggaatgaagggttgaataaaactctggggagaaatgaatgtaaaatagaaaaggttcaagcggttctacagccatcagttccaaatgaattcaagatatacgatgatgtcattattgacaataccaatggtcttttcaagattaagtaggctataataatgataaacagttacaaaatgatatcatgtttggaagtgcatactgataattgtgaattaaatatactggattaattacaatgtatggttggaatctagtcaatatgtgggttaatagttaatcatctattagctttatttgtcattcttattttaaactgtttaatttaaagatatcaaaatgtaatgaattcagcattactaaatcaacatttagttcttagaatcgaaatccatacgttgtcaaacttacagttacattaaattcttttcaattaaacctctgtaacattaattaattatcatacaagcaattataaaaaactgaggacctaatgtaatagggattcagatttcatctagtaggcttaggatcaccatactcaaacaccaatttgcctggtgtctgtccagctcaaaccgaagatcacaactaaactctcaacaagtgggcgaaacctggataaatgttaagaattgagatctcaaattgagttctcctgtaagttagggtttctgtaacacattgtcaatccaatatcatgggtaaaattaaggttataataattagctctttactactatcaactattacgactgcacaagtaggttgggacaatttaacttcgattggagttataagtactaagcaatatgattataaaataaccactttgaatactaaccagttgatggttataaagatggtccccaatatatcatcaatcatcaattgcaccaagcctgagttgattaaatatcgagagttggtcttaggggttattagaccaatcaatgaatcgttagaattgatgaattcatacattaacatgaggacaggttcagagagattcataggggctgtaatagctggagttgcattgggtgtggcaactgcagcgcaaataacatcaggaattgcattacataactcaattatgaacaaaaagcaaatacaagaattgaggaaggccctcagtaccaccaataaagcaattgatgaaataaggattgcaggtgagagaacattaatagcagtccaaggtgtacaagattacattaataatataattattcctatgcaggacaaacttcaatgtgatattttatcatcacagcttgctattgccttactcaggtattatacaaatatattgacagtttttgggccaagcatacgagatcctgttactagtacaatctcaatacaagcacttagtcaggcgtttaatggtaatctccaggcattgcttgatggattaggatataccgggagagacttacgtgatcttttagagagtagatctattactggtcagataattcatgcagatataactgatttgttccttgtcctcagaattaactatccttctataactgaaatgcagggagtaacgatatatgaacttaattcaattacatatcatattggacctgaggaatggtatactattatgcctaattttatagctgttcagggttttttaacatccaatttcgatgaaaggaagtgctcaataactaaatcaagtatactgtgccaacaaaattcaatttacccgatgtcaacagaaatgcaaagatgtatcaagggtgagataagattctgtccaagatccaaagcaattggaacattagttaataagtttatcttgactaaaggtaatttaatggctaattgccttggtattatatgcaggtgttatacttcaggccaaattataacacaagaccctagtaagttaattacaataatatcacaagaggaatgcaaagaagttggagttgatggtatccgtattatggtaggacctaggaaattaccagacattacctttaacgctaggttagaggttggtgtgccgatatcattaagtaaattagatgtaggaactgatttagcaattgcttcagctaaacttaataattctaaggcactgttggaacaatcagataaaattctggactcaatgtctaaattggattctattaattcacgaatcacagggttgatcttggcaatcatggtaatctttataatcatcgttactattgtctggatcatatacaaaagatgcagaaataaagataataaattcagtacttcaattgaaccgctttatatacctccttcttacaactcacctcacagtgtggttaagtctatttgagtactaactgtatgatttactgtgataaattcagtgaaattaacaagtgatgatattggtgtctcaataagtattgatcatgttacatactctgttaaactaaatgctgataacaggttatagatgattgtaattgtttcaatgaaattatatattaattctattaccttgcataattttcatacaattgaattatatgttattaattaataccttaatgggtttgccttatatacttagactaatagacagatatgctatattgtaatcaagaatttaatacttaaaagacggaataatttaactttttgctaattgatgattgtgtattcaattagaaaaaacttaggaatccatgttaatacaagcttattatcatggagtccaacaacattaaatattacaaagactctaatcggtatcttggtaaaatattagatgaacacaagacagttaataatcaattgtacaggttgagtattaaagtaattaccattattgctattattgtaagcttaattgcaacaataataactattattaatgccacaagtggaagaactaccctaaacagtaatacagacatactgcttagccaaagagatgagattcatagtattcatgaaatgatatttgaccgtatttatcctttgataactgctatgagtacagagctaggacttcatattcctactttattagatgaacttactaaagcaattgatcaaaaaattaaaataatgaatcctcccgttgatactgtaacatctgatcttaactggtgtatcaaacctcctaatgggattattatggatccaaaaggttattgcgaaagtatggaattatctaaaacttacaaattattgcttgatcagttagatgtctcaagaaagaaatcgctcattataaatagaaagaatatcaaccagtgtcaattagttgatgactcaaagatcacttttgctactgttaatatacaatctacaccaaggtttttaaattttggtcatacagtcagcaatcaacgtataacatttggtcaaggaacttatagtagtacttatattataactatccaagaagatggaataaatgatgttcaatatcgagtgtttgaaattggatatatctctgatcagtttggttttttcccctcattaatagtatctagggtattgcctatacgtatggtattgggaatggaatcctgtaccttgacgagtgatcgacaaggtgggtatttcttatgtatgaatacattaacacggtctatatatgattatgtcaatataagagatttgaaatcactatacataacacttcctcattatggtaaggttaattatacttacttcaattttgggaaaattaggagcccacatgagattgataaaatttggctaacgtccgaaagaggtcaaattatttctggttattttgcagcatttgtcacaattacgattcgaaattataataattatccctacaaatgtttgaataatccatgttttgacaactctgagaattactgtaggggatggtataagaacataacaggcaccgatgatgttccaatactagcatacttactagttgaaatgtatgatgaagaaggacctttaattacacttgtagcaataccaccttacaattatacagctccatctcataattctctttactatgatgacaaaattaataagttgataatgactacatctcacactgggtatatacagatcaatgaggtgcatgaggtgattgttggtgatgatttaaaggctattctcctgaacagattatctgatgaacaccctaatcttacagcctgtagacttaatcaaggcattaaagagcagtacaagtccgatggaacgataatttcaaattctgcacttattgatatacaagaacgaatgtatattacagtcaaagctattccaccagtaggtaactataactttacagttgagttgcactctagatcaaacacatcttatatattgttaccgaaacagttcaatgccaagtatgacaaattacatcttgagtgctttaattgggacaagtcttggtggtgtgctttgatacctcaattttcattaagttggaatgaatccctttctgttgatactgctatttttaatttaataaattgtaaatgaatctatcagctaatagttaatagttgttcaaatgacagttaattaaggtaaaatgaatagagaagttgaattatcaacatttgattaagtatatattcaaactagattacaaaaaacttaggagtcagaaacttcttcgcaatggagcagtcagactaccaagatattctatatccagaggtacatcttaacagtcctatagtaatttctaaattggtaggcattttggagtatgctcaagttattcataatcaacaattaacagatcatacaattattaagaatatccaatttagattaagaaatgggtttaatagtcccaggatacagacactgtcaactatgggtgaaatcatcaacaaaattaaaaacaagtatcctaattatattcatataccttatcccgaatgcaaccaaaaattgtttaggatagtagatccagaactaacatcaaaattagaatctcttctgaacaaaggtgatacactatttctcaaaattcggtcagatatcataaaatgtttcgataaactgaagatgaagatgaatataagtaatgatcttcttaatgacaatagtcaattaattttggatcttcctttaattatcaaaggatctcaatggtttttcccgtttttattttggttttctattaaaactgaaactagaagctgtattcgccaaaatccaaaagctcgtgttagatcacaatatcgaccccacttatcagagactaaaagaattacattagttgttacatctgatctgattacaatatttgatcatattaataaatgcacattttacctgacttttgaaatgctattgatgtattgcgatgtgatagaaggtaggttaatgactgaaacagctatgagcctggattgtcgatttaccaatctgttaccaagagtgcaatatatgtgggatttactagacggaatgtttgaaagtctaggtaatcagttatattcagttattgcattattagaacctctttctcttgcttatttgcaattgatagatgctgatccgcagattcggggaacattcttgcatcactgtttctcagagttagaagaaatcatatttgacaaatctccttttgacccttttgtgtatgaaaatcttatcaacggacttgattatatttatcttacagatgacattcatctaactgcagaagttttttctttttttagaagttttggtcatccttacttagaagcacaaaatgctgccaacaatgtgaggaagtatatgaatcagcctaaagtgatctcataccagaccttaatgcaaggacatgcaattttctgtggaattataataaatgggtttagagatcgtcatggaggaacatggcctcctgtagaattgccgagtcatgcatctgctgtaatcagaaatgcccaactatctggggaagggttaacatctgaacaatgtgctcaacattggagatcgttttgtgggtttaaattcaaatgttttatgccattaagtctagatagtgatcttacaatgtaccttcgagacaaagcattgtcacctgttagaagtgagtgggattctgtctatgctaaagagtatttaagatataatccaggattacctacaagttccagaagattagtgaatgtatttttagaagatgataagtttgacccatatgaaatgattatgtacgtgataaatggtgattacctacgagataatgagttcaacctttcatatagtcttaaagaaaaagagatcaaagaggttggtcgattgttcgccaaaatgacttataaaatgagggcttgtcmagtaatagctgaaaacttgattgctaatggagtagggaagttttttaaagacaatggaatggcaaaagatgaacataaactaactaagacattacacaaattagccatttcaggtgtacctaaagataattctcaactttatctagatgaatgctgggagcaggtagttcgacagtgttcaagtgatacacatacaacaaaaccgattatgagttcgcaaccaaagaggataattgaatcaaagtcttctagaccacctctcaatcatagggatacttttaaaggtaagagagacccgaatacacagttaaagtacccttcaaacaccgaatattatgagactatcagtagttttataactactgacctcaaaaagtactgtcttaattggcgatatgaatcaagtagtgtatttgcggagagacttaatgaaatttacggattgcccggatttttccagtggcttcataaaattttggaaaaatccgttttgtatgttagtgatccatctagcccacctgactttgatcaacatgtcgatatagaatcagttccaaacgaccacatctttattaaatatccaatgggtgggatagaggggttctgtcagaaattatggactattagtacaatcccatttctatacttagcagcctttgatacaggtgttagaatcgcatcattggttcagggcgataatcaagcgatcgcagtgacaaaaagagttccgtcatcttggagttactcgaagaaaaaggaagaatcaactaaaataacaacacagtatttccttaatttaaggcaacgtctgcatgatataggtcatgaattgaaagcaaatgagactatcatatcctctcatttctttgtttactctaaaggtatttattacgatggaatacttctttctcaggcacttaaaagtatggcaagatgtgtcttttggtctgaaacaattgttgatgagactagatcagcttgcagtaatatatccaccacacttgcgaaggcaattgaaaggggttatgataaatttgtggcatatgccatcaatatttataaaaccatacatcaagttttgattgcattatcttttaccatcaatcctactatgacaccagatatcacagaacctttctacaaaagcttagatctacttaaaaacctagtcttaattcctgcaccattagggggtatgaactacatgaacatgagcaggttgtttgttagaaatataggagatcccattactgcttcatttgctgatataaagcgcatgattgaatgtgggttgctgggatgtagtatcttgtcacagataatgtaccaaaagtgtggttcctctaagtatttagactgggctagcgatccttattcaataaaccttccgtatagccaaagtatgaccaaggtattgaagaatgtaacggcaagatatgtgctcatgcatagccccaaccctatgcttaaagatttgttccatgaaaagtcgcaagaagaggatgagattcttgctgagtttttattagaccgacatttaataattcctagggcagcacatgaaattttatcaaattcagtaacaggtgctagagaatctattgcaggtatgcttgacactactaagggtttgatccgtgctagtatgtcgagaggtggtttgacatcgtcacttgttttaaaattatcaacatatgattatcagcagtttagaacgtgtcttgaatggctttatgctcctaccacgggaattgctgtgagtgtcgatttatgttctgttttcttagctaagactatccgaaaaagaatgtgggttcacctaaccaaaggaagggagatttacgggttggaagtacctgacattttggaatgcatgcagaacaatataattatcgatcatgaagattgttactcatgtattcaaggatcgagatattatacatggttttttgtgccttcaaattgtcaactagatcagataaataagtcaacaaattctctccgagttccttatgttggatcaacaacagaagaaagaagtgatatgaggttatcatatgtgaggtcaccaagtcgaccacttaaagcggcagttagaattgcagctgtatatacatgggcttatggtgatgatgatttatcttggcacgaggcttggtatttagcaaggaccagagcaaatattacctttgatgaactcaaattaataacacctatagccacatctacgaatttagcacacagattaagagataggagtacccaggttaaatattcaggaacttctttagtaagagtagcgcgctacacaacaatctccaatgataatatgtcgttcattattaacaacaagaaagtagatactaactttgtctatcagcaaggcatgttgttaggcttgagtatactagagtacatatttagatattgtacaagcactggacaatcaaatactgtaattcacttacatgcagacgttaactgttgtatagtacagatgactgatcagccctatacacctagcttaacaaagaagctacctgatattaaacctattaataataaattgatatatgatccggctcctataattgatactgatgcagctagattatattctcaaaagtacctatcacatctaatagatttcccaagctggtcaactactcagcttaacacagtattggcaaaagtggtggcagtatctattgtggaattaataacaaaggcaagtaaagaccatcttaatgagataatagcagttgttggtgatgatgatattaatagttttattacggagtttctacttgttgatccacgtctgtttacactatacttaggccaatatacatcattacaatgggcatatgaagttcattaccatagaccagtaggtaagtaccagatggccgaagtgttacataatctactgtcaagggctagtcgaggtatatttagcgtattgactaatgcctttagccaccctagggtatatagaagattctgggaatgtggtttactagagcctatttatgggccctatatagggagtcagaatctacatactgcagtgattgattatatttataatgcatatattacttatctggatgcttatttatctgatcaggtagatgatactgatatcataatatgcgaaacagaggagacatgtctatcaaataggatcgacaattatcagagcaggcatttagctatacttatagatttgtattgtgattccactagatgccctaacataaaggggtcagatacaattatgcggaattcaattcttagatcttttatagacaatgagagacgaacaaatccactcggtttggcatggaatcttgatccgttacttgtggatcactttagctgttctattacatatctaagaagaggtattattaaacagatgaggttaagatttgatccaaacatatctcttgagttggctaagatgatcaaacctgatgtaatttatcaagcacctaaagttccgtcttcgtgggctcttatagatatcaatcctgaagtcaatgatcttaatacaatttttggagagctaaatagcaaatggaaagatattcctattgggcaaatcaggattcagaattatgaaatacatgcatataggagaattggggttaattcaactgcatgttataaggctctagagatattatctgttttaaatcgatttatgtccaatccattgggtgcactgtttttaggtgaaggagcaggatcaatgctggtcacataccgtgcttttattccatttaagacaatctattataatagtggtatttctgtgcaaaatgtgcaaggtcagagagaactgagtctatatccttctgaagtggcactggttgacaacaaaaatcgtttggctaatgaccctaatatcaaagtcttgtttaacggtaagccggagtctacgtgggttgggaatattgactgttttgcctatattcttagccatattgagaccgcaagcttgacattgatacatagtgatatcgagtccagtttaagcaagacaaaaaataagattcttgaagagctatgccacatcctatcaatggcacttatcttagggagacttggatccgtgttagtcattaaactactaccaagggtcggtgattatacctattcattttgcaagtatgcatcagagttctatcagcaaaactttctcatattacccagatttagtaatatgtcgtcatctgaagtttactacataggagttcaccttaatacaaacagattgattgatcctgatagaatagtacaatacataattagaaatttgcaacccaccccagttacatttttatcctatatctttgagactaaatatagaaacaatatggttacaaattatggactatgcttgtcagatggacacaaaagtgattacttatcatcaattaccaaaatagagaatgttcttctgtcatgtgaattagaattggatggacctaagattataccgccattatcaggacatgactatgcaaatggggagactagcctggaatcaagtataatgatattagttagagaatatcttaatgcaactattcaaggccgagaaacattaggcttgttttcaccttacccagtattacatgagagtcagctaagagaaattaataagtgtattgcattgaagtatattgtgtatttactcttttactcgaactctgtatcatctagtaaacagataatgagtaatcttagaaaagggatattaatgtatgatttgagagacgaatttttcatatcaagattatcagcaaattacaagaaaaaagtaatgtcacaggaagttaaaaccacatggatatttaatattgatacgccaacaagaaaagcattatacaagttagtgggttattcattgataattcatcacgtataatgatcaactgtggttattcatctctagaaaagaaagataagacctgatatattatagctactaaaacattaactctgaattgaaggattgctcagttacataattaataagtaattgagattgtatttcaaacagagcaattagaaaaaacttcctctattaatcaagccctaattcattctatgttaattttatttataatcttgagttaaatctttgtctaaaaacatcacaataatactgatctatcaagggaacataatcggtatttggtattgagtttttatttgtgtaccttaaatcttatgcctatcattatcaattgttatttaagtatctaattatagatgttaatatgttaaatgatgagaaccatcaatactgatattgctggtaattataggcactgtgtgaagcaatgtctaattctcaccaaggtacagtctcacatgtcggatccctcagcctcccctcaataggcaagtggtttgaaaaaaaacaaaaaccaatcttgaatgattgtacggacctatagctttctttgtctggt

SEQ ID NO: 4 - DNA, 1788 bp, Feline paramyxovirus type 2
  misc_feature: FPaV-2 "Gordon strain" H antigen "wild-type" nucleic acid; given as DNA sequence
atggaatctaataacaacaagtactataaagattcaaaccggtattttagcaagatactagatgagaacaagacggtaaataatcatctgtatagtcttagtataaggataattaccgttatagctattgttgtgagtctaattgcaacaacaataaccatcattaatgctataagcggaaggactactcttaataataatatggacatgctactcaaccaacaagacaagattaataatatcaaggaaatgatatttgatcgtatctatcccctgataaatgccatgagtacagagcttggtcttcacattccaactttattggatgagctgactaaatcaattgatcaaaaaatcaagataatgactccaccacttgaaactacaacatctaatctcaattggtgtatcaaccccccaaatggcattattgtagatcctaaaggttattgtgaaggcttggaactgtcaaaaacttataagttattacttgatcaattagatatgttaagaaagaaatcacttattattaataagaaaagtattaatcagtgtagacttgttgatagttcgaatatcgtctttgcaacagttaatatacaatctacaccgagattcttaaatcttggtcacacagttagtaaccaacgtataacattcggtcaaggaacatatagtagcacttatattataactatacaagaggatggattaactgatgttcagtaccgagtatttgaaataggatatatctcagatcaatttggaaccttcccttctctaatcgtttccagagtactacctgtgcgaatggtacttggaatggaatcttgtacactgaccagtgacaagtttgggggttattttttatgcatgaacattccgacacgctctatatatgattatgtcaacataagagacttaaagtcactatacgtcacaatccctcattatggcaaaattaattacacttactttaattttgggaaagtcagaagcccacatgaaattgataagatttggcttacatcagaaaggggacagatgatttcaggttactttgcagcatttgttacgattacaattagaaattataacaattatccctataaatgcttacataacccgtgtcttgaaagatctgagagttattgcaaaggatggtacaaaaatattacaggtactgatgatgttccaatattagcatatctattagttgaaatgaatgatgaggaaggacccttaattacattggttgagataccaccttacaattatacggctccttctcataattccctttactatgatgataaaattaacaaattaataatgacaacatctcatataggatacattcaaatcaatgaagtgcatgaagtcattgtcggggataatcttaaggctattctcttaaacagattatctgatgaacaccctactcttactgcttgtagatttaatcaggaaattaaagagcgacatatatctgatggattaataatatctaactctgctcttattgatatacaagaacgtatgtatgttacagttaaggctgttccacccataggaaattataacttcacggtagagttgcattcacggtcaaatacatcttacgtagggttgccaaggcagttcaatgctaggtatgacaaactgcatctcgaatgctttgcctgggataggtcttggtggtgcgctttgatacctcaattttcattaagttggaatgaatctctttcagtagatactgccattttcaacttaataaactgtaattaa

SEQ ID NO: 5 - DNA, 1788 bp, Feline paramyxovirus type 2
  misc_feature: FPaV-2 "Gordon strain" H antigen nucleic acid that has been codon-optimized for expression primarily in felines; given as DNA sequence
atggaaagcaataataacaaatactataaagacagcaatcggtacttcagcaagatcctggacgagaataagacagtcaataatcacctgtactccctgtctatcaggatcatcaccgtgatcgccatcgtggtgtccctgatcgcaaccactatcactatcatcaatgccatctctggcagaaccactctgaacaataacatggacatgctgctgaaccagcaggataagatcaataacatcaaagagatgatcttcgacaggatctatccactgatcaacgcaatgagcaccgagctggggctgcacatccctaccctgctggacgaactgactaagtccatcgatcagaagatcaaaatcatgactccacctctggaaaccactacctctaatctgaactggtgcatcaatcccccaaacggaatcatcgtggacccaaaaggctactgtgaggggctggaactgtccaagacctataaactgctgctggaccagctggatatgctgaggaagaaaagcctgatcatcaataagaaatccatcaaccagtgcagactggtggatagctccaatatcgtgttcgccaccgtgaacatccagagcactcctaggtttctgaatctgggacataccgtgtccaaccagagaatcactttcggacagggtacttactctagcacctatatcatcactatccaggaggacggtctgaccgatgtgcagtacagagtgtttgaaatcggctatatctctgaccagttcgggacttttccttctctgatcgtgagcagggtgctgcccgtgagaatggtgctggggatggagtcctgcactctgacctctgataagttcggcgggtacttcctgtgcatgaatatccccaccaggtctatctacgactatgtgaacatcagagatctgaagagcctgtacgtgaccatcccccactacggcaaaatcaattacacttatttcaactttgggaaggtgaggagcccacatgagatcgacaaaatctggctgacttctgaaagaggacagatgatcagcggttacttcgccgcatttgtgactatcaccatcaggaactacaacaactacccttacaagtgcctgcacaacccatgtctggagagaagcgaatcctactgcaagggatggtataagaacatcactggtaccgacgatgtgcccatcctggcctacctgctggtggagatgaacgatgaggaaggtccactgatcaccctggtggaaatccctccctacaattatactgcacctagccataactccctgtactatgacgataagatcaacaagctgatcatgactacctcccacatcggatatatccagatcaacgaggtgcatgaagtgatcgtgggtgacaatctgaaggccatcctgctgaacaggctgagcgatgagcacccaactctgaccgcatgtaggttcaatcaggagatcaaagaaagacatatctccgacggcctgatcatctctaacagcgccctgatcgatatccaggagaggatgtacgtgaccgtgaaggcagtgccacctatcggcaattataactttaccgtggaactgcactccagatctaatactagctacgtggggctgcctaggcagttcaacgcaagatatgacaaactgcatctggaatgctttgcctgggatagatcctggtggtgtgcactgatcccccagttttctctgtcctggaatgagagcctgtccgtggatactgctattttcaacctgataaactgtaactaa

SEQ ID NO: 6 - protein, 595 aa, Feline paramyxovirus type 2
  MISC_FEATURE: FPaV-2 "Gordon strain" H antigen translated amino acid sequence
MESNNNKYYKDSNRYFSKILDENKTVNNHLYSLSIRIITVIAIVVSLIATTITIINAISGRTTLNNNMDMLLNQQDKINNIKEMIFDRIYPLINAMSTELGLHIPTLLDELTKSIDQKIKIMTPPLETTTSNLNWCINPPNGIIVDPKGYCEGLELSKTYKLLLDQLDMLRKKSLIINKKSINQCRLVDSSNIVFATVNIQSTPRFLNLGHTVSNQRITFGQGTYSSTYIITIQEDGLTDVQYRVFEIGYISDQFGTFPSLIVSRVLPVRMVLGMESCTLTSDKFGGYFLCMNIPTRSIYDYVNIRDLKSLYVTIPHYGKINYTYFNFGKVRSPHEIDKIWLTSERGQMISGYFAAFVTITIRNYNNYPYKCLHNPCLERSESYCKGWYKNITGTDDVPILAYLLVEMNDEEGPLITLVEIPPYNYTAPSHNSLYYDDKINKLIMTTSHIGYIQINEVHEVIVGDNLKAILLNRLSDEHPTLTACRFNQEIKERHISDGLIISNSALIDIQERMYVTVKAVPPIGNYNFTVELHSRSNTSYVGLPRQFNARYDKLHLECFAWDRSWWCALIPQFSLSWNESLSVDTAIFNLINCN

SEQ ID NO: 7 - DNA, 1014 bp, Feline paramyxovirus type 2
  misc_feature: FPaV-2 "Gordon strain" M antigen "wild-type" nucleic acid; given as DNA sequence
atgactgagatattcaatctggatgaaagttcatggtcagtcaagggaacactggacccattgacgcctgatacttatcctgatgggcgcctagtacccaagattcgggttattgatcccggtctaggtgatcgtaaaagtggaggatatatgtacttactccttcacggtgtcatcgaggacagtgagaccgtcataaatccgaaagggagagcatttggagctttccctttaggcgtagggcaatcaaccgagaacccagaagacttatttaaggaaatattaaccctcaacattgttactcgcaggactgctggcttcaatgaaaaattggtgtattataatactacacctctaaatctactaaccccttggaaaaaagtactagcatatggaagtatctttactgctaatcaggtctgcaataatacaagttctatccctatagacattcctcagaaatttcgacctgtctatttaactgttaccaagttatcggatgatggatattatcagatacctaaaatgatacaggatttcaaatcatcaaactctgttgcatttaacatccttgtgcatctatcaatgggaacaattttacttgactcatctaaaggctctcgagtaggaaaccctgcagaaaatttgatcacattcatgattcatattgggaatttcaaacggaagaataataaagcttattctcccgaatattgtaagaggaaaataatgaggcttggattaattttctcactaggagccattggtggaacaagtttgcatattcgatgcacaggcaaaatgagtaagagattacaagcctacttagggtttaaaagaactttatgttatcctctgatgtatgtcaatgagggtctaaataaaaccttatggagaaatgaatgcaaaattgagaaggttcaagcagtattacagccatcagttccgaatgaatttaagatttatgatgatataatcattgataacacgaatggcctctttaaggttaagtaa

SEQ ID NO: 8 - DNA, 1014 bp, Feline paramyxovirus type 2
  misc_feature: FPaV-2 "Gordon strain" M antigen nucleic acid that has been codon-optimized for expression primarily in felines; given as DNA sequence
atgactgagatcttcaacctggacgaaagctcttggagtgttaaagggaccctggaccctctgacccccgatacctaccccgatgggaggctggtgccaaagatcagagtgatcgaccctgggctgggggataggaaaagcgggggctacatgtatctgctgctgcacggggtgatcgaggactctgaaaccgtgatcaaccccaaggggagagccttcggggcatttccactgggggtggggcagagcaccgagaatcccgaagatctgttcaaggagatcctgactctgaacatcgtgaccaggagaactgccgggtttaatgaaaaactggtgtactataacaccactcctctgaatctgctgactccctggaagaaagtgctggcctacgggtctatcttcaccgcaaaccaagtgtgtaacaatactagctccatccccatcgacatcccacagaagtttaggcctgtgtatctgaccgtgactaaactgagcgacgatgggtactatcagatccccaagatgatccaggacttcaaatctagcaactctgtggcatttaatatcctggtgcacctgagcatggggaccatcctgctggattcctctaaggggagcagggtggggaacccagccgagaatctgatcactttcatgatccatatcgggaacttcaagagaaagaacaacaaggcatactcccctgaatattgcaagaggaaaatcatgagactggggctgatcttcagcctgggggcaatcgggggcacctccctgcatatcaggtgcactgggaagatgtccaaaagactgcaggcatacctggggtttaagaggaccctgtgttaccctctgatgtatgtgaacgaggggctgaataaaactctgtggagaaacgagtgcaagatcgaaaaagtgcaggccgtgctgcagccatctgtgcctaatgagttcaaaatatacgacgacattatcatagacaatacaaacgggctgttcaaagtcaagtaa

SEQ ID NO: 9 - protein, 337 aa, Feline paramyxovirus type 2
  MISC_FEATURE: FPaV-2 "Gordon strain" M antigen translated amino acid sequence
MTEIFNLDESSWSVKGTLDPLTPDTYPDGRLVPKIRVIDPGLGDRKSGGYMYLLLHGVIEDSETVINPKGRAFGAFPLGVGQSTENPEDLFKEILTLNIVTRRTAGFNEKLVYYNTTPLNLLTPWKKVLAYGSIFTANQVCNNTSSIPIDIPQKFRPVYLTVTKLSDDGYYQIPKMIQDFKSSNSVAFNILVHLSMGTILLDSSKGSRVGNPAENLITFMIHIGNFKRKNNKAYSPEYCKRKIMRLGLIFSLGAIGGTSLHIRCTGKMSKRLQAYLGFKRTLCYPLMYVNEGLNKTLWRNECKIEKVQAVLQPSVPNEFKIYDDIIIDNTNGLFKVK

SEQ ID NO: 10 - DNA, 1632 bp, Feline paramyxovirus type 2
  misc_feature: FPaV-2 "Gordon strain" F antigen "wild-type" nucleic acid; given as DNA sequence
atgtataagattaaggttgtaatcatgggttttttactgttatcagatattacatttgcacaggtaggttgggataatttaacctcaattggagttataagtactaaacaatataactataagataactactttgaatactaatcaactcatggtgatcaaaatggtacccaatatatcatcaattattaactgtactaaacttgaattagcaaaatatagggaactgattacaggaatactgagaccaattaatgaatcattagaattgatgaattcatatatcaacatgagaacaggttcagagagattcataggggctgttatagcaggagtagctctaggggttgcaactgcggcgcagataacatcgggaattgccttacataattcgattatgaataaaaaacagatacaggaattaaggaaagcccttagtactacaaataaggcaattgatgagataaggattgcaggtgaaagaactctgatagctgtccaaggtgtgcaagattacattaacaatgttattatccctatgcaagagaaactccagtgcgatattttagcctcacagctatctattgccctactcagatactatactaatatactgactgtttttggaccaagtataagagatcctattactagtacaatttctatacaagctctcagtcaagcattcaatggtaatctacaggcattgcttgatggattagggtatactggacaagacttacatgatctcatagaaagtagatctatcactggtcaaattattcacgctgatatgactgatttattccttgtattgagaatcaattatccatctattacggatatgcaaggagtggtaatatatgagctgaattctatcacatatcatattggacctgaagagtggtacactattatgcctaatttcatagctgttcagggatttctggtatctaatttcgatgaacgtaaatgttcaattactaaaacaagtatactgtgtcaacagaattcaatttatcctatgtcaaccgaaatgcaaagatgtataaaaggtgagattaaattctgtccaaggtccaaagcaattgggacattagttaatcgatttatattaattaatgggaatctaatggccaattgtttgggtattatctgtagatgttatacctcaggtcaaattataacgcaagacccaaataaattaatcacaattatatcacaagaagaatgtagagaggttggtgttgatgggattcgtataatggtggggcctaaaaaattaccggatgttatctttaatgccagactagaaataggtgtacctatctcattaagcaagctggatgttgggaccgacttggcaattgcttcagctaaactcaataactctaaggcacttttggagcagtctgataaaatcttaaattctatgtctaagttggattctttaaattcacgtatcttaggatctgtctttataattatgataatcttcgtgactgtaattgtgattatttggattatttgtaaaaagtgtagaaataagaggaacaaattaagtgcttctattgaacccctctacatacctccctcttataattcaccccatagcatagttaaatctatttga

SEQ ID NO: 11 - DNA, 1632 bp, Feline paramyxovirus type 2
  misc_feature: FPaV-2 "Gordon strain" F antigen nucleic acid that has been codon-optimized for expression primarily in felines; given as DNA sequence
atgtacaaaatcaaggtggtcatcatggggttcctgctgctgagcgacatcacattcgcacaggttggctgggacaatctgactagcatcggggtgatcagcaccaagcagtacaactataaaatcaccactctgaacactaatcagctgatggtgatcaagatggtgcccaacatcagctccatcatcaattgcaccaagctggagctggccaaatacagggaactgatcactggaatcctgaggccaatcaatgagtctctggaactgatgaacagctatatcaatatgaggaccggaagcgagagattcatcggtgcagtgatcgcaggtgttgcactgggagtggccaccgccgcacagatcactagcggtatcgcactgcacaactccatcatgaataagaaacagatccaggaactgaggaaggccctgtccaccactaacaaagcaatcgacgagatcaggatcgccggagaaagaactctgatcgcagtgcagggtgtgcaggactacatcaacaatgtgatcatcccaatgcaggagaaactgcagtgtgatatcctggcctcccagctgtctatcgcactgctgaggtactataccaacatcctgactgtgttcggcccctccatcagggacccaatcaccagcactatctccatccaggccctgtctcaggcatttaacggcaatctgcaggccctgctggatggcctggggtataccgggcaggacctgcacgatctgatcgaatctaggagcatcaccgggcagatcatccatgcagacatgactgatctgttcctggtgctgagaatcaactacccttctatcactgacatgcagggagtggtgatctacgagctgaatagcatcacctatcatatcggtcctgaggaatggtatactatcatgcccaactttatcgccgtgcagggattcctggtgtccaattttgatgaaaggaagtgctccatcaccaaaacttctatcctgtgtcagcagaacagcatctacccaatgtccaccgagatgcagagatgcatcaagggagaaatcaaattctgtcctaggtctaaggccatcggtactctggtgaacagatttatcctgatcaacggcaatctgatggcaaattgcctggggatcatctgcaggtgttataccagcggccagatcatcactcaggatcctaacaaactgatcaccatcatctcccaggaagagtgtagggaggttggagtggacggtatcagaatcatggtggggccaaagaaactgcctgatgtgatctttaatgccagactggaaatcggcgtgcccatctccctgtctaagctggacgtggggactgatctggccatcgcatccgccaagctgaacaattctaaagcactgctggagcagtctgacaagatcctgaacagcatgtccaaactggattctctgaatagcagaatcctgggcagcgtgttcatcatcatgatcatctttgtgaccgtgatcgtgatcatctggatcatctgcaagaaatgtaggaacaagagaaataaactgtctgcaagcattgaacccctgtacattccaccatcctataactcccctcattccattgtgaaaagcatttga

SEQ ID NO: 12 - protein, 543 aa, Feline paramyxovirus type 2
  MISC_FEATURE: FPaV-2 "Gordon strain" F antigen translated amino acid sequence
MYKIKVVIMGFLLLSDITFAQVGWDNLTSIGVISTKQYNYKITTLNTNQLMVIKMVPNISSIINCTKLELAKYRELITGILRPINESLELMNSYINMRTGSERFIGAVIAGVALGVATAAQITSGIALHNSIMNKKQIQELRKALSTTNKAIDEIRIAGERTLIAVQGVQDYINNVIIPMQEKLQCDILASQLSIALLRYYTNILTVFGPSIRDPITSTISIQALSQAFNGNLQALLDGLGYTGQDLHDLIESRSITGQIIHADMTDLFLVLRINYPSITDMQGVVIYELNSITYHIGPEEWYTIMPNFIAVQGFLVSNFDERKCSITKTSILCQQNSIYPMSTEMQRCIKGEIKFCPRSKAIGTLVNRFILINGNLMANCLGIICRCYTSGQIITQDPNKLITIISQEECREVGVDGIRIMVGPKKLPDVIFNARLEIGVPISLSKLDVGTDLAIASAKLNNSKALLEQSDKILNSMSKLDSLNSRILGSVFIIMIIFVTVIVIIWIICKKCRNKRNKLSASIEPLYIPPSYNSPHSIVKSI

SEQ ID NO: 13 - DNA, 1560 bp, Feline paramyxovirus type 2
  misc_feature: FPaV-2 "Gordon strain" N antigen "wild-type" nucleic acid; given as DNA sequence
atggctagtttactcaggtcacttgcggcattcaagaaacacagagaacaaccaactgttccttctgggtcaggagggacgatcaaaggattaaaaaatacaattattgtgcctgttcctggagatacagtcatcactaccagatcgaacttactgttcagattagtctacataattggtaatccagatacacctttaagcacttcaacaggggcaataatatcattgttgacattatttgttgaatctccaggtcaattaattcaaagaatcgctgatgatcctgatgctgtttttaaattagtagaggtggttcctgaggttggtaatcctggagaattaacttttgcatctagaggaattaacttggataaacaagctcaacaatactttagattggctgagaaaaatgatcaaggatattatgtaagtttggggtttgaaaatccaccaaatgatgatgatataacgtcaagtcctgaaatctttaattatattttagcatctgtacttgcacagatctggattctcctagctaaggctgtaactgctccagacacagctgctgaggctgaaaaccgtaggtggattaaattgatgcaacaacgcagagtggatggtgagcttagattaagtaaaggatggttggacttagtgaggaataaaatcgcatcggatatcacaattagaaggtttatggtagcattagttcttgacattaaacgttctcctggaacaagaccaagaattgctgaaatgatttgtgatatagacaattatattgtggaggccggactggcaagttttctgttaactatcaaatttggtatagaaacacgttacccggcattagcgttacatgagttttcgggggaattagccactattgaaggactcatgaaattgtaccagtctatgggagaaatggcaccatacatggtcattctagagaattcgatccagactaggtttagtgctgggtcttatccgttactctggagctatgctatgggtgttggtgtagaacttgaaagatcaatgagtggattaaacttcacaagaagtttctttgatcctacgtacttcaggttgggtcaggagatggtaagaaggtcttcaggaatggttaatagctcatttgccaaagaacttggactatctgaacatgaaacacaacttgttagccagatcattaactcaggtggtgagtcaggtataccgaaatttgatggatttagagcaaacccaacaacatttctaggggctaaggacaacatcactgataggagtgaagatccattgattgcaattccagggtcatcaggacaaccattgccaggttatgaccccaatatctcaggtgactcatatagaattgatagtagcactaaagacacaaacaatatatcagatggaggaacaaatccaagtcatgatgtttccaattctgctatggaagagctgagaagattggtagagtctaccaacaagattgatacaaagaaatctgaaagcccaggcatcgttaatcattacaacgatactgaccttctgagataa

SEQ ID NO: 14 - protein, 519 aa, Feline Paramyxovirus type 2
  MISC_FEATURE: FPaV-2 "Gordon strain" N antigen translated amino acid sequence
MASLLRSLAAFKKHREQPTVPSGSGGTIKGLKNTIIVPVPGDTVITTRSNLLFRLVYIIGNPDTPLSTSTGAIISLLTLFVESPGQLIQRIADDPDAVFKLVEVVPEVGNPGELTFASRGINLDKQAQQYFRLAEKNDQGYYVSLGFENPPNDDDITSSPEIFNYILASVLAQIWILLAKAVTAPDTAAEAENRRWIKLMQQRRVDGELRLSKGWLDLVRNKIASDITIRRFMVALVLDIKRSPGTRPRIAEMICDIDNYIVEAGLASFLLTIKFGIETRYPALALHEFSGELATIEGLMKLYQSMGEMAPYMVILENSIQTRFSAGSYPLLWSYAMGVGVELERSMSGLNFTRSFFDPTYFRLGQEMVRRSSGMVNSSFAKELGLSEHETQLVSQIINSGGESGIPKFDGFRANPTTFLGAKDNITDRSEDPLIAIPGSSGQPLPGYDPNISGDSYRIDSSTKDTNNISDGGTNPSHDVSNSAMEELRRLVESTNKIDTKKSESPGIVNHYNDTDLLR

SEQ ID NO: 15 - DNA, 1476 bp, Feline paramyxovirus type 2
  misc_feature: FPaV-2 "Gordon strain" P antigen "wild-type" nucleic acid; given as DNA sequence
atgtcagcagaacaaatccaacaagttagacatggccttgaatccttgcaagagatcaaaaacaaccctccaccctctcaagatgtcaatcttgccagggaaatttacgaatccattaaacaaacaggaacaccttcaacacaaggagggaccattacaggaaataatactgcgtcagggtgtgacaattactcaatgcatagccagggatcaggtccttctgtttcaggtgctgacaagaatatcgagagacttactggacccgattattcagaattatgggatccagaaggtaacctctgcatgctattcgaaagcgatgatgatgacaacaattattcagagattaatggccggtctaccgctatcgaaggattggatgaacagaataataaggacccaggtattaaacaatcaggagatcagtgttctgaaggagtgtctaagattaattcatcttctagtccccaagaagctacattatcttctgggagatctgatatatctgggacaggagtatctccctgtgcctctttggatataactgttaatgaattagaagatgcaactgttaagaatagtaataatatgaaaggaaattggccaatcccaaagttgcttgtcaaaccaccaccaagaatgaaatcactttctgactctgttacaccattaaaaggggccaccgacgggaaatcagtcttacctgggatggagattacattgtccgggaagaatggtgcaaccctacctgtacacccatttacacaacctataaaagactcaaatgcagatgtaagcaatgtccgtcaacatgtcccaagtgtgactgatggtcatagtgatgataatgaggaagtacccggtttgcataaagaaactatagacaaagctgatctatctatgcaggacatatacaatttaattcttggatttaaggatgattacaggaaactatcaaataaattggatatgatactagagatgaaacaagatattgataatcttaaaaagagtagtgcaaaaatacaacttgcattatcaacaattgaaggacatctgtccagtgttatgattgctattccaggttcaggtattgatataaatcaagatgagaagaaggatcaattaaactctgacttaaagccattactagggagggaccattgccgtgcatttcgtgaagtcactaatcctttagatgaaacgtcattgaccaacgctccgaccaaacatgttgctaagatcaacaaaaattgcactcttcagaaaatcaataacaatgagacatctgcaattaagtttgtacctaatgatagccatgcaagtatctcgactatcaagtctattgtcaaatcctcaaaccttaatcaagagcttaaagtcaagttactgacaattctatctcaaattaaaggggtagacaatattaaggagttttatgagaaagttatgatattgatcaagaataataactga

SEQ ID NO: 16 - protein, 491 aa, Feline paramyxovirus type 2
  MISC_FEATURE: FPaV-2 "Gordon strain" P antigen translated amino acid sequence
MSAEQIQQVRHGLESLQEIKNNPPPSQDVNLAREIYESIKQTGTPSTQGGTITGNNTASGCDNYSMHSQGSGPSVSGADKNIERLTGPDYSELWDPEGNLCMLFESDDDDNNYSEINGRSTAIEGLDEQNNKDPGIKQSGDQCSEGVSKINSSSSPQEATLSSGRSDISGTGVSPCASLDITVNELEDATVKNSNNMKGNWPIPKLLVKPPPRMKSLSDSVTPLKGATDGKSVLPGMEITLSGKNGATLPVHPFTQPIKDSNADVSNVRQHVPSVTDGHSDDNEEVPGLHKETIDKADLSMQDIYNLILGFKDDYRKLSNKLDMILEMKQDIDNLKKSSAKIQLALSTIEGHLSSVMIAIPGSGIDINQDEKKDQLNSDLKPLLGRDHCRAFREVTNPLDETSLTNAPTKHVAKINKNCTLQKINNNETSAIKFVPNDSHASISTIKSIVKSSNLNQELKVKLLTILSQIKGVDNIKEFYEKVMILIKNNN

SEQ ID NO: 17 - DNA, 6609 bp, Feline paramyxovirus type 2
  misc_feature: FPaV-2 "Gordon strain" L antigen "wild-type" nucleic acid; given as DNA sequence
atggagcaatcagattatcaagatattttatatccagaggtacatctcaacagtcctatagttatctctaaattagtgggtattttggagtattctaaggttgttcacaatcagcagttatctgatcacacaatagtcaagaatatacaatttagattgagaaatggattcaatagtccaagaatacaaacactgttagttatgggtgaaattatcaataaaatcaaaaataaatacccaaattatttgcacataccttatcctgaatgtaatcaaaagttatttaggatagctgacccggagttaacatctaaactagaagccctcttggacaaaggtgacacattatatcttaagattaagacagagatcatagcttgtttcgataagttaaaaactaaaatgagcataaccaatgatctgattagtgacaataggcagctaatttcagatctacctataattgtcaagggatctcaatggtttttcccttttttgctctggttctctgttaaaactgagactaggaactgtattcgacaaaatcaaaaaactcgtgttaggtcacaataccgacctcatttgtcagaaactaaaagaattacgctggtcgttactcatgacttgatcacaatatttgaccacgtcaacaaatgtatatatcatctgacttttgagatgttgttgatgtattgtgatgtagtagaagggaggttaatgaccgaagcatctatgagtctagatcacagatttattaacctattgtcgagggtccagtatatgtgggatctattagatgggatgtttgagagtctaggaaatcagctatattcaatcattgcactcttagaacctctctctcttgcctatctacagttgatggatgcagacccacagatacggggtacatttttacaccattgcctttcagagttggaagaactcttatttagtaaattcccttttgatcctgtaatttatgaaaatctaattagtggacttgattacatctatttaacagacgatattcatttaactgctgagatattttctttctttagaagttttggtcatccttatttagaagcacaaaatgcagctagcaatgttaggaaatatatgaatcaacctaaagttatctcataccagactctaatgcaaggacatgcaattttttgtggcattataataaatgggttcagagatcgtcacggagggacatggccacccgtagagctaccacatcatgcatccgctgtaattagaaatgctcagttatctggagaaggattaacacctgagcagtgtgctcaatactggaggtcattttgtggatttaaatttaaatgttttatgccattaagtttagatagcgacctcaccatgtaccttagagacaaggcattatcacctattaagaatgagtgggactctgtgtatgctaaagagtatttaagatacaaccctggcttaccgactagctctcgaagattagtcaatgtatttcttgaagatgataaatttgatccgtacgaaatgattatgtacgtaataaacggtgattatttaagggataatgagttcaatctctcatatagtcttaaagaaaaggagatcaaggaggtaggccgattgttcgctaaaatgacttataaaatgagagcttgtcaggtaatagcagaaaatttaattgcaaatggagttgggaaattttttaaagacaatgggatggcgaaggatgaacataaattaaccaaaacattacataagctggccatttctggtgtacctaaagataattttcaactctatttaagtgaatgttgggaacaagtggtagaacaatgcgtaaccagtacgcaaacaaaaaatcaaattatcagttcacactcaagaaaatcagttgcatcaaagtttccaagatcaaatcccaatgataggggtattctaaatagtggcagacatttgaataaacatccaaaacatccttcaaacaccgaatactatgaaactgtcagtagttttataactactgatctcaagaaatattgcctcaactggcgctatgaatcaagtagtgtgtttgcagaaagactcaatgagatttatgggttaccaggattttttcattggcttcatagaattttggagaaatctgtattatatgttagtgatccatccagtccacctgattttgatcaacatgttgatattgattcagttccaaatgatcatatttttatcaaatacccaatgggtgggatagaaggattttgtcaaaaattatggacaatcagcacaatcccatttttatatttagcagcttttgatacaggggttagaatatcttcgttggttcaaggtgataatcaagcaattgcagtgaccaaaagagttccatcgtcctggagttattcgagaaaaaaagaggagtcaactaaagttacaacacaatattttttaaacttaagacaacgcttacatgatataggtcatgagttaaaggcaaatgagactattatatcttcacacttttttgtttactctaagggtatttattatgatggtatacttctttcacaatcccttaaaagtattgcaagatgtgttttttggtccgagacaattgtcgatgagactaggtcagcttgcagcaatatatccactacccttgctaaagctattgaacggggttatgataaattcgtggcatacgctattaatatatataagactatacaccaggtcttaattgcattatcttttactattaatcccactatgactccggacataacagaacctttttataaaagtttagatttacttaaaaacctcattctgataccagcaccattgggtgggatgaattacatgaatatgagcagattatttgttagaaacataggtgatcccattacagcttcatttgctgacatcaagcgtatgatcgaatgcgggttattagggcacaatgttctctcacaaataatgtatcagaaatgtggtacctcgaaatacttagattgggctagtgacccttattccataaatcttccttatagtcaaagcatgaccaaagtattaaaaaatataaccgcgagatatgttctcatgcacagtcctaaccctatgctaaaagatttattccatgagaagtcacaagaagaagatgagattcttgctgaatttttgctggatcgtcagttaataatccctagagctgcacatgaaattttatcgaattcagtaacaggagctagagagtcgattgcagggatgcttgatactactaaaggacttattcgagccagtatgtcaagaggtggtctgacatcttcacttgtgttgaaattgtcaacatatgattatcaacaatttagaacatgccttgaatggctttatgcccctaccacaggaatagcagtaagtgctgattcttgttcagtttttttagccagagctattcgaaaaaggatgtgggttcacctgactaaaggaagagaaatttatggcctagaagtgcctgatatattagaatgtatgcagagcaatgtaattgttgatcatgaagattgttattcatgtattcaaggatcaagatactacacatggttttttgtaccttctaattgtcagcttgatcagattaacaagtctacaaattctctacgggttccttacattggctctactacagaggaaagaagtgacatgaaattatcatacgtcagatcccctagtaggccacttaaggcagcagtccgaattgcagcagtctacacatgggcatacggtgatgacgatctgtcttggcgtgaggcttggtacttggcaaggactagggcaaatgttactttcgatgagcttaaattagtaacacccatagctacctctacgaacttggcacatagattaagggacaggagtactcaagttaagtattcaggaacttcattagtaagagtggcacgctatacaacaatatccaatgataatatgtcatttgtcattaatgacaaaaaggtagatactaattttgtctatcaacagggcatgttattgggtttgagtatcctagaatatatatttagatactgtaaaagtactggtcaatcaaatactgtagttcacttgcatgcagatgttaattgttgcataatccaaatgacagatcaaccttatactccaagcttaacgaaaaaattacctgagattaaacctattaataataagttgatttatgatccagctcctataattgatactgatgcagctaggttatattctcagaagtacttatcacacctgatagattttccaaattggtcaatgaatcagctaaatgtagttttagcaaaagtagttgcaatatctattgtggacttgataactaaagcgagtaaagatcatctcaatgaaattatggcagttgttggagatgatgacattaatagctttataacagaatttttgctagttgatccgaggctatttacattgtacttaggtcaatacacgtcacttcaatgggcatatgaaattcattatcaccgacccgtaggcaaataccagatggcagaagtgttacacactttactgtcaagagcaagtaaaggtatatttaatatattaactaatgcttttagtcatcctagagtttacaaaagattttgggaatgtggattactggagcctatttatggaccatacatagggagccaaaatttatatagtacagtaattgattacctttacaatgcttatataacttatttagatgcttatctatctgatcatatcgaagatgcagacatagtaatatgtgagacagaagaaacttgtctagctaataggattgataactatcaaggtaggcatctagccgtacttattgatctttattgtgattctactaggtgtcctaatataaaagggtcagacacaatcatgcgaaactcaattctcaaatcttttattgataatgagagaaggacaagtccattaggtctaacatggaatcttgatccattactcatagatcatttcagttgttcaattacttatctgaggagaggtattattaaacagattaggctaaggtttgatccaaacatatctattgagttggttaaattggcaaaacctgaagtgattcatcaaggaccaaaaataccgtcttcttgggcccttatagatattaatcctgaggtcaatgatcttaatacagttttcggagaattaaatagtaaatggaaagatattcctattggacaaattagaattcaaaattatgagatccatgcttaccgaagaattggagttaattcaactgcatgttataaagcattggaaatgctatctgtactaacccggtttatgtctaacccagcaggagctttgtttttaggagagggtgcagggtcaatgttagttacctatcgtgcgtttatcccgttcaagagaatttattataatagtggaatttctatacaaaatattcaaagccaaagagaactaagtctatacccatctgaagtagccttggttgataataaaaatcgtttgaccagtgatcctgatatcaaagtcttatttaatggcaagccagaatccacgtgggttgggaatatagactgctttgcttatattctgagtcatattgaaacttctagtttaacattaatccacagtgatattgaatctagcttgagtaaaacaaagaataagattcttgaggagctttgccatattctatcaatggcactgattttaggaaagattggatctgtattagttattaagctgttaccacgggttggtgactacacatattcattttgcaagtatgcgtcagaattctaccaacagaatttttttattttacctagatttagcaacatgtcatcatctgaaatttactacgttggagttcatttaaataccaatagactggttgatccagataggattgtgcaatatataatcaggaatctccaatctactccagttactttcttatcttacattttggaaactaaatatagaaataatatggttacaaattatgggctctgcttgtctgatggacataaaagcgattacttgtcatcaatcaccaagatagaaaatgttcttttatcatgtggattggaattgaatggacctaagattatacagcaattatctggacatgactacgccaatggagagattagcttagaatcaagtataatggtactggttagagaatatctaaatgcaactatccaaggtcgggaaacactaggtcttttttcaccttaccctgtgttacatgagagtcagttaagagaaattaacaggtgcattgcattgaagtatgttgtatatttacttttttactcaacctctgtaggatctagtagacaaatcatgagcaatctcagaaaaggagtattaatgtatgacttaagagatgagtttttcatggaaaggttatcaacaaatttcaagaaaaaaataatgtcacaagaggttaaaactacatggatctttaatattgatgtaccaacaagaaaagctctgtataaattagttggttattcacttatcattaatcacgtataa

SEQ ID NO: 18 - protein, 2202 aa, Feline paramyxovirus type 2
  MISC_FEATURE: FPaV-2 "Gordon strain" L antigen translated amino acid sequence
MEQSDYQDILYPEVHLNSPIVISKLVGILEYSKVVHNQQLSDHTIVKNIQFRLRNGFNSPRIQTLLVMGEIINKIKNKYPNYLHIPYPECNQKLFRIADPELTSKLEALLDKGDTLYLKIKTEIIACFDKLKTKMSITNDLISDNRQLISDLPIIVKGSQWFFPFLLWFSVKTETRNCIRQNQKTRVRSQYRPHLSETKRITLVVTHDLITIFDHVNKCIYHLTFEMLLMYCDVVEGRLMTEASMSLDHRFINLLSRVQYMWDLLDGMFESLGNQLYSIIALLEPLSLAYLQLMDADPQIRGTFLHHCLSELEELLFSKFPFDPVIYENLISGLDYIYLTDDIHLTAEIFSFFRSFGHPYLEAQNAASNVRKYMNQPKVISYQTLMQGHAIFCGIIINGFRDRHGGTWPPVELPHHASAVIRNAQLSGEGLTPEQCAQYWRSFCGFKFKCFMPLSLDSDLTMYLRDKALSPIKNEWDSVYAKEYLRYNPGLPTSSRRLVNVFLEDDKFDPYEMIMYVINGDYLRDNEFNLSYSLKEKEIKEVGRLFAKMTYKMRACQVIAENLIANGVGKFFKDNGMAKDEHKLTKTLHKLAISGVPKDNFQLYLSECWEQVVEQCVTSTQTKNQIISSHSRKSVASKFPRSNPNDRGILNSGRHLNKHPKHPSNTEYYETVSSFITTDLKKYCLNWRYESSSVFAERLNEIYGLPGFFHWLHRILEKSVLYVSDPSSPPDFDQHVDIDSVPNDHIFIKYPMGGIEGFCQKLWTISTIPFLYLAAFDTGVRISSLVQGDNQAIAVTKRVPSSWSYSRKKEESTKVTTQYFLNLRQRLHDIGHELKANETIISSHFFVYSKGIYYDGILLSQSLKSIARCVFWSETIVDETRSACSNISTTLAKAIERGYDKFVAYAINIYKTIHQVLIALSFTINPTMTPDITEPFYKSLDLLKNLILIPAPLGGMNYMNMSRLFVRNIGDPITASFADIKRMIECGLLGHNVLSQIMYQKCGTSKYLDWASDPYSINLPYSQSMTKVLKNITARYVLMHSPNPMLKDLFHEKSQEEDEILAEFLLDRQLIIPRAAHEILSNSVTGARESIAGMLDTTKGLIRASMSRGGLTSSLVLKLSTYDYQQFRTCLEWLYAPTTGIAVSADSCSVFLARAIRKRMWVHLTKGREIYGLEVPDILECMQSNVIVDHEDCYSCIQGSRYYTWFFVPSNCQLDQINKSTNSLRVPYIGSTTEERSDMKLSYVRSPSRPLKAAVRIAAVYTWAYGDDDLSWREAWYLARTRANVTFDELKLVTPIATSTNLAHRLRDRSTQVKYSGTSLVRVARYTTISNDNMSFVINDKKVDTNFVYQQGMLLGLSILEYIFRYCKSTGQSNTVVHLHADVNCCIIQMTDQPYTPSLTKKLPEIKPINNKLIYDPAPIIDTDAARLYSQKYLSHLIDFPNWSMNQLNVVLAKVVAISIVDLITKASKDHLNEIMAVVGDDDINSFITEFLLVDPRLFTLYLGQYTSLQWAYEIHYHRPVGKYQMAEVLHTLLSRASKGIFNILTNAFSHPRVYKRFWECGLLEPIYGPYIGSQNLYSTVIDYLYNAYITYLDAYLSDHIEDADIVICETEETCLANRIDNYQGRHLAVLIDLYCDSTRCPNIKGSDTIMRNSILKSFIDNERRTSPLGLTWNLDPLLIDHFSCSITYLRRGIIKQIRLRFDPNISIELVKLAKPEVIHQGPKIPSSWALIDINPEVNDLNTVFGELNSKWKDIPIGQIRIQNYEIHAYRRIGVNSTACYKALEMLSVLTRFMSNPAGALFLGEGAGSMLVTYRAFIPFKRIYYNSGISIQNIQSQRELSLYPSEVALVDNKNRLTSDPDIKVLFNGKPESTWVGNIDCFAYILSHIETSSLTLIHSDIESSLSKTKNKILEELCHILSMALILGKIGSVLVIKLLPRVGDYTYSFCKYASEFYQQNFFILPRFSNMSSSEIYYVGVHLNTNRLVDPDRIVQYIIRNLQSTPVTFLSYILETKYRNNMVTNYGLCLSDGHKSDYLSSITKIENVLLSCGLELNGPKIIQQLSGHDYANGEISLESSIMVLVREYLNATIQGRETLGLFSPYPVLHESQLREINRCIALKYVVYLLFYSTSVGSSRQIMSNLRKGVLMYDLRDEFFMERLSTNFKKKIMSQEVKTTWIFNIDVPTRKALYKLVGYSLIINHV

SEQ ID NO: 19 - DNA, 1788 bp, Feline paramyxovirus type 2
  misc_feature: FPaV-2 "TV25 strain" H antigen "wild-type" nucleic acid; given as DNA sequence
atggagtctaataacaacaagtactataaagattcaaaccggtattttagcaagatactagatgagaacaagacggtaaataatcatctgtatagtcttagtataaggataattaccgttatagctattgttgtgagtctaattgcaacaacaataaccatcattaatgctataagcggaaggactactcttaataataatatggacatgctactcaaccaacaagacaagattaataatatcaaggaaatgatatttgatcgtatctatcccctgataaatgccatgagtacagagcttggtcttcacattccaactttattggatgagctgactaaatcaattgatcaaaaaatcaagataatgactccaccacttgaaactacgacatctaatctcaattggtgtatcaaccccccaaatggcattattgtagatcctaaaggttactgtgaaggcttggaactgtcaaaaacttataagttattacttgatcaattagatatgttaagaaagaaatcacttattattaataagaaaagtattaatcagtgtagacttgttgatagctcgaatatcatctttgcaacagttaatatacaatctacaccgagattcttaaatcttggtcacacagttagtaaccaacgtataacattcggtcaaggaacatatagtagcacttatattataactatacaagaggatggattaactgatgttcagtaccgagtatttgaaataggatatatctcagatcaatttggaaccttcccttctctaatcgtttctagagtactacctgtgcgaatggtacttggaatggaatcttgtacactgaccagtgacaagttcgggggttattttttatgcatgaacattccgacacgctctatatatgattatgtcaacataagagacttaaagtcactatacgtcacaatccctcattatggcaaaattaattacacttactttaattttggaaaagtcagaagcccacatgaaattgataagatttggcttacatcagaaaggggacagatgatttcaggttactttgcagcatttgttacgattacaattagaaattataacaattatccctataaatgcttacataacccgtgtcttgaaagatctgagagttattgcaaaggatggtacaaaaatattacaggtactgatgatgttccaatattagcatatctattagttgaaatgaaggatgaggaaggacctttaattacactggttgaaataccaccttacaattatacggctccttctcataattccctttactatgatgataaaattaacaaattaataatgacaacatctcatataggatacattcaaatcaatgaagtgcatgaagtcattgtcggggataatcttaaggctattctcttaaacagattatctgatgaacaccctactcttactgcttgtagatttaatcaggaaattaaagagcgacatatatctgatgggttaataatatctaactctgctcttattgatatacaagaacgtatgtatattacagttaaggctgttccacccataggaaattataacttcacggtagagttgcattcacggtcaaatacatcttacgtagggttgccaaggcagttcaatgctaggtatgacaaactgcatctcgaatgctttgcctgggataggtcttggtggtgcgctttgatacctcaattttcattaagttggaatgaatctctttcagtagatactgccattttcaacttaataaactgtaattaa

SEQ ID NO: 20 - protein, 595 aa, Feline paramyxovirus type 2
  MISC_FEATURE: FPaV-2 "TV25 strain" H antigen translated amino acid sequence
MESNNNKYYKDSNRYFSKILDENKTVNNHLYSLSIRIITVIAIVVSLIATTITIINAISGRTTLNNNMDMLLNQQDKINNIKEMIFDRIYPLINAMSTELGLHIPTLLDELTKSIDQKIKIMTPPLETTTSNLNWCINPPNGIIVDPKGYCEGLELSKTYKLLLDQLDMLRKKSLIINKKSINQCRLVDSSNIIFATVNIQSTPRFLNLGHTVSNQRITFGQGTYSSTYIITIQEDGLTDVQYRVFEIGYISDQFGTFPSLIVSRVLPVRMVLGMESCTLTSDKFGGYFLCMNIPTRSIYDYVNIRDLKSLYVTIPHYGKINYTYFNFGKVRSPHEIDKIWLTSERGQMISGYFAAFVTITIRNYNNYPYKCLHNPCLERSESYCKGWYKNITGTDDVPILAYLLVEMKDEEGPLITLVEIPPYNYTAPSHNSLYYDDKINKLIMTTSHIGYIQINEVHEVIVGDNLKAILLNRLSDEHPTLTACRFNQEIKERHISDGLIISNSALIDIQERMYITVKAVPPIGNYNFTVELHSRSNTSYVGLPRQFNARYDKLHLECFAWDRSWWCALIPQFSLSWNESLSVDTAIFNLINCN

SEQ ID NO: 21 - DNA, 1014 bp, Feline paramyxovirus type 2
  misc_feature: FPaV-2 "TV25 strain" M antigen "wild-type" nucleic acid; given as DNA sequence
atgactgagatattcaatctggatgaaagttcatggtcagtcaagggaacactggacccattgacgcctgatacttatcctgatgggcgcctagtacccaagattcgggttattgatcccggtctaggtgatcgtaaaagtggaggatatatgtacttactccttcacggtgtcatcgaggacagtgagaccgtcataaatccgaaagggagagcatttggagctttccctttaggtgtagggcaatcaaccgagaacccagaagacttatttaaggaaatattaaccctcaacattgttactcgcaggactgctggcttcaatgaaaaattggtgtattataatactacacctctaaatctactaaccccttggaaaaaagtactagcatatggaagtatctttactgctaatcaggtctgcaataatacaagttctatccctatagacattcctcagaaatttcgacctgtctatttaactgttaccaagttatcggatgatggatattatcagatacctaaaatgatacaggatttcaaatcatcaaactctgttgcatttaacatccttgtgcatctatcaatgggaacaattttacttgactcatctaaaggctctcgagtaggaaatcctgcagaaaatttgatcacattcatgattcatattgggaatttcaaacggaagaataataaagcttattctcccgaatattgtaagaggaaaataatgaggcttggattaatcttctcactaggagccattggtggaacaagtttgcatattcgatgcacaggcaaaatgagtaagcgattacaagcctacttagggtttaaaagaactttatgttatcctctgatgtatgtcaatgagggtctaaacaaaaccttatggagaaatgaatgcagaattgagaaggttcaagcagtattacagccatcagttccgaatgaatttaagatttatgatgatataatcattgataacacgaatggcctctttaaggttaagtaa

SEQ ID NO: 22 - protein, 337 aa, Feline paramyxovirus type 2
  MISC_FEATURE: FPaV-2 "TV25 strain" M antigen translated amino acid sequence
MTEIFNLDESSWSVKGTLDPLTPDTYPDGRLVPKIRVIDPGLGDRKSGGYMYLLLHGVIEDSETVINPKGRAFGAFPLGVGQSTENPEDLFKEILTLNIVTRRTAGFNEKLVYYNTTPLNLLTPWKKVLAYGSIFTANQVCNNTSSIPIDIPQKFRPVYLTVTKLSDDGYYQIPKMIQDFKSSNSVAFNILVHLSMGTILLDSSKGSRVGNPAENLITFMIHIGNFKRKNNKAYSPEYCKRKIMRLGLIFSLGAIGGTSLHIRCTGKMSKRLQAYLGFKRTLCYPLMYVNEGLNKTLWRNECRIEKVQAVLQPSVPNEFKIYDDIIIDNTNGLFKVK

SEQ ID NO: 23 - DNA, 1632 bp, Feline paramyxovirus type 2
  misc_feature: FPaV-2 "TV25 strain" F antigen "wild-type" nucleic acid; given as DNA sequence
atgtataagattaaggttgtaatcatgggttttttactgttatcagatattacatttgcacaggtaggttgggataatttaacctcaattggagttataagtactaaacaatataactataagataactactttgaatactaatcaactcatggtgattaaaatggtacccaatatatcatcaattattaactgtactaaacttgaattagcaaaatatagggaactgattacaggaatactgagaccaattaatgaatcattagaattgatgaattcatatatcaacatgagaacaggttcagagagattcataggggctgttatagcaggagtagctctaggggttgcaactgcggcgcagataacatcgggaattgccttacataattcgattatgaataaaaaacagatacaggaattaaggaaagcccttagtactacaaataaggcaattgatgagataaggattgcaggtgaaagaactctgatagctgtccaaggtgtgcaagattacattaacaatgttattatccctatgcaagagaaactccagtgcgatattttagcctcacagctatctattgccctactcagatactatactaatatactgactgtttttggaccaagtataagagatcctattactagtacaatttctatacaagctctcagtcaagcattcaatggtaatctacaggcattgcttgatggattagggtatactggacaagacttacatgatctcatagaaagtagatctatcactggtcaaataattcacgctgatatgactgatttattccttatattgagaatcaattatccatctattacggatatgcaaggagtggtaatatatgagctgaattctatcacatatcatattggacctgaagagtggtacactattatgcctaatttcatagctgttcagggatttctggtatctaatttcgatgaacgtaaatgttcaattactaaaacaagtatactgtgtcaacagaattcaatttatcctatgtcaaccgaaatgcaaagatgtataaaaggtgagattaaattctgtccaaggtccaaagcaattgggacattagttaatcgatttatattaattaatgggaatctaatggccaattgtttgggtattatttgtagatgttatacctcaggtcaaattataacgcaagacccaaataaattaatcacaattatatcacaagaagaatgtagagaggttggtgttgatgggattcgtataatggtgggacctaaaaaattaccggatgttatctttaatgccagactagaaataggtgtacctatctcattaagcaagctggatgttgggaccgatttggcaattgcttcagctaaactcaataactctaaggcacttttggagcagtctgataaaatcttaaattctatgtctaagttggattctttaaattcacgtatcttaggatctgtctttataatgatgataatctttgtgattgtaattgtgattatttggattatttgtaagaagtgtagaaataagaggaacaaattaagtgcttctattgaacccctctacatacctccctcttataattcaccccatagcatagttaaatctatttga

SEQ ID NO: 24 - protein, 543 aa, Feline paramyxovirus type 2
  MISC_FEATURE: FPaV-2 "TV25 strain" F antigen translated amino acid sequence
MYKIKVVIMGFLLLSDITFAQVGWDNLTSIGVISTKQYNYKITTLNTNQLMVIKMVPNISSIINCTKLELAKYRELITGILRPINESLELMNSYINMRTGSERFIGAVIAGVALGVATAAQITSGIALHNSIMNKKQIQELRKALSTTNKAIDEIRIAGERTLIAVQGVQDYINNVIIPMQEKLQCDILASQLSIALLRYYTNILTVFGPSIRDPITSTISIQALSQAFNGNLQALLDGLGYTGQDLHDLIESRSITGQIIHADMTDLFLILRINYPSITDMQGVVIYELNSITYHIGPEEWYTIMPNFIAVQGFLVSNFDERKCSITKTSILCQQNSIYPMSTEMQRCIKGEIKFCPRSKAIGTLVNRFILINGNLMANCLGIICRCYTSGQIITQDPNKLITIISQEECREVGVDGIRIMVGPKKLPDVIFNARLEIGVPISLSKLDVGTDLAIASAKLNNSKALLEQSDKILNSMSKLDSLNSRILGSVFIMMIIFVIVIVIIWIICKKCRNKRNKLSASIEPLYIPPSYNSPHSIVKSI

SEQ ID NO: 25 - DNA, 1560 bp, Feline paramyxovirus type 2
  misc_feature: FPaV-2 "TV25 strain" N antigen "wild-type" nucleic acid; given as DNA sequence
atggctagtttactcaggtcacttgcggcattcaagaaacacagagaacaaccaactgttccttctgggtcaggagggacgatcaaaggattaaaaaatacaattattgtgcctgttcctggagatacagtcatcactaccagatcgaacttactgttcagattagtctacataattggtaatccagatacacctttaagcacttcaacaggggcaataatatcattgttgacattatttgttgaatctccaggtcaattaattcaaagaatcgctgatgatcctgatgctgtttttaaattagtagaggtggttcctgaggttggtaatcctggagaattaacttttgcatctagaggaattaacttggataaacaagctcaacaatactttagattggctgagaaaaatgatcaaggatattatgtaagtttggggtttgaaaatccaccaaatgatgatgatataacgtcaagtcctgaaatcttaaattatattttagcatctgtacttgcacagatctggattctcctagctaaggctgtaactgctccagacacaggtggtgaggctgaaaatcgtaggtggattaaattgatgcaacaacgcagagtggatggtgagcttagattaagtaaaggatggttggacttagtgaggaataaaatcgcatcggatatcacaattagaaggtttatggtagcattagttcttgacattaaacgttctcctggaacaagaccaagaattgctgaaatgatttgtgatatagacaattatattgtggaggccggactggcaagttttctgttaactatcaaatttggtatagaaacacgttacccagcattggcgttacatgagttttcgggggaattagccactattgaaggactcatgaaattgtaccagtctatgggagaaatggcaccatacatggtcattctagagaattcgatccagactaggtttagtgctgggtcttatccgttactctggagctatgctatgggtgttggtgtagaacttgagagatcaatgagtggattaaacttcacaagaagtttctttgatcctacgtacttcaggttgggtcaggagatggtaagaaggtcttcaggaatggttaatagctcatttgctaaagaacttggactatctgaacatgaaacacaacttgttagccagatcattaactctggtggtgaatcaggtataccgaaatttgatggatttagagcaaacccaacaacatttctaggggctaaggacaacatcactgataggagtgaagatccattgattgcaattccagggtcatcaggacaaccattgccaggtcatgaccccaatatctcaggtgactcatatagaattgatagtagcactaaagacacgaacaatatatcagatggaggaacaaatccaagtcatgatgtttccaattctgctatggaagagctgagaagattggtagagtctaccaacaagattgatacaaagaaatctgaaagcccaggcattgttaatcattacaacgatactgaccttctgagataa

SEQ ID NO: 26 - protein, 519 aa, Feline paramyxovirus type 2
  MISC_FEATURE: FPaV-2 "TV25 strain" N antigen translated amino acid sequence
MASLLRSLAAFKKHREQPTVPSGSGGTIKGLKNTIIVPVPGDTVITTRSNLLFRLVYIIGNPDTPLSTSTGAIISLLTLFVESPGQLIQRIADDPDAVFKLVEVVPEVGNPGELTFASRGINLDKQAQQYFRLAEKNDQGYYVSLGFENPPNDDDITSSPEILNYILASVLAQIWILLAKAVTAPDTGGEAENRRWIKLMQQRRVDGELRLSKGWLDLVRNKIASDITIRRFMVALVLDIKRSPGTRPRIAEMICDIDNYIVEAGLASFLLTIKFGIETRYPALALHEFSGELATIEGLMKLYQSMGEMAPYMVILENSIQTRFSAGSYPLLWSYAMGVGVELERSMSGLNFTRSFFDPTYFRLGQEMVRRSSGMVNSSFAKELGLSEHETQLVSQIINSGGESGIPKFDGFRANPTTFLGAKDNITDRSEDPLIAIPGSSGQPLPGHDPNISGDSYRIDSSTKDTNNISDGGTNPSHDVSNSAMEELRRLVESTNKIDTKKSESPGIVNHYNDTDLLR

SEQ ID NO: 27 - DNA, 1476 bp, Feline paramyxovirus type 2
  misc_feature: FPaV-2 "TV25 strain" P antigen "wild-type" nucleic acid; given as DNA sequence
atgtcagcagaacaaatccaacaagttagacatggccttgaatccttgcaagagatcaaaaacaaccctccaccctctcaagatgtcaatcttgccagggaaatttacgaatccattaaacaaacaggaacaccttcaacacaaggagggaccattacaggaaataatactacgtcagggtgtgacaattactcaatgcatagccagggatcaggtccttctgtttcaggtgctgacaagaatatcgagagacttactggacccgattattcagaattatgggatccagaaggtaacctctgcatgctattcgaaagcgatgatgatgacaacaattattcagagattaatggccggtctaccgctatcgaaggattggatgaacagaataataaggacccaggtattaaacaatcaggagatcagtgttctgaaggagtgtctaagattaattcatcttctagtccccaagaagctacattatcttctgggagatctgatatatctgggacaggagtatctccctgtgcctctttggatataactgttaatgaattagaagatgcaactgttaagaatagtaataatatgaaaggaaattggccaatcccaaagttgcttgtcaaaccaccaccaagaatgaaatcactttctgactctgttacaccattaaaaggggccaccgacgggaaatcagtcttacctgggatggagattacattgtccgggaagaatggtgcaaccctacctgtacacccatttacacaacctgtaaaagactcaaatgcagatgtaagcaatgtccgtcaacatgtcccaagtgtgactgatggttatagtgatgataatgaggaagtacccggtttgcataaagaaactatagacaaagctgatctatctatgcaggacatatacaatttaattcttggatttaaggatgattacaggaaactatcaaataaattggatatgatactagagatgaaacaagatattgataatcttaaaaagagtagtgcaaaaatacaacttgcattatcaacaattgaaggacatctgtccagtgttatgattgctattccaggttcaggtattgatatgaatcaagatgagaagaaggatcaattaaactctgacttaaagccattactagggagggaccattgccgtgcatttcgtgaagtcactaatcctttagatgaaacgtcattgaccaacgctccgaccaaacatgttgctaagatcaacaaaaattgcactcttcagaaaatcaataagaatgagacatctgcaattaagtttgtacctaatgatagctatgcaagtatctcgactatcaagtctattgtcaaatcctcaaaccttaatcaagagcttaaagtcaagttactgacaattctatctcaaattaaaggggtagacaatattaaggagttttatgagaaagttatgatattgatcaagaataataactga

SEQ ID NO: 28 - protein, 491 aa, Feline paramyxovirus type 2
  MISC_FEATURE: FPaV-2 "TV25 strain" P antigen translated amino acid sequence
MSAEQIQQVRHGLESLQEIKNNPPPSQDVNLAREIYESIKQTGTPSTQGGTITGNNTTSGCDNYSMHSQGSGPSVSGADKNIERLTGPDYSELWDPEGNLCMLFESDDDDNNYSEINGRSTAIEGLDEQNNKDPGIKQSGDQCSEGVSKINSSSSPQEATLSSGRSDISGTGVSPCASLDITVNELEDATVKNSNNMKGNWPIPKLLVKPPPRMKSLSDSVTPLKGATDGKSVLPGMEITLSGKNGATLPVHPFTQPVKDSNADVSNVRQHVPSVTDGYSDDNEEVPGLHKETIDKADLSMQDIYNLILGFKDDYRKLSNKLDMILEMKQDIDNLKKSSAKIQLALSTIEGHLSSVMIAIPGSGIDMNQDEKKDQLNSDLKPLLGRDHCRAFREVTNPLDETSLTNAPTKHVAKINKNCTLQKINKNETSAIKFVPNDSYASISTIKSIVKSSNLNQELKVKLLTILSQIKGVDNIKEFYEKVMILIKNNN

SEQ ID NO: 29 - DNA, 6609 bp, Feline paramyxovirus type 2
  misc_feature: FPaV-2 "TV25 strain" L antigen "wild-type" nucleic acid; given as DNA sequence
atggagcaatcagattatcaagatattttatatccagaggtacatctcaacagtcctatagttatctctaaattagtgggtattttggagtattctaaggttgttcacaatcagcagttatctgatcacacaatagtcaagaatatacaatttagattgagaaatggattcaatagtccaagagtacaaacactgttagttatgggtgaaattatcaataaaatcaaaaataaatacccaaattatttgcacataccttatcctgaatgtaatcaaaagttatttaggatggctgacccggagttaacatctaaactagaagccctcttggacaaaggtgacacattatatcttaagattaagacagagatcatagcttgtttcgataagttaaaaactaaaatgagcataaccaatgatctgattagtgacaataggcagctaatttcagatctacctctaattgtcaagggatctcaatggtttttcccttttttgctctggttttctgttaaaactgagactaggaactgtattcgacaaaatcaaaaaactcgtgttaggtcacaataccgacctcatttgtcagaaactaaaagaattacgctggtcgttacccctgacttgatcacaatatttgaccacgtcaacaaatgtatatatcatctgacttttgagatgttgttgatgtattgtgatgtagtagaagggaggttaatgaccgaagcatctatgagtctagatcacagatttattaacctattgtcgagggtccagtatatgtgggatctattagatgggatgtttgagagtctaggaaatcagctatattcaatcattgcactcttagaacctctctctcttgcctatctacagttgatggatgcagacccacagatacggggtacatttttacaccattgcctttcagagttggaagaactcttatttagtaaatccccttttgatcctgtgatttatgaaaatctaattagtggacttgattacatctatttaacagacgatattcatttaactgctgagatattttctttctttagaagttttggtcatccttatttagaagcacaaaatgcagctagcaatgttaggaaatatatgaatcaacctaaagttatctcataccagactctaatgcaaggacatgcaattttttgtggcattataataaatgggttcagagatcgtcacggagggacatggccacctgtagagctaccacatcatgcatccgctgtaattagaaatgctcagttatctggagaaggattaacacctgagcagtgtgctcaatactggaggtcattttgtggatttaaatttaaatgttttatgccattaagtctagatagcgacctcaccatgtaccttagagataaggcattatcacctattaagaatgagtgggattctgtgtatgctaaagagtatttaagatacaaccctggcttaccgactagctctcgaagattagtcaatgtatttctagaagatgataaatttgatccgtacgaaatgattatgtacgtaataaacggtgattatttaagggataatgagttcaatctctcatatagtcttaaagaaaaggagatcaaggaggtaggccgattgttcgctaaaatgacttataagatgagagcttgtcaggtaatagcagaaaatttaattgcaaatggagttgggaaattttttaaagacaatgggatggcgaaggatgaacataaattaaccaaaacattacataagctggctatttctggtgtacctaaagataattctcaactctatttaagtgaatgttgggaacaagtggtagaacaatgcgtaaccagtacgcaaacaaaaaatcaaattatcagttcacactcaggaaaatcagttgcatcaaagttttcaagatcaaatcccaatgataggggtattctaaatagtggtagacatttgaataaacatccaaaacatccatcaaacaccgaatactatgaaactgtcagtagttttataactactgatctcaagaaatattgcctcaactggcgctatgaatcaagtagtgtgtttgcagaaagactcaatgagatttatgggttaccaggatttttccattggcttcatagaattttggagaaatctgtattatatgttagtgatccatccagtccacctgattttgatcaacatgtcgatattgattcagttccaaatgatcatatttttatcaaatacccaatgggtgggataaaaggattttgtcaaaaattatggacaatcagcacaatcccatttttatatttagcagcctttgatacaggggttagaatatcttcgttggttcaaggtgataatcaagcaattgcagtgaccaaaagagttccatcatcctggagttattcgagaaaaaaagaggagtcaactaaagttacaacacaatattttttaaacttgagacaacgcttacatgatataggtcatgagttaaaggcaaatgagactattatatcttcacacttttttgtttactctaagggtatttattatgatggtatacttctttcacaatcccttaaaagtattgcaagatgtgttttttggtccgagacaattgtcgatgagactaggtcagcttgcagcaatatatccactacccttgctaaagctattgaacggggttatgataaatttgtagcatacgctattaatatatataagactatacaccaggtcttaattgcattatcttttactattaatcccactatgactccggacataacagaacctttttataaaagtttagatttacttaaaaacctcattctgataccagcaccattgggtgggatgaattacatgaatatgagcagattatttgttaggaacataggtgatcccattacagcttcatttgctgacatcaagcgtatgatcgaatgcgggttattagggcacaatgttctctcacaaataatgtatcagaaatgtggtacctcgaaatacttagattgggctagtgacccttattccataaatcttccttatagtcaaagcatgaccaaagtattaaaaaatataaccgcgagatatgttctcatgcatagtcctaaccctatgctaaaagatttattccatgagaagtcacaagaagaggatgagattcttgctgaatttttgctggatcgtcagttaataatccctagagctgcacatgaaattttatcgaattcagtaacaggagctagagagtcgattgcagggatgcttgatactactaaaggacttattcgagccagtatgtcaagaggtggtctgacatcttcacttgttttgaaattgtcaacatatgattatcaacaatttagaacatgccttgaatggctttatgcccctaccacaggaatagcagtaagtgctgattcttgttcagtttttttagccagagctattcgaaaaaggatgtgggttcacctgactaaaggaagagaaatttatggcctagaagtgcctgatatattagaatgtatgcagagcaatgtaattgttgatcatgaagattgttattcatgtattcaaggatcaagatactacacatggttttttgtaccttctaattgtcagcttgatcagattaacaagtctacaaattctctacgggttccttacattggctctactacagaggaaagaagtgacatgaaattatcatacgtcagatcccctagtaggccacttaaggcagcagtccgaattgcagcagtctacacatgggcatacggtgatgacgatctgtcttggcgtgaggcttggtacttggcaaggactagggcaaatgttactttcgatgagcttaaattagtaacacccatagctacctctactaacttggcacatagattaagggacaggagtactcaagttaagtattcaggaacttcattggtaagagtggcacgctatacaacaatatccaatgataatatgtcatttgttattaatgacaaaaaggtagatactaattttgtctatcaacagggcatgttattgggtttgagtatcctagaatatatatttagatactgtaaaagtactggtcaatcaaatactgtagttcacttgcatgcagatgttaattgttgcataatccaaatgacagatcaaccttatactccaagcttaacgaaaaaattacctgagattaaacctattaataataaattgatttatgatccagctcctataattgatactgatgcagctaggttatattctcagaagtacttatcacacctgatagattttccaaattggtcaatgaatcagctaaatgtagttttagcaaaagtagttgcaatatctattgtggacttgataactaaagcgagtaaagatcatctcaatgaaattatggcagttgttggagatgatgacattaatagctttataacagaatttttgctagttgatccgaggctatttacattgtacttaggtcaatacacgtcacttcaatgggcatatgaaattcattatcaccgacccgtaggcaaataccagatggcagaagtgttacacactttactgtcaagagcaagtaaaggtatatttaatatattgactaatgcctttagtcatcctagagtttacaaaagattttgggaatgtggattactggagcctatttatggaccatacatagggagccaaaatttatatagtacagtaattgattacctttacaatgcttatataacttatttagatgcttatctatctgatcatatcgaagatgcagacatagtaatatgtgagacagaagaaacttgtctagctaataggattgataactatcaaggtaggcatctcgccgtacttattgatctttattgtgattctactaggtgtcctaatataaaagggtcagacacaatcatgcgaaactcaattctcaaatcttttattgataatgagagaaggacaagtccattaggtctaacatggaatcttgatccattactcatagatcatttcagttgttcaattacttatctgaggagaggtattattaaacagattaggctaaggtttgatccaaacatatctattgagttggttaaattggcaaaacctgaagtgattcatcaaggaccaaaaataccgtcttcttgggcccttatagatattaatcctgaggtcaatgatcttaatacagttttcggagaattaaatagtaaatggaaagatattcctattggacaaattagaattcaaaattttgagatccatgcttaccgaagaattggagttaattcaactgcatgttataaagcattggaaatgctatctgtactaactcggtttatgtctaacccagcaggagctttgtttttaggagagggtgcagggtcaatgttagttacctatcgtgcgtttatcccgttcaagagaatttattataatagtggagtttctatacaaaatattcaaagccaaagggaactaagtctatacccatctgaagtagccttggtcgataataaaaatcgtttgaccagtgatcctgatatcaaagtcttatttaatggcaagccagaatccacgtgggttgggaatatagactgctttgcttatattctgagtcatattgaaacttctagtttaacattaatccacagtgatattgaatctagcttgagtaaaacaaagaataagattcttgaggagctttgccatattctatcaatggcactgattctaggaaagattggatctgtattagttattaagctattaccacgggttggtgactacacatattcattttgcaagtatgcgtcagaattctaccaacagaatttcttcattttacctagatttagtaacatgtcatcatctgaaatttactacgttggagttcatttaaataccaatagactggttgatccagataggattgtgcaatatataatcaggaatctccaatctactccagtcactttcttatcttacattttggaaactaaatatagaaataatatggttacaaattatgggctctgtttgtctgatggacataaaagcgattacttgtcatcaatcaccaagatagaaaatgttcttttatcatgtggattggaattgaatggacctaagattattcagcaattatctggacatgactacgccaatggagagattagcttagaatcaagtataatggtactggtcagagaatatctaaatgcaactatccaaggtcgagaaacactaggtcttttttcaccttaccctgtgttacatgagagtcagttaagagaaattaacaggtgcattgcattgaagtatgttgtatatttacttttttactcaacctctgtaggatctagtagacagatcatgagcaatctcagaaaaggagtattaatgtatgacttaagagatgagtttttcatggaaaggttatcaacaaatttcaagaaaaaaataatgtcacaagaggttaaaactacatggatctttaatattgatgtaccaacaagaaaagctctgtataaattagttggttattcacttatcattaatcacgtataa

SEQ ID NO: 30 - protein, 2202 aa, Feline paramyxovirus type 2
  MISC_FEATURE: FPaV-2 "TV25 strain" L antigen translated amino acid sequence
MEQSDYQDILYPEVHLNSPIVISKLVGILEYSKVVHNQQLSDHTIVKNIQFRLRNGFNSPRVQTLLVMGEIINKIKNKYPNYLHIPYPECNQKLFRMADPELTSKLEALLDKGDTLYLKIKTEIIACFDKLKTKMSITNDLISDNRQLISDLPLIVKGSQWFFPFLLWFSVKTETRNCIRQNQKTRVRSQYRPHLSETKRITLVVTPDLITIFDHVNKCIYHLTFEMLLMYCDVVEGRLMTEASMSLDHRFINLLSRVQYMWDLLDGMFESLGNQLYSIIALLEPLSLAYLQLMDADPQIRGTFLHHCLSELEELLFSKSPFDPVIYENLISGLDYIYLTDDIHLTAEIFSFFRSFGHPYLEAQNAASNVRKYMNQPKVISYQTLMQGHAIFCGIIINGFRDRHGGTWPPVELPHHASAVIRNAQLSGEGLTPEQCAQYWRSFCGFKFKCFMPLSLDSDLTMYLRDKALSPIKNEWDSVYAKEYLRYNPGLPTSSRRLVNVFLEDDKFDPYEMIMYVINGDYLRDNEFNLSYSLKEKEIKEVGRLFAKMTYKMRACQVIAENLIANGVGKFFKDNGMAKDEHKLTKTLHKLAISGVPKDNSQLYLSECWEQVVEQCVTSTQTKNQIISSHSGKSVASKFSRSNPNDRGILNSGRHLNKHPKHPSNTEYYETVSSFITTDLKKYCLNWRYESSSVFAERLNEIYGLPGFFHWLHRILEKSVLYVSDPSSPPDFDQHVDIDSVPNDHIFIKYPMGGIKGFCQKLWTISTIPFLYLAAFDTGVRISSLVQGDNQAIAVTKRVPSSWSYSRKKEESTKVTTQYFLNLRQRLHDIGHELKANETIISSHFFVYSKGIYYDGILLSQSLKSIARCVFWSETIVDETRSACSNISTTLAKAIERGYDKFVAYAINIYKTIHQVLIALSFTINPTMTPDITEPFYKSLDLLKNLILIPAPLGGMNYMNMSRLFVRNIGDPITASFADIKRMIECGLLGHNVLSQIMYQKCGTSKYLDWASDPYSINLPYSQSMTKVLKNITARYVLMHSPNPMLKDLFHEKSQEEDEILAEFLLDRQLIIPRAAHEILSNSVTGARESIAGMLDTTKGLIRASMSRGGLTSSLVLKLSTYDYQQFRTCLEWLYAPTTGIAVSADSCSVFLARAIRKRMWVHLTKGREIYGLEVPDILECMQSNVIVDHEDCYSCIQGSRYYTWFFVPSNCQLDQINKSTNSLRVPYIGSTTEERSDMKLSYVRSPSRPLKAAVRIAAVYTWAYGDDDLSWREAWYLARTRANVTFDELKLVTPIATSTNLAHRLRDRSTQVKYSGTSLVRVARYTTISNDNMSFVINDKKVDTNFVYQQGMLLGLSILEYIFRYCKSTGQSNTVVHLHADVNCCIIQMTDQPYTPSLTKKLPEIKPINNKLIYDPAPIIDTDAARLYSQKYLSHLIDFPNWSMNQLNVVLAKVVAISIVDLITKASKDHLNEIMAVVGDDDINSFITEFLLVDPRLFTLYLGQYTSLQWAYEIHYHRPVGKYQMAEVLHTLLSRASKGIFNILTNAFSHPRVYKRFWECGLLEPIYGPYIGSQNLYSTVIDYLYNAYITYLDAYLSDHIEDADIVICETEETCLANRIDNYQGRHLAVLIDLYCDSTRCPNIKGSDTIMRNSILKSFIDNERRTSPLGLTWNLDPLLIDHFSCSITYLRRGIIKQIRLRFDPNISIELVKLAKPEVIHQGPKIPSSWALIDINPEVNDLNTVFGELNSKWKDIPIGQIRIQNFEIHAYRRIGVNSTACYKALEMLSVLTRFMSNPAGALFLGEGAGSMLVTYRAFIPFKRIYYNSGVSIQNIQSQRELSLYPSEVALVDNKNRLTSDPDIKVLFNGKPESTWVGNIDCFAYILSHIETSSLTLIHSDIESSLSKTKNKILEELCHILSMALILGKIGSVLVIKLLPRVGDYTYSFCKYASEFYQQNFFILPRFSNMSSSEIYYVGVHLNTNRLVDPDRIVQYIIRNLQSTPVTFLSYILETKYRNNMVTNYGLCLSDGHKSDYLSSITKIENVLLSCGLELNGPKIIQQLSGHDYANGEISLESSIMVLVREYLNATIQGRETLGLFSPYPVLHESQLREINRCIALKYVVYLLFYSTSVGSSRQIMSNLRKGVLMYDLRDEFFMERLSTNFKKKIMSQEVKTTWIFNIDVPTRKALYKLVGYSLIINHV

SEQ ID NO: 31 - DNA, 1788 bp, Feline Morbillivirus
  misc_feature: FeMoV "Lapön strain" H antigen "wild-type" nucleic acid; given as DNA sequence
atggagtccaacaacattaaatattacaaagactctaatcggtatcttggtaaaatattagatgaacacaagacagttaataatcaattgtacaggttgagtattaaagtaattaccattattgctattattgtaagcttaattgcaacaataataactattattaatgccacaagtggaagaactaccctaaacagtaatacagacatactgcttagccaaagagatgagattcatagtattcatgaaatgatatttgaccgtatttatcctttgataactgctatgagtacagagctaggacttcatattcctactttattagatgaacttactaaagcaattgatcaaaaaattaaaataatgaatcctcccgttgatactgtaacatctgatcttaactggtgtatcaaacctcctaatgggattattatggatccaaaaggttattgcgaaagtatggaattatctaaaacttacaaattattgcttgatcagttagatgtctcaagaaagaaatcgctcattataaatagaaagaatatcaaccagtgtcaattagttgatgactcaaagatcacttttgctactgttaatatacaatctacaccaaggtttttaaattttggtcatacagtcagcaatcaacgtataacatttggtcaaggaacttatagtagtacttatattataactatccaagaagatggaataaatgatgttcaatatcgagtgtttgaaattggatatatctctgatcagtttggttttttcccctcattaatagtatctagggtattgcctatacgtatggtattgggaatggaatcctgtaccttgacgagtgatcgacaaggtgggtatttcttatgtatgaatacattaacacggtctatatatgattatgtcaatataagagatttgaaatcactatacataacacttcctcattatggtaaggttaattatacttacttcaattttgggaaaattaggagcccacatgagattgataaaatttggctaacgtccgaaagaggtcaaattatttctggttattttgcagcatttgtcacaattacgattcgaaattataataattatccctacaaatgtttgaataatccatgttttgacaactctgagaattactgtaggggatggtataagaacataacaggcaccgatgatgttccaatactagcatacttactagttgaaatgtatgatgaagaaggacctttaattacacttgtagcaataccaccttacaattatacagctccatctcataattctctttactatgatgacaaaattaataagttgataatgactacatctcacactgggtatatacagatcaatgaggtgcatgaggtgattgttggtgatgatttaaaggctattctcctgaacagattatctgatgaacaccctaatcttacagcctgtagacttaatcaaggcattaaagagcagtacaagtccgatggaacgataatttcaaattctgcacttattgatatacaagaacgaatgtatattacagtcaaagctattccaccagtaggtaactataactttacagttgagttgcactctagatcaaacacatcttatatattgttaccgaaacagttcaatgccaagtatgacaaattacatcttgagtgctttaattgggacaagtcttggtggtgtgctttgatacctcaattttcattaagttggaatgaatccctttctgttgatactgctatttttaatttaataaattgtaaatga

SEQ ID NO: 32 - DNA, 1784 bp, Feline Morbillivirus
  misc_feature: FeMoV "Lapön strain" H antigen nucleic acid that has been codon-optimized for expression primarily in felines; given as DNA sequence
atggaaagcaataacatcaagtactataaagacagcaacaggtatctgggaaaaattctggacgaacataagacagtcaataatcagctgtacaggctgtctatcaaggtgatcaccatcatcgccatcatcgtgagcctgatcgcaaccatcatcactatcatcaacgccacttccggcagaaccactctgaactctaataccgacatcctgctgagccagagggatgagatccactccatccatgaaatgatcttcgacagaatctatccactgatcaccgccatgtctactgagctggggctgcacatccctactctgctggacgaactgaccaaagcaatcgatcagaagatcaaaatcatgaacccacctgtggacaccgtgactagcgatctgaactggtgcatcaagcccccaaatggaatcatcatggatccaaaaggttactgtgagtctatggaactgagcaagacctataaactgctgctggaccagctggatgtgtccaggaagaaatctctgatcatcaacagaaagaacatcaatcagtgccagctggtggacgatagcaaaatcaccttcgcaactgtgaatatccagtccactcctaggttcctgaactttggacatactgtgtccaatcagagaatcacctttggacagggtacctacagctccacttatatcatcaccatccaggaagacggtatcaacgatgtgcagtacagggtgttcgaaatcggctatatctctgaccagtttgggttctttcctagcctgatcgtgtccagggtgctgcccatcagaatggtgctgggcatggagtcttgcaccctgactagcgatagacagggcgggtacttcctgtgtatgaacaccctgactaggtccatctacgactatgtgaatatcagagatctgaagtctctgtacatcactctgccccactatggaaaagtgaactacacctatttcaattttggaaagatcaggagcccacatgagatcgacaaaatctggctgacctctgaaagaggccagatcatcagcgggtacttcgccgcatttgtgaccatcactatcaggaactataacaattacccctataagtgcctgaacaatccatgttttgacaactccgagaattactgcagaggatggtataagaatatcaccggtactgacgatgtgcccatcctggcctacctgctggtggaaatgtatgatgaggaaggaccactgatcactctggtggccatccctccctacaactataccgcacctagccacaattccctgtactatgacgataagatcaacaaactgatcatgaccactagccacactggctacatccagatcaatgaggtgcatgaagtgatcgtgggggacgatctgaaggccatcctgctgaacaggctgagcgatgagcatcccaacctgactgcatgtagactgaatcagggcatcaaggaacagtataaatccgacgggaccatcatctctaatagcgccctgatcgatatccaggagaggatgtacatcactgtgaaagcaatcccacctgtgggcaactataatttcactgtggaactgcactccagatctaacacctcctacatcctgctgcctaagcagttcaatgccaagtatgacaaactgcatctggagtgctttaactgggataaatcctggtggtgtgcactgatcccccagttttctctgtcctggaacgaaagcctgtccgtggataccgcaatcttcaatctgataaactgtaa

SEQ ID NO: 33 - protein, 595 aa, Feline Morbillivirus
  MISC_FEATURE: FeMoV "Lapön strain" H antigen translated amino acid sequence
MESNNIKYYKDSNRYLGKILDEHKTVNNQLYRLSIKVITIIAIIVSLIATIITIINATSGRTTLNSNTDILLSQRDEIHSIHEMIFDRIYPLITAMSTELGLHIPTLLDELTKAIDQKIKIMNPPVDTVTSDLNWCIKPPNGIIMDPKGYCESMELSKTYKLLLDQLDVSRKKSLIINRKNINQCQLVDDSKITFATVNIQSTPRFLNFGHTVSNQRITFGQGTYSSTYIITIQEDGINDVQYRVFEIGYISDQFGFFPSLIVSRVLPIRMVLGMESCTLTSDRQGGYFLCMNTLTRSIYDYVNIRDLKSLYITLPHYGKVNYTYFNFGKIRSPHEIDKIWLTSERGQIISGYFAAFVTITIRNYNNYPYKCLNNPCFDNSENYCRGWYKNITGTDDVPILAYLLVEMYDEEGPLITLVAIPPYNYTAPSHNSLYYDDKINKLIMTTSHTGYIQINEVHEVIVGDDLKAILLNRLSDEHPNLTACRLNQGIKEQYKSDGTIISNSALIDIQERMYITVKAIPPVGNYNFTVELHSRSNTSYILLPKQFNAKYDKLHLECFNWDKSWWCALIPQFSLSWNESLSVDTAIFNLINCK

SEQ ID NO: 34 - DNA, 1014 bp, Feline Morbillivirus
  misc_feature: FeMoV "Lapön strain" M antigen "wild-type" nucleic acid; given as DNA sequence
atgactgagatattcaatcttgatgaaagctcatggtcagtcaaaggaacacttgatccactaacccctgatacctatcctgatgggcgacttgtacctaaagtccgggtaatcgatccaggtttaggagatcgcaagagtggagggtatatgtatctacttcttcatggtgtcatagaagatagtgaaaccatggttagcccgaaaggaagagcatttggggcgttcccattaggagtaggtcagtcaactgaaaacccagaagatttgtttaaagaagtattaaccctcaacattgtaactcgtaggactgctggctttaatgaaaaattagtttattataataccacgcctctacacttattgactccctggaagaaagtgttggcgtatgggagcattttcaatgctaatcaggtctgcagtgatacaagttctatcccgatagatattccacaaaaatttagacctgtatacttgactattacaaaattatctgacgatggctattatcagataccgaagatgatccaagatttcaaatcatcaaattctgttgcatttaatatccttgtgcatttatcaatgggcacaactttaattgaccaatccaaagaccctcgattaagaagtgctccagaaactatgatcacattcatgattcatattggaaatttcaaacggaagagtaacaaatcttattctcctgaatactgcaagagaaaaataataagacttggtttgatattctcattaggtgcaattggcggcacaagcttacatattagatgtacaggtaagatgagcaaacggctacaggcttatctaggattcaaaaggactctatgttaccccctgatgtatgggaatgaagggttgaataaaactctggggagaaatgaatgtaaaatagaaaaggttcaagcggttctacagccatcagttccaaatgaattcaagatatacgatgatgtcattattgacaataccaatggtcttttcaagattaagtag

SEQ ID NO: 35 - DNA, 1014 bp, Feline Morbillivirus
  misc_feature: FeMoV "Lapön strain" M antigen nucleic acid that has been codon-optimized for expression primarily in felines; given as DNA sequence
atgaccgagatcttcaacctggacgagagcagctggagcgttaaaggcacactggaccccctgacccctgacacttaccctgacggaaggctggtgcccaaagtgagagtgatcgacccaggcctgggggataggaaatccggcgggtacatgtatctgctgctgcacggcgtgatcgaggacagcgaaaccatggtgtcccctaagggaagagccttcggtgcatttcccctgggagtgggacagtctaccgagaacccagaagatctgttcaaagaggtgctgactctgaatatcgtgaccaggagaactgccggctttaacgaaaaactggtgtactataataccactcctctgcatctgctgaccccctggaagaaagtgctggcctacgggagcatcttcaacgcaaatcaagtgtgttccgacactagctccatccccatcgatatcccacagaagtttaggccagtgtatctgaccatcactaaactgtctgacgatgggtactatcagatccctaagatgatccaggacttcaaatctagcaactctgtggcctttaatatcctggtgcacctgagcatgggaaccactctgatcgaccagtctaaggacccaaggctgagaagcgcacctgagactatgatcactttcatgatccatatcggtaacttcaagagaaagagcaacaagtcctactctcccgaatattgcaagaggaaaatcatcagactgggcctgatcttctccctgggggccatcggaggtacctctctgcacatcaggtgcactggaaagatgtccaaaagactgcaggcatacctgggttttaagaggaccctgtgttacccactgatgtatggcaacgaggggctgaataaaactctgggcagaaacgagtgcaagatcgaaaaagtgcaggcagtgctgcagccatccgtgcctaatgagttcaagatatacgacgatgtcataatagataatactaatggtctgttcaagataaaatag

SEQ ID NO: 36 - protein, 337 aa, Feline Morbillivirus
  MISC_FEATURE: FeMoV "Lapön strain" M antigen translated amino acid sequence
MTEIFNLDESSWSVKGTLDPLTPDTYPDGRLVPKVRVIDPGLGDRKSGGYMYLLLHGVIEDSETMVSPKGRAFGAFPLGVGQSTENPEDLFKEVLTLNIVTRRTAGFNEKLVYYNTTPLHLLTPWKKVLAYGSIFNANQVCSDTSSIPIDIPQKFRPVYLTITKLSDDGYYQIPKMIQDFKSSNSVAFNILVHLSMGTTLIDQSKDPRLRSAPETMITFMIHIGNFKRKSNKSYSPEYCKRKIIRLGLIFSLGAIGGTSLHIRCTGKMSKRLQAYLGFKRTLCYPLMYGNEGLNKTLGRNECKIEKVQAVLQPSVPNEFKIYDDVIIDNTNGLFKIK

SEQ ID NO: 37 - DNA, 1632 bp, Feline Morbillivirus
  misc_feature: FeMoV "Lapön strain" F antigen "wild-type" nucleic acid; given as DNA sequence
atgggtaaaattaaggttataataattagctctttactactatcaactattacgactgcacaagtaggttgggacaatttaacttcgattggagttataagtactaagcaatatgattataaaataaccactttgaatactaaccagttgatggttataaagatggtccccaatatatcatcaatcatcaattgcaccaagcctgagttgattaaatatcgagagttggtcttaggggttattagaccaatcaatgaatcgttagaattgatgaattcatacattaacatgaggacaggttcagagagattcataggggctgtaatagctggagttgcattgggtgtggcaactgcagcgcaaataacatcaggaattgcattacataactcaattatgaacaaaaagcaaatacaagaattgaggaaggccctcagtaccaccaataaagcaattgatgaaataaggattgcaggtgagagaacattaatagcagtccaaggtgtacaagattacattaataatataattattcctatgcaggacaaacttcaatgtgatattttatcatcacagcttgctattgccttactcaggtattatacaaatatattgacagtttttgggccaagcatacgagatcctgttactagtacaatctcaatacaagcacttagtcaggcgtttaatggtaatctccaggcattgcttgatggattaggatataccgggagagacttacgtgatcttttagagagtagatctattactggtcagataattcatgcagatataactgatttgttccttgtcctcagaattaactatccttctataactgaaatgcagggagtaacgatatatgaacttaattcaattacatatcatattggacctgaggaatggtatactattatgcctaattttatagctgttcagggttttttaacatccaatttcgatgaaaggaagtgctcaataactaaatcaagtatactgtgccaacaaaattcaatttacccgatgtcaacagaaatgcaaagatgtatcaagggtgagataagattctgtccaagatccaaagcaattggaacattagttaataagtttatcttgactaaaggtaatttaatggctaattgccttggtattatatgcaggtgttatacttcaggccaaattataacacaagaccctagtaagttaattacaataatatcacaagaggaatgcaaagaagttggagttgatggtatccgtattatggtaggacctaggaaattaccagacattacctttaacgctaggttagaggttggtgtgccgatatcattaagtaaattagatgtaggaactgatttagcaattgcttcagctaaacttaataattctaaggcactgttggaacaatcagataaaattctggactcaatgtctaaattggattctattaattcacgaatcacagggttgatcttggcaatcatggtaatctttataatcatcgttactattgtctggatcatatacaaaagatgcagaaataaagataataaattcagtacttcaattgaaccgctttatatacctccttcttacaactcacctcacagtgtggttaagtctatttga

SEQ ID NO: 38 - protein, 543 aa, Feline Morbillivirus
  MISC_FEATURE: FeMoV "Lapön strain" F antigen translated amino acid sequence
MGKIKVIIISSLLLSTITTAQVGWDNLTSIGVISTKQYDYKITTLNTNQLMVIKMVPNISSIINCTKPELIKYRELVLGVIRPINESLELMNSYINMRTGSERFIGAVIAGVALGVATAAQITSGIALHNSIMNKKQIQELRKALSTTNKAIDEIRIAGERTLIAVQGVQDYINNIIIPMQDKLQCDILSSQLAIALLRYYTNILTVFGPSIRDPVTSTISIQALSQAFNGNLQALLDGLGYTGRDLRDLLESRSITGQIIHADITDLFLVLRINYPSITEMQGVTIYELNSITYHIGPEEWYTIMPNFIAVQGFLTSNFDERKCSITKSSILCQQNSIYPMSTEMQRCIKGEIRFCPRSKAIGTLVNKFILTKGNLMANCLGIICRCYTSGQIITQDPSKLITIISQEECKEVGVDGIRIMVGPRKLPDITFNARLEVGVPISLSKLDVGTDLAIASAKLNNSKALLEQSDKILDSMSKLDSINSRITGLILAIMVIFIIIVTIVWIIYKRCRNKDNKFSTSIEPLYIPPSYNSPHSVVKSI

SEQ ID NO: 39 - DNA, 1560 bp, Feline Morbillivirus
  misc_feature: FeMoV "Lapön strain" N antigen "wild-type" nucleic acid; given as DNA sequence
atgtcgagtctactaaggtcacttgctgcatttaaaagacatagggagcaaccaactgcaccgtcaggctcaggtggtacaattaaaggattgaagaatacaattattgttccagttccaggggatacagtaattactacgaggtctaacttgttatttagattagtttatataataggcaatccagatacacctttaagtacctcaacgggagcaataatatcattgctgaccctatttgttgaatcccccggtcaattaattcaaaggattgctgatgatcctgacgcagtttttaaattagtagaagtcattcctgaagtcggtaatcctggagagctgacttttgcatctcgaggaattaatttggataagcaagctcaacaatatttcaaactggctgaaaaaaatgatcaggggtattacgttagcttaggatttgagaacccaccaaatgatgacgatataacatctagtcctgagatatttaattatattctggcatctgtacttgcacaggtttggattcttctggcaaaagctgttactgccccagataccgctgctgaggctgaaaaccgtagatggattaagttgatgcagcaacgtagagtggatggtgaactaagattgagcaaaggatggctggatctggtgaggaacaagattgcatcagatattacaataagacgattcatggtagcattagtccttgatatcaaacgttcccccggaacaagaccaagaatagctgagatgatttgtgatattgataattatattgtagaagcagggcttgcaagctttttgttgactatcaaatttggcatagaaacacgttacccagcattggcattacatgaattttctggagaactagctaccattgaggggcttatgaaattgtaccaatctatgggggaaatggcaccttacatggtaattctggaaaattcaatccaaaccaggttcagtgcagggtcttatcctctgttatggagttatgctatgggtgttggcgtagagcttgaaagatcaatgggtggacttaattttactaggagtttctttgatcctacatatttcagacttggtcaggagatggtgcgaagatcttcagggatggttaatagttcatttgcaagagaacttgggttgtctgaacatgagacacaacttgtcagccaaattgtcaattctggaggtgaatctggtatacctaagtttgatggattcagagcaaatcctacaacttttctaggagccaaggacaacataaatgatggaggtgaggaccagtcaaattcagtatcaggattgcctggaccaatattgccaagtcatgacttgaatctgtcaggtgattcatatgggaatgatagtggtatgaaaaatgtcaacgacagactaaatgaaggagtaagtccagaccatgatgtttctagctctgccatggaagaattaaggagattggttgagtctactaacagaattgacactaaaaagccagaggctccaggtgttactaaccattacaatgatactgaccttctgaaataa

SEQ ID NO: 40 - protein, 519 aa, Feline Morbillivirus
  MISC_FEATURE: FeMoV "Lapön strain" N antigen translated amino acid sequence
MSSLLRSLAAFKRHREQPTAPSGSGGTIKGLKNTIIVPVPGDTVITTRSNLLFRLVYIIGNPDTPLSTSTGAIISLLTLFVESPGQLIQRIADDPDAVFKLVEVIPEVGNPGELTFASRGINLDKQAQQYFKLAEKNDQGYYVSLGFENPPNDDDITSSPEIFNYILASVLAQVWILLAKAVTAPDTAAEAENRRWIKLMQQRRVDGELRLSKGWLDLVRNKIASDITIRRFMVALVLDIKRSPGTRPRIAEMICDIDNYIVEAGLASFLLTIKFGIETRYPALALHEFSGELATIEGLMKLYQSMGEMAPYMVILENSIQTRFSAGSYPLLWSYAMGVGVELERSMGGLNFTRSFFDPTYFRLGQEMVRRSSGMVNSSFARELGLSEHETQLVSQIVNSGGESGIPKFDGFRANPTTFLGAKDNINDGGEDQSNSVSGLPGPILPSHDLNLSGDSYGNDSGMKNVNDRLNEGVSPDHDVSSSAMEELRRLVESTNRIDTKKPEAPGVTNHYNDTDLLK

SEQ ID NO: 41 - DNA, 1476 bp, Feline Morbillivirus
  misc_feature: FeMoV "Lapön strain" P antigen "wild-type" nucleic acid; given as DNA sequence
atgtcctctcaccaaatccaacaggttaaacatggcctcgaatctttacaagagatcaaaaacaaccctccatcttcccaagatgtcaatcttgccagggagatttacgaatccattaaacaaacaggaacaccttcagtgcaaggaggagccattacgggagataatactacgccagggggtaacaattacacaatgtatagccaaggaccaagtccttctattccaagtgttaacaagaatatcgaaggacttactggatccgatcattcaggactatgggatccagaggataacctctgcatgttattcgaaagcgatgatgatgaaaaccattattcagagattaatggccggccttccactatcgaaagattggatgaacaggataatgagaacccaagtattaaacaaccaggaaatcaatgtactgaaggagtgtttaagactgattcatcttctaattcccaagaaactacactacctgttgggagatctgatatacctgggacaggaatatcaacctgtgcctctttggatataaccgtaaatgaactcgaggatgcaactgtaagaaatagcgacaatatgaagggaaactggccaataccaaagttacttgttaagccaccacccagggcaaaatcaagcgttgatcatagcaatccattaaaaggggccacaggagggaaattagtcttacctgggatggagactacattgtccgggaagagtggtgtaaccccatctgtgcacctatctactcaacctgtaaacgacttcaatgtaaatgtaagcaatgcccgtcaacctgccccaaatgtgaataatgatcacagtgacagtggggtaatagtgcccaacttacataaagacattgaagataagtctgaaatatccattcaagatatatacaacttaatacttgggtttaaggatgattatagaaaattgtctaataaactggatatggtattagagatgaaacaagatattgacaatcttaaaaagagtagtgctaaattacaattggcattatcaactattgagggacatctatctagtgttatgatcgctattccagggtcaggtattgattccaccggggatgagaaaaaggatcagatgaacactgacttaaagccgttattggggagggatcattgcagagcatttcgagaagttaccagtcctttagatgagatgtcattagccaattctcccacaaaacatgttgctaaaataaacaaaaactgcacccttcagaaaatcaataagaatgaaacatctgcaatcaaatttgtccccaatgatagtcatgcaagcacatcaaccatcagatcaatcatcagatcatccaatcttgatcaggatttgaaaacgaaactactcacaattctatctcagattcgggggatagataatattaaggaattttatgaaaaagtcatgatactaataaagaataggaactaa

SEQ ID NO: 42 - protein, 491 aa, Feline Morbillivirus
  MISC_FEATURE: FeMoV "Lapön strain" P antigen translated amino acid sequence
MSSHQIQQVKHGLESLQEIKNNPPSSQDVNLAREIYESIKQTGTPSVQGGAITGDNTTPGGNNYTMYSQGPSPSIPSVNKNIEGLTGSDHSGLWDPEDNLCMLFESDDDENHYSEINGRPSTIERLDEQDNENPSIKQPGNQCTEGVFKTDSSSNSQETTLPVGRSDIPGTGISTCASLDITVNELEDATVRNSDNMKGNWPIPKLLVKPPPRAKSSVDHSNPLKGATGGKLVLPGMETTLSGKSGVTPSVHLSTQPVNDFNVNVSNARQPAPNVNNDHSDSGVIVPNLHKDIEDKSEISIQDIYNLILGFKDDYRKLSNKLDMVLEMKQDIDNLKKSSAKLQLALSTIEGHLSSVMIAIPGSGIDSTGDEKKDQMNTDLKPLLGRDHCRAFREVTSPLDEMSLANSPTKHVAKINKNCTLQKINKNETSAIKFVPNDSHASTSTIRSIIRSSNLDQDLKTKLLTILSQIRGIDNIKEFYEKVMILIKNRN

SEQ ID NO: 43 - DNA, 6609 bp, Feline Morbillivirus
  misc_feature: FeMoV "Lapön strain" L antigen "wild-type" nucleic acid; given as DNA sequence
atggagcagtcagactaccaagatattctatatccagaggtacatcttaacagtcctatagtaatttctaaattggtaggcattttggagtatgctcaagttattcataatcaacaattaacagatcatacaattattaagaatatccaatttagattaagaaatgggtttaatagtcccaggatacagacactgtcaactatgggtgaaatcatcaacaaaattaaaaacaagtatcctaattatattcatataccttatcccgaatgcaaccaaaaattgtttaggatagtagatccagaactaacatcaaaattagaatctcttctgaacaaaggtgatacactatttctcaaaattcggtcagatatcataaaatgtttcgataaactgaagatgaagatgaatataagtaatgatcttcttaatgacaatagtcaattaattttggatcttcctttaattatcaaaggatctcaatggtttttcccgtttttattttggttttctattaaaactgaaactagaagctgtattcgccaaaatccaaaagctcgtgttagatcacaatatcgaccccacttatcagagactaaaagaattacattagttgttacatctgatctgattacaatatttgatcatattaataaatgcacattttacctgacttttgaaatgctattgatgtattgcgatgtgatagaaggtaggttaatgactgaaacagctatgagcctggattgtcgatttaccaatctgttaccaagagtgcaatatatgtgggatttactagacggaatgtttgaaagtctaggtaatcagttatattcagttattgcattattagaacctctttctcttgcttatttgcaattgatagatgctgatccgcagattcggggaacattcttgcatcactgtttctcagagttagaagaaatcatatttgacaaatctccttttgacccttttgtgtatgaaaatcttatcaacggacttgattatatttatcttacagatgacattcatctaactgcagaagttttttctttttttagaagttttggtcatccttacttagaagcacaaaatgctgccaacaatgtgaggaagtatatgaatcagcctaaagtgatctcataccagaccttaatgcaaggacatgcaattttctgtggaattataataaatgggtttagagatcgtcatggaggaacatggcctcctgtagaattgccgagtcatgcatctgctgtaatcagaaatgcccaactatctggggaagggttaacatctgaacaatgtgctcaacattggagatcgttttgtgggtttaaattcaaatgttttatgccattaagtctagatagtgatcttacaatgtaccttcgagacaaagcattgtcacctgttagaagtgagtgggattctgtctatgctaaagagtatttaagatataatccaggattacctacaagttccagaagattagtgaatgtatttttagaagatgataagtttgacccatatgaaatgattatgtacgtgataaatggtgattacctacgagataatgagttcaacctttcatatagtcttaaagaaaaagagatcaaagaggttggtcgattgttcgccaaaatgacttataaaatgagggcttgtcmagtaatagctgaaaacttgattgctaatggagtagggaagttttttaaagacaatggaatggcaaaagatgaacataaactaactaagacattacacaaattagccatttcaggtgtacctaaagataattctcaactttatctagatgaatgctgggagcaggtagttcgacagtgttcaagtgatacacatacaacaaaaccgattatgagttcgcaaccaaagaggataattgaatcaaagtcttctagaccacctctcaatcatagggatacttttaaaggtaagagagacccgaatacacagttaaagtacccttcaaacaccgaatattatgagactatcagtagttttataactactgacctcaaaaagtactgtcttaattggcgatatgaatcaagtagtgtatttgcggagagacttaatgaaatttacggattgcccggatttttccagtggcttcataaaattttggaaaaatccgttttgtatgttagtgatccatctagcccacctgactttgatcaacatgtcgatatagaatcagttccaaacgaccacatctttattaaatatccaatgggtgggatagaggggttctgtcagaaattatggactattagtacaatcccatttctatacttagcagcctttgatacaggtgttagaatcgcatcattggttcagggcgataatcaagcgatcgcagtgacaaaaagagttccgtcatcttggagttactcgaagaaaaaggaagaatcaactaaaataacaacacagtatttccttaatttaaggcaacgtctgcatgatataggtcatgaattgaaagcaaatgagactatcatatcctctcatttctttgtttactctaaaggtatttattacgatggaatacttctttctcaggcacttaaaagtatggcaagatgtgtcttttggtctgaaacaattgttgatgagactagatcagcttgcagtaatatatccaccacacttgcgaaggcaattgaaaggggttatgataaatttgtggcatatgccatcaatatttataaaaccatacatcaagttttgattgcattatcttttaccatcaatcctactatgacaccagatatcacagaacctttctacaaaagcttagatctacttaaaaacctagtcttaattcctgcaccattagggggtatgaactacatgaacatgagcaggttgtttgttagaaatataggagatcccattactgcttcatttgctgatataaagcgcatgattgaatgtgggttgctgggatgtagtatcttgtcacagataatgtaccaaaagtgtggttcctctaagtatttagactgggctagcgatccttattcaataaaccttccgtatagccaaagtatgaccaaggtattgaagaatgtaacggcaagatatgtgctcatgcatagccccaaccctatgcttaaagatttgttccatgaaaagtcgcaagaagaggatgagattcttgctgagtttttattagaccgacatttaataattcctagggcagcacatgaaattttatcaaattcagtaacaggtgctagagaatctattgcaggtatgcttgacactactaagggtttgatccgtgctagtatgtcgagaggtggtttgacatcgtcacttgttttaaaattatcaacatatgattatcagcagtttagaacgtgtcttgaatggctttatgctcctaccacgggaattgctgtgagtgtcgatttatgttctgttttcttagctaagactatccgaaaaagaatgtgggttcacctaaccaaaggaagggagatttacgggttggaagtacctgacattttggaatgcatgcagaacaatataattatcgatcatgaagattgttactcatgtattcaaggatcgagatattatacatggttttttgtgccttcaaattgtcaactagatcagataaataagtcaacaaattctctccgagttccttatgttggatcaacaacagaagaaagaagtgatatgaggttatcatatgtgaggtcaccaagtcgaccacttaaagcggcagttagaattgcagctgtatatacatgggcttatggtgatgatgatttatcttggcacgaggcttggtatttagcaaggaccagagcaaatattacctttgatgaactcaaattaataacacctatagccacatctacgaatttagcacacagattaagagataggagtacccaggttaaatattcaggaacttctttagtaagagtagcgcgctacacaacaatctccaatgataatatgtcgttcattattaacaacaagaaagtagatactaactttgtctatcagcaaggcatgttgttaggcttgagtatactagagtacatatttagatattgtacaagcactggacaatcaaatactgtaattcacttacatgcagacgttaactgttgtatagtacagatgactgatcagccctatacacctagcttaacaaagaagctacctgatattaaacctattaataataaattgatatatgatccggctcctataattgatactgatgcagctagattatattctcaaaagtacctatcacatctaatagatttcccaagctggtcaactactcagcttaacacagtattggcaaaagtggtggcagtatctattgtggaattaataacaaaggcaagtaaagaccatcttaatgagataatagcagttgttggtgatgatgatattaatagttttattacggagtttctacttgttgatccacgtctgtttacactatacttaggccaatatacatcattacaatgggcatatgaagttcattaccatagaccagtaggtaagtaccagatggccgaagtgttacataatctactgtcaagggctagtcgaggtatatttagcgtattgactaatgcctttagccaccctagggtatatagaagattctgggaatgtggtttactagagcctatttatgggccctatatagggagtcagaatctacatactgcagtgattgattatatttataatgcatatattacttatctggatgcttatttatctgatcaggtagatgatactgatatcataatatgcgaaacagaggagacatgtctatcaaataggatcgacaattatcagagcaggcatttagctatacttatagatttgtattgtgattccactagatgccctaacataaaggggtcagatacaattatgcggaattcaattcttagatcttttatagacaatgagagacgaacaaatccactcggtttggcatggaatcttgatccgttacttgtggatcactttagctgttctattacatatctaagaagaggtattattaaacagatgaggttaagatttgatccaaacatatctcttgagttggctaagatgatcaaacctgatgtaatttatcaagcacctaaagttccgtcttcgtgggctcttatagatatcaatcctgaagtcaatgatcttaatacaatttttggagagctaaatagcaaatggaaagatattcctattgggcaaatcaggattcagaattatgaaatacatgcatataggagaattggggttaattcaactgcatgttataaggctctagagatattatctgttttaaatcgatttatgtccaatccattgggtgcactgtttttaggtgaaggagcaggatcaatgctggtcacataccgtgcttttattccatttaagacaatctattataatagtggtatttctgtgcaaaatgtgcaaggtcagagagaactgagtctatatccttctgaagtggcactggttgacaacaaaaatcgtttggctaatgaccctaatatcaaagtcttgtttaacggtaagccggagtctacgtgggttgggaatattgactgttttgcctatattcttagccatattgagaccgcaagcttgacattgatacatagtgatatcgagtccagtttaagcaagacaaaaaataagattcttgaagagctatgccacatcctatcaatggcacttatcttagggagacttggatccgtgttagtcattaaactactaccaagggtcggtgattatacctattcattttgcaagtatgcatcagagttctatcagcaaaactttctcatattacccagatttagtaatatgtcgtcatctgaagtttactacataggagttcaccttaatacaaacagattgattgatcctgatagaatagtacaatacataattagaaatttgcaacccaccccagttacatttttatcctatatctttgagactaaatatagaaacaatatggttacaaattatggactatgcttgtcagatggacacaaaagtgattacttatcatcaattaccaaaatagagaatgttcttctgtcatgtgaattagaattggatggacctaagattataccgccattatcaggacatgactatgcaaatggggagactagcctggaatcaagtataatgatattagttagagaatatcttaatgcaactattcaaggccgagaaacattaggcttgttttcaccttacccagtattacatgagagtcagctaagagaaattaataagtgtattgcattgaagtatattgtgtatttactcttttactcgaactctgtatcatctagtaaacagataatgagtaatcttagaaaagggatattaatgtatgatttgagagacgaatttttcatatcaagattatcagcaaattacaagaaaaaagtaatgtcacaggaagttaaaaccacatggatatttaatattgatacgccaacaagaaaagcattatacaagttagtgggttattcattgataattcatcacgtataa

SEQ ID NO: 44 - protein, 2201 aa, Feline Morbillivirus
  MISC_FEATURE: FeMoV "Lapön strain" L antigen translated amino acid sequence
MEQSDYQDILYPEVHLNSPIVISKLVGILEYAQVIHNQQLTDHTIIKNIQFRLRNGFNSPRIQTLSTMGEIINKIKNKYPNYIHIPYPECNQKLFRIVDPELTSKLESLLNKGDTLFLKIRSDIIKCFDKLKMKMNISNDLLNDNSQLILDLPLIIKGSQWFFPFLFWFSIKTETRSCIRQNPKARVRSQYRPHLSETKRITLVVTSDLITIFDHINKCTFYLTFEMLLMYCDVIEGRLMTETAMSLDCRFTNLLPRVQYMWDLLDGMFESLGNQLYSVIALLEPLSLAYLQLIDADPQIRGTFLHHCFSELEEIIFDKSPFDPFVYENLINGLDYIYLTDDIHLTAEVFSFFRSFGHPYLEAQNAANNVRKYMNQPKVISYQTLMQGHAIFCGIIINGFRDRHGGTWPPVELPSHASAVIRNAQLSGEGLTSEQCAQHWRSFCGFKFKCFMPLSLDSDLTMYLRDKALSPVRSEWDSVYAKEYLRYNPGLPTSSRRLVNVFLEDDKFDPYEMIMYVINGDYLRDNEFNLSYSLKEKEIKEVGRLFAKMTYKMRACVIAENLIANGVGKFFKDNGMAKDEHKLTKTLHKLAISGVPKDNSQLYLDECWEQVVRQCSSDTHTTKPIMSSQPKRIIESKSSRPPLNHRDTFKGKRDPNTQLKYPSNTEYYETISSFITTDLKKYCLNWRYESSSVFAERLNEIYGLPGFFQWLHKILEKSVLYVSDPSSPPDFDQHVDIESVPNDHIFIKYPMGGIEGFCQKLWTISTIPFLYLAAFDTGVRIASLVQGDNQAIAVTKRVPSSWSYSKKKEESTKITTQYFLNLRQRLHDIGHELKANETIISSHFFVYSKGIYYDGILLSQALKSMARCVFWSETIVDETRSACSNISTTLAKAIERGYDKFVAYAINIYKTIHQVLIALSFTINPTMTPDITEPFYKSLDLLKNLVLIPAPLGGMNYMNMSRLFVRNIGDPITASFADIKRMIECGLLGCSILSQIMYQKCGSSKYLDWASDPYSINLPYSQSMTKVLKNVTARYVLMHSPNPMLKDLFHEKSQEEDEILAEFLLDRHLIIPRAAHEILSNSVTGARESIAGMLDTTKGLIRASMSRGGLTSSLVLKLSTYDYQQFRTCLEWLYAPTTGIAVSVDLCSVFLAKTIRKRMWVHLTKGREIYGLEVPDILECMQNNIIIDHEDCYSCIQGSRYYTWFFVPSNCQLDQINKSTNSLRVPYVGSTTEERSDMRLSYVRSPSRPLKAAVRIAAVYTWAYGDDDLSWHEAWYLARTRANITFDELKLITPIATSTNLAHRLRDRSTQVKYSGTSLVRVARYTTISNDNMSFIINNKKVDTNFVYQQGMLLGLSILEYIFRYCTSTGQSNTVIHLHADVNCCIVQMTDQPYTPSLTKKLPDIKPINNKLIYDPAPIIDTDAARLYSQKYLSHLIDFPSWSTTQLNTVLAKVVAVSIVELITKASKDHLNEIIAVVGDDDINSFITEFLLVDPRLFTLYLGQYTSLQWAYEVHYHRPVGKYQMAEVLHNLLSRASRGIFSVLTNAFSHPRVYRRFWECGLLEPIYGPYIGSQNLHTAVIDYIYNAYITYLDAYLSDQVDDTDIIICETEETCLSNRIDNYQSRHLAILIDLYCDSTRCPNIKGSDTIMRNSILRSFIDNERRTNPLGLAWNLDPLLVDHFSCSITYLRRGIIKQMRLRFDPNISLELAKMIKPDVIYQAPKVPSSWALIDINPEVNDLNTIFGELNSKWKDIPIGQIRIQNYEIHAYRRIGVNSTACYKALEILSVLNRFMSNPLGALFLGEGAGSMLVTYRAFIPFKTIYYNSGISVQNVQGQRELSLYPSEVALVDNKNRLANDPNIKVLFNGKPESTWVGNIDCFAYILSHIETASLTLIHSDIESSLSKTKNKILEELCHILSMALILGRLGSVLVIKLLPRVGDYTYSFCKYASEFYQQNFLILPRFSNMSSSEVYYIGVHLNTNRLIDPDRIVQYIIRNLQPTPVTFLSYIFETKYRNNMVTNYGLCLSDGHKSDYLSSITKIENVLLSCELELDGPKIIPPLSGHDYANGETSLESSIMILVREYLNATIQGRETLGLFSPYPVLHESQLREINKCIALKYIVYLLFYSNSVSSSKQIMSNLRKGILMYDLRDEFFISRLSANYKKKVMSQEVKTTWIFNIDTPTRKALYKLVGYSLIIHHV

SEQ ID NO: 45 - DNA, 940 bp, Artificial Sequence
  ALVAC insertion locus C3 flanking region left arm; given as DNA sequence
caaatgtgagttaatattagtatactacattactaatttattacatattcatttatatcaatctagtagcatttagcttttataaaacaatataactgaatagtacatactttactaataagttataaataagagatacatatttatagtattttactttctacactgaatataataatataattatacaaatataatttttaatactatatagtatataactgaaataaaataccagtgtaatatagttattatacatttataccacatcaaagatgagttataacatcagtgtcactgttagcaacagtagttatacgatgagtagttactctcgtatggcgttagtatgtatgtatcttctagttttcttagtaggcattataggaaacgtcaagcttataaggttattaatggtatctagaaatatatctattataccgtttctcaacttgggaatagccgatttgctgtttgtgatattcatacctttatacattatatacatactaagtaatttccattggcattttggtaaagcactttgtaaaattagttctttcttttttacttctaacatgtttgcaagtatatttttaataactgtaataagcgtatatagatatgtaaaaattacccttcctggatttacctataaatatgttaacattagaaatatgtacattactatatttttcatatggattatttctattatactagggattcctgctctttactttagaaatactatcgtaacaaaaaataacgacacgctgtgtattaatcattatcatgataatagagaaattgctgaattgatttacaaagttattatctgtatcagatttattttaggatacctactacctacgataattatactcgtatgctatacgttactgatctacagaactaacaatgcatgtcgacgcggccg

SEQ ID NO: 46 - DNA, 1999 bp, Artificial Sequence
  ALVAC insertion locus C3 flanking region right arm; given as DNA sequence
atattattaaaactattagataacatagctttatgtaaaggagtatttccagataacttagctttagcatttacgtaagcaccgtggtcaagtaagagtttaacaaattctgttttcatagaactaactgccatgtatagaggagtgaaacctttatgattatagacgtttacatagcaaccatataataagatcgcattcagtatattaatatctttcatttctatagctatgtgaataacatgtttatctaatcctaccaactttgtatcagtaccgtacttcagtaataagtttactatagttttgtttttagatgcaacagctatatttagaacggtatctatatgattattaaccacattaacattagatcctctttctaaaagtgtctttgttgtttcgatatcgttacgtgaaacagcgtaatgtaagggactgcccatacagtcatctattacgtttatatcagctcctagatttaacagaagtgctgttacatcttttcttctattaattaccgaatgatgtaatggggttttacctaaatcatcttgttcgtttataggcactccgtgatttataagtaacgctattatatcgtaactacaattatttttaagtgcctttatgagatactgtttatgcaaaaataaacttttatctattttaatactattatctaacaatatcctaattaaatctatattcttatactttatagcgtaatgtaacggagtttcaaaatttctagtttgtatattaagatcaatattaaaatctataaatattttatacatatcatcagatatcttatcatacagtacatcgtaataatttagaaagaatctattacaattaacacctttttttaataaatatctagttaatgacttattgtttctatatacagaaatatataacggactatttccagaatgtatctgttctatgtcagcgccagaatctattagtagtttagcaatttctgtattatctaaactagcagctttatgaagaggaggatttttacattttaaaatatcggcaccgtgttctagtaataattttaccatttctatatcagaaatacttacggctaaatacaaagacgttgatagtatatttacgttattgtatttgcattttttaagtatataccttactaaatttatatctctataccttatagctttatgcagttcatttataagtcttccattactcatttctggtaatgaagtattatatatcattatgatattatctctattttattctaataaaaaccgttatcatgttatttattatttgttataattatactatttaataaattataccaaatacttagatacttattaataccatcctagaacttgtatttcttgccccctaaacttggacatgcactccattaggcgtttcttgttttcgacatcgtcctccttaacatatcctactgttatgtgaggattccacggattatctactgtgatatcaccaaacacgtccttcgaacagggtaccgcattcagcagaacatttcttagggctctaagttcatcagatacctccagtttcataactacagcgcatcctttcgctcccaactgtttagaggcgttactctgaggaaaacacatctcttctttacagactatagaaatagtctgtaaatcttgatcagttatttgctttttgaaattttcaaatctatcacattgatccatatttgctattccaagagttatatgaggaaaaatatcacatcctgtcatgtattttattgtaacattattataatctgtaacatcagtatctaacctaacgtcgtaaaagttaacagatgcccagttactataatcccaaggaaccttaacatctaatcccattaaaatagtatcctttctactatttttttcattggcaagtatgtggcttagtttacacaaaattcctgccattttgtaacgatagcgaagcaatagcttgtatg

SEQ ID NO: 47 - DNA, 405 bp, Artificial Sequence
  ALVAC insertion locus C5 flanking region left arm; given as DNA sequence
cttataaagatctaaaatgcataatttctaaataatgaaaaaaagtacatcatgagcaacgcgttagtatattttacaatggagattaacgctctataccgttctatgtttattgattcagatgatgttttagaaaagaaagttattgaatatgaaaactttaatgaagatgaagatgacgacgatgattattgttgtaaatctgttttagatgaagaagatgacgcgctaaagtatactatggttacaaagtataagtctatactactaatggcgacttgtgcaagaaggtatagtatagtgaaaatgttgttagattatgattatgaaaaaccaaataaatcagatccatatctaaaggtatctcctttgcacataatttcatctattcctagtttagaatac

SEQ ID NO: 48 - DNA, 1536 bp, Artificial Sequence
  ALVAC insertion locus C5 flanking region right arm; given as DNA sequence
tgaatgttaaatgttatactttggatgaagctataaatatgcattggaaaaataatccatttaaagaaaggattcaaatactacaaaacctaagcgataatatgttaactaagcttattcttaacgacgctttaaatatacacaaataaacataatttttgtataacctaacaaataactaaaacataaaaataataaaaggaaatgtaatatcgtaattattttactcaggaatggggttaaatatttatatcacgtgtatatctatactgttatcgtatactctttacaattactattacgaatatgcaagagataataagattacgtatttaagagaatcttgtcatgataattgggtacgacatagtgataaatgctatttcgcatcgttacataaagtcagttggaaagatggatttgacagatgtaacttaataggtgcaaaaatgttaaataacagcattctatcggaagataggataccagttatattatacaaaaatcactggttggataaaacagattctgcaatattcgtaaaagatgaagattactgcgaatttgtaaactatgacaataaaaagccatttatctcaacgacatcgtgtaattcttccatgttttatgtatgtgtttcagatattatgagattactataaactttttgtatacttatattccgtaaactatattaatcatgaagaaaatgaaaaagtatagaagctgttcacgagcggttgttgaaaacaacaaaattatacattcaagatggcttacatatacgtctgtgaggctatcatggataatgacaatgcatctctaaataggtttttggacaatggattcgaccctaacacggaatatggtactctacaatctcctcttgaaatggctgtaatgttcaagaataccgaggctataaaaatcttgatgaggtatggagctaaacctgtagttactgaatgcacaacttcttgtctgcatgatgcggtgttgagagacgactacaaaatagtgaaagatctgttgaagaataactatgtaaacaatgttctttacagcggaggctttactcctttgtgtttggcagcttaccttaacaaagttaatttggttaaacttctattggctcattcggcggatgtagatatttcaaacacggatcggttaactcctctacatatagccgtatcaaataaaaatttaacaatggttaaacttctattgaacaaaggtgctgatactgacttgctggataacatgggacgtactcctttaatgatcgctgtacaatctggaaatattgaaatatgtagcacactacttaaaaaaaataaaatgtccagaactgggaaaaattgatcttgccagctgtaattcatggtagaaaagaagtgctcaggctacttttcaacaaaggagcagatgtaaactacatctttgaaagaaatggaaaatcatatactgttttggaattgattaaagaaagttactctgagacacaaaagaggtagctgaagtggtactctcaaa

SEQ ID NO: 49 - DNA, 4170 bp, Artificial Sequence
  passage 3 C5 insertion locus of vCP3025 including C5 flanking region right arm, H6 vaccinia promoter, codon-optimized Gordon H antigen, C5 flanking region left arm, i.e. base pairs 304,701 to 308,870
aaatgactatgtaccgttattgcatgaacgatattataaatataggttctcgtaggagagaactattgactatggcaatgaatgttaaatgttatactttggatgaagctataaatatgcattggaaaaataatccatttaaagaaaggattcaaatactacaaaacctaagcgataatatgttaactaagcttattcttaacgacgctttaaatatacacaaataaacataatttttgtataacctaacaaataactaaaacataaaaataataaaaggaaatgtaatatcgtaattattttactcaggaatggggttaaatatttatatcacgtgtatatctatactgttatcgtatactctttacaattactattacgaatatgcaagagataataagattacgtatttaagagaatcttgtcatgataattgggtacgacatagtgataaatgctatttcgcatcgttacataaagtcagttggaaagatggatttgacagatgtaacttaataggtgcaaaaatgttaaataacagcattctatcggaagataggataccagttatattatacaaaaatcactggttggataaaacagattctgcaatattcgtaaaagatgaagattactgcgaatttgtaaactatgacaataaaaagccatttatctcaacgacatcgtgtaattcttccatgttttatgtatgtgtttcagatattatgagattactataaactttttgtatacttatattccgtaaactatattaatcatgaagaaaatgaaaaagtatagaagctgttcacgagcggttgttgaaaacaacaaaattatacattcaagatggcttacatatacgtctgtgaggctatcatggataatgacaatgcatctctaaataggtttttggacaatggattcgaccctaacacggaatatggtactctacaatctcctcttgaaatggctgtaatgttcaagaataccgaggctataaaaatcttgatgaggtatggagctaaacctgtagttactgaatgcacaacttcttgtctgcatgatgcggtgttgagagacgactacaaaatagtgaaagatctgttgaagaataactatgtaaacaatgttctttacagcggaggctttactcctttgtgtttggcagcttaccttaacaaagttaatttggttaaacttctattggctcattcggcggatgtagatatttcaaacacggatcggttaactcctctacatatagccgtatcaaataaaaatttaacaatggttaaacttctattgaacaaaggtgctgatactgacttgctggataacatgggacgtactcctttaatgatcgctgtacaatctggaaatattgaaatatgtagcacactacttaaaaaaaataaaatgtccagaactgggaaaaattgatcttgccagctgtaattcatggtagaaaagaagtgctcaggctacttttcaacaaaggagcagatgtaaactacatctttgaaagaaatggaaaatcatatactgttttggaattgattaaagaaagttactctgagacacaaaagaggtagctgaagtggtactctcaaaggtacgtgactaattagctataaaaaggatccgggttaattaattagtcatcaggcagggcgagaacgagactatctgctcgttaattaattagagcttctttattctatacttaaaaagtgaaaataaatacaaaggttcttgagggttgtgttaaattgaaagcgagaaataatcataaattatttcattatcgcgatatccgttaagtttgtatcgtaatggaaagcaataataacaaatactataaagacagcaatcggtacttcagcaagatcctggacgagaataagacagtcaataatcacctgtactccctgtctatcaggatcatcaccgtgatcgccatcgtggtgtccctgatcgcaaccactatcactatcatcaatgccatctctggcagaaccactctgaacaataacatggacatgctgctgaaccagcaggataagatcaataacatcaaagagatgatcttcgacaggatctatccactgatcaacgcaatgagcaccgagctggggctgcacatccctaccctgctggacgaactgactaagtccatcgatcagaagatcaaaatcatgactccacctctggaaaccactacctctaatctgaactggtgcatcaatcccccaaacggaatcatcgtggacccaaaaggctactgtgaggggctggaactgtccaagacctataaactgctgctggaccagctggatatgctgaggaagaaaagcctgatcatcaataagaaatccatcaaccagtgcagactggtggatagctccaatatcgtgttcgccaccgtgaacatccagagcactcctaggtttctgaatctgggacataccgtgtccaaccagagaatcactttcggacagggtacttactctagcacctatatcatcactatccaggaggacggtctgaccgatgtgcagtacagagtgtttgaaatcggctatatctctgaccagttcgggacttttccttctctgatcgtgagcagggtgctgcccgtgagaatggtgctggggatggagtcctgcactctgacctctgataagttcggcgggtacttcctgtgcatgaatatccccaccaggtctatctacgactatgtgaacatcagagatctgaagagcctgtacgtgaccatcccccactacggcaaaatcaattacacttatttcaactttgggaaggtgaggagcccacatgagatcgacaaaatctggctgacttctgaaagaggacagatgatcagcggttacttcgccgcatttgtgactatcaccatcaggaactacaacaactacccttacaagtgcctgcacaacccatgtctggagagaagcgaatcctactgcaagggatggtataagaacatcactggtaccgacgatgtgcccatcctggcctacctgctggtggagatgaacgatgaggaaggtccactgatcaccctggtggaaatccctccctacaattatactgcacctagccataactccctgtactatgacgataagatcaacaagctgatcatgactacctcccacatcggatatatccagatcaacgaggtgcatgaagtgatcgtgggtgacaatctgaaggccatcctgctgaacaggctgagcgatgagcacccaactctgaccgcatgtaggttcaatcaggagatcaaagaaagacatatctccgacggcctgatcatctctaacagcgccctgatcgatatccaggagaggatgtacgtgaccgtgaaggcagtgccacctatcggcaattataactttaccgtggaactgcactccagatctaatactagctacgtggggctgcctaggcagttcaacgcaagatatgacaaactgcatctggaatgctttgcctgggatagatcctggtggtgtgcactgatcccccagttttctctgtcctggaatgagagcctgtccgtggatactgctattttcaacctgataaactgtaactaactcgagtctagaatcgatcccgggtttttatgactagttaatcacggccgcttataaagatctaaaatgcataatttctaaataatgaaaaaaagtacatcatgagcaacgcgttagtatattttacaatggagattaacgctctataccgttctatgtttattgattcagatgatgttttagaaaagaaagttattgaatatgaaaactttaatgaagatgaagatgacgacgatgattattgttgtaaatctgttttagatgaagaagatgacgcgctaaagtatactatggttacaaagtataagtctatactactaatggcgacttgtgcaagaaggtatagtatagtgaaaatgttgttagattatgattatgaaaaaccaaataaatcagatccatatctaaaggtatctcctttgcacataatttcatctattcctagtttagaatacttttcattatatttgtttacagctgaagacgaaaaaaatatatcgataatagaagattatgttaactctgctaataagatgaaattgaatga

SEQ ID NO: 50 - DNA, 4215 bp, Artificial Sequence
  passage 3 C5 insertion locus of vCP3029 including C5 flanking region right arm, H6 vaccinia promoter, codon-optimized Gordon H antigen, C5 flanking region left arm, i.e. base pairs 304,166 to 308,380
tagttacttggataaattaatcgagacgcgtgataaaatgactatgtaccgttattgcatgaacgatattataaatataggttctcgtaggagagaactattgactatggcaatgaatgttaaatgttatactttggatgaagctataaatatgcattggaaaaataatccatttaaagaaaggattcaaatactacaaaacctaagcgataatatgttaactaagcttattcttaacgacgctttaaatatacacaaataaacataatttttgtataacctaacaaataactaaaacataaaaataataaaaggaaatgtaatatcgtaattattttactcaggaatggggttaaatatttatatcacgtgtatatctatactgttatcgtatactctttacaattactattacgaatatgcaagagataataagattacgtatttaagagaatcttgtcatgataattgggtacgacatagtgataaatgctatttcgcatcgttacataaagtcagttggaaagatggatttgacagatgtaacttaataggtgcaaaaatgttaaataacagcattctatcggaagataggataccagttatattatacaaaaatcactggttggataaaacagattctgcaatattcgtaaaagatgaagattactgcgaatttgtaaactatgacaataaaaagccatttatctcaacgacatcgtgtaattcttccatgttttatgtatgtgtttcagatattatgagattactataaactttttgtatacttatattccgtaaactatattaatcatgaagaaaatgaaaaagtatagaagctgttcacgagcggttgttgaaaacaacaaaattatacattcaagatggcttacatatacgtctgtgaggctatcatggataatgacaatgcatctctaaataggtttttggacaatggattcgaccctaacacggaatatggtactctacaatctcctcttgaaatggctgtaatgttcaagaataccgaggctataaaaatcttgatgaggtatggagctaaacctgtagttactgaatgcacaacttcttgtctgcatgatgcggtgttgagagacgactacaaaatagtgaaagatctgttgaagaataactatgtaaacaatgttctttacagcggaggctttactcctttgtgtttggcagcttaccttaacaaagttaatttggttaaacttctattggctcattcggcggatgtagatatttcaaacacggatcggttaactcctctacatatagccgtatcaaataaaaatttaacaatggttaaacttctattgaacaaaggtgctgatactgacttgctggataacatgggacgtactcctttaatgatcgctgtacaatctggaaatattgaaatatgtagcacactacttaaaaaaaataaaatgtccagaactgggaaaaattgatcttgccagctgtaattcatggtagaaaagaagtgctcaggctacttttcaacaaaggagcagatgtaaactacatctttgaaagaaatggaaaatcatatactgttttggaattgattaaagaaagttactctgagacacaaaagaggtagctgaagtggtactctcaaaggtacgtgactaattagctataaaaaggatccgggttaattaattagtcatcaggcagggcgagaacgagactatctgctcgttaattaattagagcttctttattctatacttaaaaagtgaaaataaatacaaaggttcttgagggttgtgttaaattgaaagcgagaaataatcataaattatttcattatcgcgatatccgttaagtttgtatcgtaatggaaagcaataataacaaatactataaagacagcaatcggtacttcagcaagatcctggacgagaataagacagtcaataatcacctgtactccctgtctatcaggatcatcaccgtgatcgccatcgtggtgtccctgatcgcaaccactatcactatcatcaatgccatctctggcagaaccactctgaacaataacatggacatgctgctgaaccagcaggataagatcaataacatcaaagagatgatcttcgacaggatctatccactgatcaacgcaatgagcaccgagctggggctgcacatccctaccctgctggacgaactgactaagtccatcgatcagaagatcaaaatcatgactccacctctggaaaccactacctctaatctgaactggtgcatcaatcccccaaacggaatcatcgtggacccaaaaggctactgtgaggggctggaactgtccaagacctataaactgctgctggaccagctggatatgctgaggaagaaaagcctgatcatcaataagaaatccatcaaccagtgcagactggtggatagctccaatatcgtgttcgccaccgtgaacatccagagcactcctaggtttctgaatctgggacataccgtgtccaaccagagaatcactttcggacagggtacttactctagcacctatatcatcactatccaggaggacggtctgaccgatgtgcagtacagagtgtttgaaatcggctatatctctgaccagttcgggacttttccttctctgatcgtgagcagggtgctgcccgtgagaatggtgctggggatggagtcctgcactctgacctctgataagttcggcgggtacttcctgtgcatgaatatccccaccaggtctatctacgactatgtgaacatcagagatctgaagagcctgtacgtgaccatcccccactacggcaaaatcaattacacttatttcaactttgggaaggtgaggagcccacatgagatcgacaaaatctggctgacttctgaaagaggacagatgatcagcggttacttcgccgcatttgtgactatcaccatcaggaactacaacaactacccttacaagtgcctgcacaacccatgtctggagagaagcgaatcctactgcaagggatggtataagaacatcactggtaccgacgatgtgcccatcctggcctacctgctggtggagatgaacgatgaggaaggtccactgatcaccctggtggaaatccctccctacaattatactgcacctagccataactccctgtactatgacgataagatcaacaagctgatcatgactacctcccacatcggatatatccagatcaacgaggtgcatgaagtgatcgtgggtgacaatctgaaggccatcctgctgaacaggctgagcgatgagcacccaactctgaccgcatgtaggttcaatcaggagatcaaagaaagacatatctccgacggcctgatcatctctaacagcgccctgatcgatatccaggagaggatgtacgtgaccgtgaaggcagtgccacctatcggcaattataactttaccgtggaactgcactccagatctaatactagctacgtggggctgcctaggcagttcaacgcaagatatgacaaactgcatctggaatgctttgcctgggatagatcctggtggtgtgcactgatcccccagttttctctgtcctggaatgagagcctgtccgtggatactgctattttcaacctgataaactgtaactaactcgagtctagaatcgatcccgggtttttatgactagttaatcacggccgcttataaagatctaaaatgcataatttctaaataatgaaaaaaagtacatcatgagcaacgcgttagtatattttacaatggagattaacgctctataccgttctatgtttattgattcagatgatgttttagaaaagaaagttattgaatatgaaaactttaatgaagatgaagatgacgacgatgattattgttgtaaatctgttttagatgaagaagatgacgcgctaaagtatactatggttacaaagtataagtctatactactaatggcgacttgtgcaagaaggtatagtatagtgaaaatgttgttagattatgattatgaaaaaccaaataaatcagatccatatctaaaggtatctcctttgcacataatttcatctattcctagtttagaatacttttcattatatttgtttacagctgaagacgaaaaaaatatatcgataatagaagattatgttaactctgctaataagatgaaattgaatgagtctgtgata

SEQ ID NO: 51 - DNA, 4200 bp, Artificial Sequence
  passage 3 C3 insertion locus of vCP3029 including C3 flanking region right arm, 42k (long) poxviral promoter, codon-optimized Gordon M antigen, C3 flanking region left arm, i.e. base pairs 38,608 to 42,807
cgtattaccgtgattatttagagaattatagtcggcgttataagataaaagtaattttatattattaaaactattagataacatagctttatgtaaaggagtatttccagataacttagctttagcatttacgtaagcaccgtggtcaagtaagagtttaacaaattctgttttcatagaactaactgccatgtatagaggagtgaaacctttatgattatagacgtttacatagcaaccatataataagatcgcattcagtatattaatatctttcatttctatagctatgtgaataacatgtttatctaatcctaccaactttgtatcagtaccgtacttcagtaataagtttactatagttttgtttttagatgcaacagctatatttagaacggtatctatatgattattaaccacattaacattagatcctctttctaaaagtgtctttgttgtttcgatatcgttacgtgaaacagcgtaatgtaagggactgcccatacagtcatctattacgtttatatcagctcctagatttaacagaagtgctgttacatcttttcttctattaattaccgaatgatgtaatggggttttacctaaatcatcttgttcgtttataggcactccgtgatttataagtaacgctattatatcgtaactacaattatttttaagtgcctttatgagatactgtttatgcaaaaataaacttttatctattttaatactattatctaacaatatcctaattaaatctatattcttatactttatagcgtaatgtaacggagtttcaaaatttctagtttgtatattaagatcaatattaaaatctataaatattttatacatatcatcagatatcttatcatacagtacatcgtaataatttagaaagaatctattacaattaacacctttttttaataaatatctagttaatgacttattgtttctatatacagaaatatataacggactatttccagaatgtatctgttctatgtcagcgccagaatctattagtagtttagcaatttctgtattatctaaactagcagctttatgaagaggaggatttttacattttaaaatatcggcaccgtgttctagtaataattttaccatttctatatcagaaatacttacggctaaatacaaagacgttgatagtatatttacgttattgtatttgcattttttaagtatataccttactaaatttatatctctataccttatagctttatgcagttcatttataagtcttccattactcatttctggtaatgaagtattatatatcattatgatattatctctattttattctaataaaaaccgttatcatgttatttattatttgttataattatactatttaataaattataccaaatacttagatacttattaataccatcctagaacttgtatttcttgccccctaaacttggacatgcactccattaggcgtttcttgttttcgacatcgtcctccttaacatatcctactgttatgtgaggattccacggattatctactgtgatatcaccaaacacgtccttcgaacagggtaccgcattcagcagaacatttcttagggctctaagttcatcagatacctccagtttcataactacagcgcatcctttcgctcccaactgtttagaggcgttactctgaggaaaacacatctcttctttacagactatagaaatagtctgtaaatcttgatcagttatttgctttttgaaattttcaaatctatcacattgatccatatttgctattccaagagttatatgaggaaaaatatcacatcctgtcatgtattttattgtaacattattataatctgtaacatcagtatctaacctaacgtcgtaaaagttaacagatgcccagttactataatcccaaggaaccttaacatctaatcccattaaaatagtatcctttctactatttttttcattggcaagtatgtggcttagtttacacaaaattcctgccattttgtaacgatagcgaagcaatagcttgtatgctttttatttgattaactagtcataaaaatcgggatcctcaaaaaaatataaatgattcaccatctgatagaaaaaaaatttattgggagaatatgataatattttgggatttcaaaattgaaaatatataattacaatataaaatgactgagatcttcaacctggacgaaagctcttggagtgttaaagggaccctggaccctctgacccccgatacctaccccgatgggaggctggtgccaaagatcagagtgatcgaccctgggctgggggataggaaaagcgggggctacatgtatctgctgctgcacggggtgatcgaggactctgaaaccgtgatcaaccccaaggggagagccttcggggcatttccactgggggtggggcagagcaccgagaatcccgaagatctgttcaaggagatcctgactctgaacatcgtgaccaggagaactgccgggtttaatgaaaaactggtgtactataacaccactcctctgaatctgctgactccctggaagaaagtgctggcctacgggtctatcttcaccgcaaaccaagtgtgtaacaatactagctccatccccatcgacatcccacagaagtttaggcctgtgtatctgaccgtgactaaactgagcgacgatgggtactatcagatccccaagatgatccaggacttcaaatctagcaactctgtggcatttaatatcctggtgcacctgagcatggggaccatcctgctggattcctctaaggggagcagggtggggaacccagccgagaatctgatcactttcatgatccatatcgggaacttcaagagaaagaacaacaaggcatactcccctgaatattgcaagaggaaaatcatgagactggggctgatcttcagcctgggggcaatcgggggcacctccctgcatatcaggtgcactgggaagatgtccaaaagactgcaggcatacctggggtttaagaggaccctgtgttaccctctgatgtatgtgaacgaggggctgaataaaactctgtggagaaacgagtgcaagatcgaaaaagtgcaggccgtgctgcagccatctgtgcctaatgagttcaaaatatacgacgacattatcatagacaatacaaacgggctgttcaaagtcaagtaactcgaggaattcctgcagcccgggtttttatagctaattagtcaaatgtgagttaatattagtatactacattactaatttattacatattcatttatatcaatctagtagcatttagcttttataaaacaatataactgaatagtacatactttactaataagttataaataagagatacatatttatagtattttactttctacactgaatataataatataattatacaaatataatttttaatactatatagtatataactgaaataaaataccagtgtaatatagttattatacatttataccacatcaaagatgagttataacatcagtgtcactgttagcaacagtagttatacgatgagtagttactctcgtatggcgttagtatgtatgtatcttctagttttcttagtaggcattataggaaacgtcaagcttataaggttattaatggtatctagaaatatatctattataccgtttctcaacttgggaatagccgatttgctgtttgtgatattcatacctttatacattatatacatactaagtaatttccattggcattttggtaaagcactttgtaaaattagttctttcttttttacttctaacatgtttgcaagtatatttttaataactgtaataagcgtatatagatatgtaaaaattacccttcctggatttacctataaatatgttaacattagaaatatgtacattactatatttttcatatggattatttctattatactagggattcctgctctttactttagaaatactatcgtaacaaaaaataacgacacgctgtgtattaatcattatcatgataatagagaaattgctgaattgatttacaaagttattatctgtatcagatttattttaggatacctactacctacgataattatactcgtatgctatacgttactgatctacagaactaacaatgcatctaatatatctgataa

SEQ ID NO: 52 - DNA, 23 bp, Artificial Sequence
  PCR Primer "Gordon_M_probe_F"
ggagatcctgactctgaacatcg

SEQ ID NO: 53 - DNA, 23 bp, Artificial Sequence
  PCR Primer "Gordon_M_probe_R"
ctccacagagttttattcagccc

SEQ ID NO: 54 - DNA, 25 bp, Artificial Sequence
  PCR Primer "C3F"
cgtagagttttttgtctagttctat

SEQ ID NO: 55 - DNA, 25 bp, Artificial Sequence
  PCR Primer "C3R"
gttgttttatgcggtaaagaataat

SEQ ID NO: 56 - DNA, 24 bp, Artificial Sequence
  PCR Primer "7520"
tcttgcttcgcagtcatcgttctg

SEQ ID NO: 57 - DNA, 21 bp, Artificial Sequence
  PCR Primer "7521"
tctaaaatgcataatttctaa

SEQ ID NO: 58 - DNA, 26 bp, Artificial Sequence
  PCR Primer "C3-PCR-F"
gctaacacaagttagaggcgtattac

SEQ ID NO: 59 - DNA, 27 bp, Artificial Sequence
  PCR Primer "C3-PCR-R"
cattaattatgtgatgaggcatccaac

SEQ ID NO: 60 - DNA, 20 bp, Artificial Sequence
  PCR Primer "C3-R1"
tttataggtaaatccaggaa

SEQ ID NO: 61 - DNA, 25 bp, Artificial Sequence
  PCR Primer "C3-R2"
gcctactaagaaaactagaagatac

SEQ ID NO: 62 - DNA, 24 bp, Artificial Sequence
  PCR Primer "C3-R3"
agattgatataaatgaatatgtaa

SEQ ID NO: 63 - DNA, 20 bp, Artificial Sequence
  PCR Primer "C3-R4"
cgacgttaggttagatactg

SEQ ID NO: 64 - DNA, 20 bp, Artificial Sequence
  PCR Primer "C3-R5"
atgcggtaccctgttcgaag

SEQ ID NO: 65 - DNA, 20 bp, Artificial Sequence
  PCR Primer "C3-R6"
cagaaatgagtaatggaaga

SEQ ID NO: 66 - DNA, 20 bp, Artificial Sequence
  PCR Primer "C3-R7"
ctggaaatagtccgttatat

SEQ ID NO: 67 - DNA, 22 bp, Artificial Sequence
  PCR Primer "C3-R8"
cagtatctcataaaggcactta

SEQ ID NO: 68 - DNA, 24 bp, Artificial Sequence
  PCR Primer "C3-R9"
ccgttctaaatatagctgttgcat

SEQ ID NO: 69 - DNA, 22 bp, Artificial Sequence
  PCR Primer "Gordon_M_1F"
atgactgagatcttcaacctgg

SEQ ID NO: 70 - DNA, 20 bp, Artificial Sequence
  PCR Primer "Gordon_M_2F"
tgagcatggggaccatcctg

SEQ ID NO: 71 - DNA, 23 bp, Artificial Sequence
  PCR Primer "Gordon_M_3F"
gggctgaataaaactctgtggag

SEQ ID NO: 72 - DNA, 23 bp, Artificial Sequence
  PCR Primer "Gordon_M_1R"
cgatgttcagagtcaggatctcc

SEQ ID NO: 73 - DNA, 20 bp, Artificial Sequence
  PCR Primer "C3-F5"
cacggattatctactgtgat

SEQ ID NO: 74 - DNA, 22 bp, Artificial Sequence
  PCR Primer "C3-F7"
gcaacagtagttatacgatgag

SEQ ID NO: 75 - DNA, 25 bp, Artificial Sequence
  PCR Primer "7931"
gaatctgttagttagttacttggat

SEQ ID NO: 76 - DNA, 25 bp, Artificial Sequence
  PCR Primer "7932"
tgattatagctattatcacagactc

SEQ ID NO: 77 - DNA, 26 bp, Artificial Sequence
  PCR Primer "7927.DC"
ctcttgcatattcgtaatagtaattg

SEQ ID NO: 78 - DNA, 25 bp, Artificial Sequence
  PCR Primer "7696.CXL"
attctatcggaagataggataccag

SEQ ID NO: 79 - DNA, 26 bp, Artificial Sequence
  PCR Primer "7697.CXL"
atgcacaacttcttgtctgcatgatg

SEQ ID NO: 80 - DNA, 26 bp, Artificial Sequence
  PCR Primer "7925.DC"
tacggctatatgtagaggagttaacc

SEQ ID NO: 81 - DNA, 25 bp, Artificial Sequence
  PCR Primer "7792.SL"
ctctgagacacaaaagaggtagctg

SEQ ID NO: 82 - DNA, 25 bp, Artificial Sequence
  PCR Primer "7793SL"
catagaacggtatagagcgttaatc

SEQ ID NO: 83 - DNA, 25 bp, Artificial Sequence
  PCR Primer "7928.DC"
catcatgagcaacgcgttagtatat

SEQ ID NO: 84 - DNA, 25 bp, Artificial Sequence
  PCR Primer "7929.DC"
ggagatacctttagatatggatctg

SEQ ID NO: 85 - DNA, 25 bp, Artificial Sequence
  PCR Primer "7926.DC"
tcaacaaccgctcgtgaacagcttc

SEQ ID NO: 86 - DNA, 20 bp, Artificial Sequence
  PCR Primer "Gordon_H_1R"
gctcggtgctcattgcgttg

SEQ ID NO: 87 - DNA, 20 bp, Artificial Sequence
  PCR Primer "Gordon_H_2F"
caacgcaatgagcaccgagc

SEQ ID NO: 88 - DNA, 19 bp, Artificial Sequence
  PCR Primer "Gordon_H_probe_R"
cactgccttcacggtcacg

SEQ ID NO: 89 - DNA, 20 bp, Artificial Sequence
  PCR Primer "Gordon_H_probe_F"
gttcgccaccgtgaacatcc

SEQ ID NO: 90 - DNA, 23 bp, Artificial Sequence
  PCR Primer "Gordon_H_1F"
tcgcgatatccgttaagtttgta

SEQ ID NO: 91 - DNA, 25 bp, Artificial Sequence
  PCR Primer "Gordon_H_3F"
gaatatccccaccaggtctatctac

SEQ ID NO: 92 - DNA, 20 bp, Artificial Sequence
  PCR Primer "Gordon_H_4F"
taccgacgatgtgcccatcc

SEQ ID NO: 93 - DNA, 20 bp, Artificial Sequence
  PCR Primer "Gordon_H_5F"
atctccgacggcctgatcat

SEQ ID NO: 94 - DNA, 1788 bp, Feline Morbillivirus
  misc_feature: FeMoV "Lapön strain" H antigen "wild-type" - without BamH1 restriction enzyme site - nucleic acid; given as DNA sequence
atggagtccaacaacattaaatattacaaagactctaatcggtatcttggtaaaatattagatgaacacaagacagttaataatcaattgtacaggttgagtattaaagtaattaccattattgctattattgtaagcttaattgcaacaataataactattattaatgccacaagtggaagaactaccctaaacagtaatacagacatactgcttagccaaagagatgagattcatagtattcatgaaatgatatttgaccgtatttatcctttgataactgctatgagtacagagctaggacttcatattcctactttattagatgaacttactaaagcaattgatcaaaaaattaaaataatgaatcctcccgttgatactgtaacatctgatcttaactggtgtatcaaacctcctaatgggattattatggacccaaaaggttattgcgaaagtatggaattatctaaaacttacaaattattgcttgatcagttagatgtctcaagaaagaaatcgctcattataaatagaaagaatatcaaccagtgtcaattagttgatgactcaaagatcacttttgctactgttaatatacaatctacaccaaggtttttaaattttggtcatacagtcagcaatcaacgtataacatttggtcaaggaacttatagtagtacttatattataactatccaagaagatggaataaatgatgttcaatatcgagtgtttgaaattggatatatctctgatcagtttggttttttcccctcattaatagtatctagggtattgcctatacgtatggtattgggaatggaatcctgtaccttgacgagtgatcgacaaggtgggtatttcttatgtatgaatacattaacacggtctatatatgattatgtcaatataagagatttgaaatcactatacataacacttcctcattatggtaaggttaattatacttacttcaattttgggaaaattaggagcccacatgagattgataaaatttggctaacgtccgaaagaggtcaaattatttctggttattttgcagcatttgtcacaattacgattcgaaattataataattatccctacaaatgtttgaataatccatgttttgacaactctgagaattactgtaggggatggtataagaacataacaggcaccgatgatgttccaatactagcatacttactagttgaaatgtatgatgaagaaggacctttaattacacttgtagcaataccaccttacaattatacagctccatctcataattctctttactatgatgacaaaattaataagttgataatgactacatctcacactgggtatatacagatcaatgaggtgcatgaggtgattgttggtgatgatttaaaggctattctcctgaacagattatctgatgaacaccctaatcttacagcctgtagacttaatcaaggcattaaagagcagtacaagtccgatggaacgataatttcaaattctgcacttattgatatacaagaacgaatgtatattacagtcaaagctattccaccagtaggtaactataactttacagttgagttgcactctagatcaaacacatcttatatattgttaccgaaacagttcaatgccaagtatgacaaattacatcttgagtgctttaattgggacaagtcttggtggtgtgctttgatacctcaattttcattaagttggaatgaatccctttctgttgatactgctatttttaatttaataaattgtaaatga

SEQ ID NO: 95 - DNA, 4900 bp, Artificial Sequence
  vCP3041:cloned insertion locus C3 and its theoretical nucleotide sequence from  38,619 to 43,588 bp including C3 right flanking sequence, 42k (long) promoter, Lapön H (wt; no BamH I restriction enzyme site) and C3 left flanking sequence
atattattaaaactattagataacatagctttatgtaaaggagtatttccagataacttagctttagcatttacgtaagcaccgtggtcaagtaagagtttaacaaattctgttttcatagaactaactgccatgtatagaggagtgaaacctttatgattatagacgtttacatagcaaccatataataagatcgcattcagtatattaatatctttcatttctatagctatgtgaataacatgtttatctaatcctaccaactttgtatcagtaccgtacttcagtaataagtttactatagttttgtttttagatgcaacagctatatttagaacggtatctatatgattattaaccacattaacattagatcctctttctaaaagtgtctttgttgtttcgatatcgttacgtgaaacagcgtaatgtaagggactgcccatacagtcatctattacgtttatatcagctcctagatttaacagaagtgctgttacatcttttcttctattaattaccgaatgatgtaatggggttttacctaaatcatcttgttcgtttataggcactccgtgatttataagtaacgctattatatcgtaactacaattatttttaagtgcctttatgagatactgtttatgcaaaaataaacttttatctattttaatactattatctaacaatatcctaattaaatctatattcttatactttatagcgtaatgtaacggagtttcaaaatttctagtttgtatattaagatcaatattaaaatctataaatattttatacatatcatcagatatcttatcatacagtacatcgtaataatttagaaagaatctattacaattaacacctttttttaataaatatctagttaatgacttattgtttctatatacagaaatatataacggactatttccagaatgtatctgttctatgtcagcgccagaatctattagtagtttagcaatttctgtattatctaaactagcagctttatgaagaggaggatttttacattttaaaatatcggcaccgtgttctagtaataattttaccatttctatatcagaaatacttacggctaaatacaaagacgttgatagtatatttacgttattgtatttgcattttttaagtatataccttactaaatttatatctctataccttatagctttatgcagttcatttataagtcttccattactcatttctggtaatgaagtattatatatcattatgatattatctctattttattctaataaaaaccgttatcatgttatttattatttgttataattatactatttaataaattataccaaatacttagatacttattaataccatcctagaacttgtatttcttgccccctaaacttggacatgcactccattaggcgtttcttgttttcgacatcgtcctccttaacatatcctactgttatgtgaggattccacggattatctactgtgatatcaccaaacacgtccttcgaacagggtaccgcattcagcagaacatttcttagggctctaagttcatcagatacctccagtttcataactacagcgcatcctttcgctcccaactgtttagaggcgttactctgaggaaaacacatctcttctttacagactatagaaatagtctgtaaatcttgatcagttatttgctttttgaaattttcaaatctatcacattgatccatatttgctattccaagagttatatgaggaaaaatatcacatcctgtcatgtattttattgtaacattattataatctgtaacatcagtatctaacctaacgtcgtaaaagttaacagatgcccagttactataatcccaaggaaccttaacatctaatcccattaaaatagtatcctttctactatttttttcattggcaagtatgtggcttagtttacacaaaattcctgccattttgtaacgatagcgaagcaatagcttgtatgctttttatttgattaactagtcataaaaatcgggatcctcaaaaaaatataaatgattcaccatctgatagaaaaaaaatttattgggagaatatgataatattttgggatttcaaaattgaaaatatataattacaatataaaatggagtccaacaacattaaatattacaaagactctaatcggtatcttggtaaaatattagatgaacacaagacagttaataatcaattgtacaggttgagtattaaagtaattaccattattgctattattgtaagcttaattgcaacaataataactattattaatgccacaagtggaagaactaccctaaacagtaatacagacatactgcttagccaaagagatgagattcatagtattcatgaaatgatatttgaccgtatttatcctttgataactgctatgagtacagagctaggacttcatattcctactttattagatgaacttactaaagcaattgatcaaaaaattaaaataatgaatcctcccgttgatactgtaacatctgatcttaactggtgtatcaaacctcctaatgggattattatggacccaaaaggttattgcgaaagtatggaattatctaaaacttacaaattattgcttgatcagttagatgtctcaagaaagaaatcgctcattataaatagaaagaatatcaaccagtgtcaattagttgatgactcaaagatcacttttgctactgttaatatacaatctacaccaaggtttttaaattttggtcatacagtcagcaatcaacgtataacatttggtcaaggaacttatagtagtacttatattataactatccaagaagatggaataaatgatgttcaatatcgagtgtttgaaattggatatatctctgatcagtttggttttttcccctcattaatagtatctagggtattgcctatacgtatggtattgggaatggaatcctgtaccttgacgagtgatcgacaaggtgggtatttcttatgtatgaatacattaacacggtctatatatgattatgtcaatataagagatttgaaatcactatacataacacttcctcattatggtaaggttaattatacttacttcaattttgggaaaattaggagcccacatgagattgataaaatttggctaacgtccgaaagaggtcaaattatttctggttattttgcagcatttgtcacaattacgattcgaaattataataattatccctacaaatgtttgaataatccatgttttgacaactctgagaattactgtaggggatggtataagaacataacaggcaccgatgatgttccaatactagcatacttactagttgaaatgtatgatgaagaaggacctttaattacacttgtagcaataccaccttacaattatacagctccatctcataattctctttactatgatgacaaaattaataagttgataatgactacatctcacactgggtatatacagatcaatgaggtgcatgaggtgattgttggtgatgatttaaaggctattctcctgaacagattatctgatgaacaccctaatcttacagcctgtagacttaatcaaggcattaaagagcagtacaagtccgatggaacgataatttcaaattctgcacttattgatatacaagaacgaatgtatattacagtcaaagctattccaccagtaggtaactataactttacagttgagttgcactctagatcaaacacatcttatatattgttaccgaaacagttcaatgccaagtatgacaaattacatcttgagtgctttaattgggacaagtcttggtggtgtgctttgatacctcaattttcattaagttggaatgaatccctttctgttgatactgctatttttaatttaataaattgtaaatgactcgaggaattcctgcagcccgggtttttatagctaattagtcaaatgtgagttaatattagtatactacattactaatttattacatattcatttatatcaatctagtagcatttagcttttataaaacaatataactgaatagtacatactttactaataagttataaataagagatacatatttatagtattttactttctacactgaatataataatataattatacaaatataatttttaatactatatagtatataactgaaataaaataccagtgtaatatagttattatacatttataccacatcaaagatgagttataacatcagtgtcactgttagcaacagtagttatacgatgagtagttactctcgtatggcgttagtatgtatgtatcttctagttttcttagtaggcattataggaaacgtcaagcttataaggttattaatggtatctagaaatatatctattataccgtttctcaacttgggaatagccgatttgctgtttgtgatattcatacctttatacattatatacatactaagtaatttccattggcattttggtaaagcactttgtaaaattagttctttcttttttacttctaacatgtttgcaagtatatttttaataactgtaataagcgtatatagatatgtaaaaattacccttcctggatttacctataaatatgttaacattagaaatatgtacattactatatttttcatatggattatttctattatactagggattcctgctctttactttagaaatactatcgtaacaaaaaataacgacacgctgtgtattaatcattatcatgataatagagaaattgctgaattgatttacaaagttattatctgtatcagatttattttaggatacctactacctacgataattatactcgtatgctatacgttactgatctacagaactaacaatgcat